European Patent Application EP 4 480 965 A1, published December 25, 2024. Title: Transferrin receptor-binding molecules, conjugates thereof and their uses to prevent or treat CNS diseases. Applicant: VECT-HORUS. The sequence listing filed with the application follows.

SEQUENCE LISTING (738 sequences)

SEQ ID NO: 1 - protein, 8 aa, synthetic construct
GTDFSINF

SEQ ID NO: 2 - protein, 7 aa, synthetic construct
FTATGNT

SEQ ID NO: 3 - protein, 5 aa, synthetic construct
YMLDK

SEQ ID NO: 4 - protein, 136 aa, synthetic construct
EVQLVESGGGVVQPGGSLKLSCVASGTDFSINFIRWYRQAPGKQREFVAGFTATGNTNYADSMKGRFTISRDNTKNAVYLQIDSLKPEDTAVYYCYMLDKWGQGTQVTVSSAAAEQKLISEEDLNGAAHHHHHHGS

SEQ ID NO: 5 - protein, 8 aa, synthetic construct
GEIFSINF

SEQ ID NO: 6 - protein, 7 aa, synthetic construct
FTRDGST

SEQ ID NO: 7 - protein, 5 aa, synthetic construct
YMLDT

SEQ ID NO: 8 - protein, 136 aa, synthetic construct
EVQLVESGGGVVQPGGSLRLSCAASGEIFSINFMRWYRQAPGKQREWVAGFTRDGSTNYPDSAKGRFTISRDNAKNTVYLQIDSLKPEDTAVYYCYMLDTWGQGTQVTVSSAAAEQKLISEEDLNGAAHHHHHHGS

SEQ ID NO: 9 - protein, 8 aa, synthetic construct
GGPIEQYP

SEQ ID NO: 10 - protein, 9 aa, synthetic construct
ISRSGDGTY

SEQ ID NO: 11 - protein, 9 aa, synthetic construct
GAGINPTKI

SEQ ID NO: 12 - protein, 142 aa, synthetic construct
EVQLVESGGGLVQPGGSLRLSCTASGGPIEQYPMGWFRRAPGKERELVASISRSGDGTYYAISSVKGRFTISRDNAENTVFLQMNSLKPDDTAVYYCGAGINPTKIWGQGTQVTVSSAAAEQKLISEEDLNGAAHHHHHHGS

SEQ ID NO: 13 - protein, 8 aa, synthetic construct
GTDFSINF

SEQ ID NO: 14 - protein, 7 aa, synthetic construct
FTANGDT

SEQ ID NO: 15 - protein, 5 aa, synthetic construct
YMLDN

SEQ ID NO: 16 - protein, 136 aa, synthetic construct
EVQLVESGGGEVQPGGSLKLSCVASGTDFSINFVRWYRQRPGKQREWVAGFTANGDTNYPDSMKGRFTISRDNAKNTVYLQINSLKSEDTAVYYCYMLDNWGQGTQVTVSSAAAEQKLISEEDLNGAAHHHHHHGS

SEQ ID NO: 17 - protein, 8 aa, synthetic construct
GADFSINF

SEQ ID NO: 18 - protein, 136 aa, synthetic construct
EVQLVESGGGVVQPGGSLKLSCVASGADFSINFIRWYRQAPGKQREFVAGFTATGNTNYADSMKGRFTISRDNTKNAVYLQIDSLKPEDTAVYYCYMLDKWGQGTQVTVSSAAAEQKLISEEDLNGAAHHHHHHGS

SEQ ID NO: 19 - protein, 8 aa, synthetic construct
GTAFSINF

SEQ ID NO: 20 - protein, 136 aa, synthetic construct
EVQLVESGGGVVQPGGSLKLSCVASGTAFSINFIRWYRQAPGKQREFVAGFTATGNTNYADSMKGRFTISRDNTKNAVYLQIDSLKPEDTAVYYCYMLDKWGQGTQVTVSSAAAEQKLISEEDLNGAAHHHHHHGS

SEQ ID NO: 21 - protein, 7 aa, synthetic construct
FTAAGNT

SEQ ID NO: 22 - protein, 136 aa, synthetic construct
EVQLVESGGGVVQPGGSLKLSCVASGTDFSINFIRWYRQAPGKQREFVAGFTAAGNTNYADSMKGRFTISRDNTKNAVYLQIDSLKPEDTAVYYCYMLDKWGQGTQVTVSSAAAEQKLISEEDLNGAAHHHHHHGS

SEQ ID NO: 23 - protein, 7 aa, synthetic construct
FTATGAT

SEQ ID NO: 24 - protein, 136 aa, synthetic construct
EVQLVESGGGVVQPGGSLKLSCVASGTDFSINFIRWYRQAPGKQREFVAGFTATGATNYADSMKGRFTISRDNTKNAVYLQIDSLKPEDTAVYYCYMLDKWGQGTQVTVSSAAAEQKLISEEDLNGAAHHHHHHGS

SEQ ID NO: 25 - protein, 5 aa, synthetic construct
AMLDK

SEQ ID NO: 26 - protein, 136 aa, synthetic construct
EVQLVESGGGVVQPGGSLKLSCVASGTDFSINFIRWYRQAPGKQREFVAGFTATGNTNYADSMKGRFTISRDNTKNAVYLQIDSLKPEDTAVYYCAMLDKWGQGTQVTVSSAAAEQKLISEEDLNGAAHHHHHHGS

SEQ ID NO: 27 - protein, 5 aa, synthetic construct
YALDK

SEQ ID NO: 28 - protein, 136 aa, synthetic construct
EVQLVESGGGVVQPGGSLKLSCVASGTDFSINFIRWYRQAPGKQREFVAGFTATGNTNYADSMKGRFTISRDNTKNAVYLQIDSLKPEDTAVYYCYALDKWGQGTQVTVSSAAAEQKLISEEDLNGAAHHHHHHGS

SEQ ID NO: 29 - protein, 5 aa, synthetic construct
YMADK

SEQ ID NO: 30 - protein, 136 aa, synthetic construct
EVQLVESGGGVVQPGGSLKLSCVASGTDFSINFIRWYRQAPGKQREFVAGFTATGNTNYADSMKGRFTISRDNTKNAVYLQIDSLKPEDTAVYYCYMADKWGQGTQVTVSSAAAEQKLISEEDLNGAAHHHHHHGS

SEQ ID NO: 31 - protein, 5 aa, synthetic construct
YMLAK

SEQ ID NO: 32 - protein, 136 aa, synthetic construct
EVQLVESGGGVVQPGGSLKLSCVASGTDFSINFIRWYRQAPGKQREFVAGFTATGNTNYADSMKGRFTISRDNTKNAVYLQIDSLKPEDTAVYYCYMLAKWGQGTQVTVSSAAAEQKLISEEDLNGAAHHHHHHGS

SEQ ID NO: 33 - protein, 5 aa, synthetic construct
YMLDA

SEQ ID NO: 34 - protein, 136 aa, synthetic construct
EVQLVESGGGVVQPGGSLKLSCVASGTDFSINFIRWYRQAPGKQREFVAGFTATGNTNYADSMKGRFTISRDNTKNAVYLQIDSLKPEDTAVYYCYMLDAWGQGTQVTVSSAAAEQKLISEEDLNGAAHHHHHHGS

SEQ ID NO: 35 - protein, 25 aa, synthetic construct
EVQLVESGGGLVQPGGSLKLSCAAS

SEQ ID NO: 36 - protein, 25 aa, synthetic construct
EVQLVESGGGVVQPGGSLKLSCVAS

SEQ ID NO: 37 - protein, 25 aa, synthetic construct
EVQLVESGGGVVQPGGSLRLSCAAS

SEQ ID NO: 38 - protein, 25 aa, synthetic construct
EVQLVESGGGLVQPGGSLRLSCTAS

SEQ ID NO: 39 - protein, 25 aa, synthetic construct
EVQLVESGGGEVQPGGSLKLSCVAS

SEQ ID NO: 40 - protein, 17 aa, synthetic construct
MRWYRQAPGKQRELVAT

SEQ ID NO: 41 - protein, 17 aa, synthetic construct
IRWYRQAPGKQREFVAG

SEQ ID NO: 42 - protein, 17 aa, synthetic construct
MRWYRQAPGKQREWVAG

SEQ ID NO: 43 - protein, 17 aa, synthetic construct
MGWFRRAPGKERELVAS

SEQ ID NO: 44 - protein, 17 aa, synthetic construct
VRWYRQRPGKQREWVAG

SEQ ID NO: 45 - protein, 38 aa, synthetic construct
YYADSVKGRFTISRDNAKNTVYLQMNSLKPEDTAVYYC

SEQ ID NO: 46 - protein, 38 aa, synthetic construct
NYADSMKGRFTISRDNTKNAVYLQIDSLKPEDTAVYYC

SEQ ID NO: 47 - protein, 38 aa, synthetic construct
NYPDSAKGRFTISRDNAKNTVYLQIDSLKPEDTAVYYC

SEQ ID NO: 48 - protein, 38 aa, synthetic construct
YAISSVKGRFTISRDNAENTVFLQMNSLKPDDTAVYYC

SEQ ID NO: 49 - protein, 38 aa, synthetic construct
NYPDSMKGRFTISRDNAKNTVYLQINSLKSEDTAVYYC

SEQ ID NO: 50 - protein, 11 aa, synthetic construct
WGQGTQVTVSS

SEQ ID NO: 51 - protein, 25 aa, synthetic construct
AAAEQKLISEEDLNGAAHHHHHHGS

SEQ ID NO: 52 - DNA, 411 bp, synthetic construct
  source 1..411: mol_type = other DNA
gaggtgcagctggtggagtctgggggaggcgtggtgcagcctggggggtctctaaaactctcctgcgtagcctcgggaacggacttcagtatcaattttatacgctggtaccgccaggctccagggaagcagcgcgagttcgtcgcaggatttactgcgactggtaacacaaactatgcagactccatgaaggggcgattcaccatctccagagacaacaccaagaacgcggtgtatctgcaaatagacagcctgaaacctgaggacacggccgtgtattactgctatatgttggacaagtggggccaggggacccaggtcaccgtctcctcagcggccgcagaacaaaaactcatctcagaagaggatctgaatggggccgcacatcaccaccatcaccatgggagctag

SEQ ID NO: 53 - DNA, 411 bp, synthetic construct
  source 1..411: mol_type = other DNA
gaggtgcagctggtggagtctgggggaggcgtggtgcagcctggggggtctctaaaactctcctgcgtagcctcgggagcggacttcagtatcaattttatacgctggtaccgccaggctccagggaagcagcgcgagttcgtcgcaggatttactgcgactggtaacacaaactatgcagactccatgaaggggcgattcaccatctccagagacaacaccaagaacgcggtgtatctgcaaatagacagcctgaaacctgaggacacggccgtgtattactgctatatgttggacaagtggggccaggggacccaggtcaccgtctcctcagcggccgcagaacaaaaactcatctcagaagaggatctgaatggggccgcacatcaccaccatcaccatgggagctag

SEQ ID NO: 54 - DNA, 411 bp, synthetic construct
  source 1..411: mol_type = other DNA
gaggtgcagctggtggagtctgggggaggcgtggtgcagcctggggggtctctaaaactctcctgcgtagcctcgggaacggcgttcagtatcaattttatacgctggtaccgccaggctccagggaagcagcgcgagttcgtcgcaggatttactgcgactggtaacacaaactatgcagactccatgaaggggcgattcaccatctccagagacaacaccaagaacgcggtgtatctgcaaatagacagcctgaaacctgaggacacggccgtgtattactgctatatgttggacaagtggggccaggggacccaggtcaccgtctcctcagcggccgcagaacaaaaactcatctcagaagaggatctgaatggggccgcacatcaccaccatcaccatgggagctag

SEQ ID NO: 55 - DNA, 411 bp, synthetic construct
  source 1..411: mol_type = other DNA
gaggtgcagctggtggagtctgggggaggcgtggtgcagcctggggggtctctaaaactctcctgcgtagcctcgggaacggacttcagtatcaattttatacgctggtaccgccaggctccagggaagcagcgcgagttcgtcgcaggatttactgcggcgggtaacacaaactatgcagactccatgaaggggcgattcaccatctccagagacaacaccaagaacgcggtgtatctgcaaatagacagcctgaaacctgaggacacggccgtgtattactgctatatgttggacaagtggggccaggggacccaggtcaccgtctcctcagcggccgcagaacaaaaactcatctcagaagaggatctgaatggggccgcacatcaccaccatcaccatgggagctag

SEQ ID NO: 56 - DNA, 411 bp, synthetic construct
  source 1..411: mol_type = other DNA
gaggtgcagctggtggagtctgggggaggcgtggtgcagcctggggggtctctaaaactctcctgcgtagcctcgggaacggacttcagtatcaattttatacgctggtaccgccaggctccagggaagcagcgcgagttcgtcgcaggatttactgcgactggtgcgacaaactatgcagactccatgaaggggcgattcaccatctccagagacaacaccaagaacgcggtgtatctgcaaatagacagcctgaaacctgaggacacggccgtgtattactgctatatgttggacaagtggggccaggggacccaggtcaccgtctcctcagcggccgcagaacaaaaactcatctcagaagaggatctgaatggggccgcacatcaccaccatcaccatgggagctag

SEQ ID NO: 57 - DNA, 411 bp, synthetic construct
  source 1..411: mol_type = other DNA
gaggtgcagctggtggagtctgggggaggcgtggtgcagcctggggggtctctaaaactctcctgcgtagcctcgggaacggacttcagtatcaattttatacgctggtaccgccaggctccagggaagcagcgcgagttcgtcgcaggatttactgcgactggtaacacaaactatgcagactccatgaaggggcgattcaccatctccagagacaacaccaagaacgcggtgtatctgcaaatagacagcctgaaacctgaggacacggccgtgtattactgcgcgatgttggacaagtggggccaggggacccaggtcaccgtctcctcagcggccgcagaacaaaaactcatctcagaagaggatctgaatggggccgcacatcaccaccatcaccatgggagctag

SEQ ID NO: 58 - DNA, 411 bp, synthetic construct
  source 1..411: mol_type = other DNA
gaggtgcagctggtggagtctgggggaggcgtggtgcagcctggggggtctctaaaactctcctgcgtagcctcgggaacggacttcagtatcaattttatacgctggtaccgccaggctccagggaagcagcgcgagttcgtcgcaggatttactgcgactggtaacacaaactatgcagactccatgaaggggcgattcaccatctccagagacaacaccaagaacgcggtgtatctgcaaatagacagcctgaaacctgaggacacggccgtgtattactgctatgcgttggacaagtggggccaggggacccaggtcaccgtctcctcagcggccgcagaacaaaaactcatctcagaagaggatctgaatggggccgcacatcaccaccatcaccatgggagctag

SEQ ID NO: 59 - DNA, 411 bp, synthetic construct
  source 1..411: mol_type = other DNA
gaggtgcagctggtggagtctgggggaggcgtggtgcagcctggggggtctctaaaactctcctgcgtagcctcgggaacggacttcagtatcaattttatacgctggtaccgccaggctccagggaagcagcgcgagttcgtcgcaggatttactgcgactggtaacacaaactatgcagactccatgaaggggcgattcaccatctccagagacaacaccaagaacgcggtgtatctgcaaatagacagcctgaaacctgaggacacggccgtgtattactgctatatggcggacaagtggggccaggggacccaggtcaccgtctcctcagcggccgcagaacaaaaactcatctcagaagaggatctgaatggggccgcacatcaccaccatcaccatgggagctag

SEQ ID NO: 60 - DNA, 411 bp, synthetic construct
  source 1..411: mol_type = other DNA
gaggtgcagctggtggagtctgggggaggcgtggtgcagcctggggggtctctaaaactctcctgcgtagcctcgggaacggacttcagtatcaattttatacgctggtaccgccaggctccagggaagcagcgcgagttcgtcgcaggatttactgcgactggtaacacaaactatgcagactccatgaaggggcgattcaccatctccagagacaacaccaagaacgcggtgtatctgcaaatagacagcctgaaacctgaggacacggccgtgtattactgctatatgttggcgaagtggggccaggggacccaggtcaccgtctcctcagcggccgcagaacaaaaactcatctcagaagaggatctgaatggggccgcacatcaccaccatcaccatgggagctag

SEQ ID NO: 61 - DNA, 411 bp, synthetic construct
  source 1..411: mol_type = other DNA
gaggtgcagctggtggagtctgggggaggcgtggtgcagcctggggggtctctaaaactctcctgcgtagcctcgggaacggacttcagtatcaattttatacgctggtaccgccaggctccagggaagcagcgcgagttcgtcgcaggatttactgcgactggtaacacaaactatgcagactccatgaaggggcgattcaccatctccagagacaacaccaagaacgcggtgtatctgcaaatagacagcctgaaacctgaggacacggccgtgtattactgctatatgttggacgcgtggggccaggggacccaggtcaccgtctcctcagcggccgcagaacaaaaactcatctcagaagaggatctgaatggggccgcacatcaccaccatcaccatgggagctag

SEQ ID NO: 62 - DNA, 411 bp, synthetic construct
  source 1..411: mol_type = other DNA
gaggtgcagctggtggagtctgggggaggcgtggtgcagcctggggggtctctgagactctcctgtgcagcctctggagagatcttcagtatcaattttatgcgctggtaccgccaggctccagggaagcagcgcgagtgggtcgcaggttttactagggatggaagcacaaactatccagactccgcgaagggccgattcaccatctctagagacaacgccaagaacacggtgtatctgcaaatagacagcctgaaacctgaggacacggccgtctattattgttatatgttggacacctggggccaggggacccaggtcactgtctcctcagcggccgcagaacaaaaactcatctcagaagaggatctgaatggggccgcacatcaccaccatcaccatgggagctag

SEQ ID NO: 63 - DNA, 429 bp, synthetic construct
  source 1..429: mol_type = other DNA
gaggtgcagctggtggagtctgggggaggcttggtgcagcctgggggttctctgagactctcctgtacagcctctggaggccccatcgagcagtatcccatgggctggttccgccgggccccaggaaaggagcgtgaattggtagcaagtattagccgaagtggagatggcacatactatgcaatctcttccgtgaagggccgattcaccatctctagagacaacgccgagaacacggtatttctgcaaatgaacagcctgaaacctgacgacacggccgtttattactgtggggctggtataaacccaaccaagatctggggccaggggacccaggtcaccgtctcctcagcggccgcagaacaaaaactcatctcagaagaggatctgaatggggccgcacatcaccaccatcaccatgggagctag

SEQ ID NO: 64 - DNA, 411 bp, synthetic construct
  source 1..411: mol_type = other DNA
gaggtgcagctggtggagtctgggggaggcgaggtgcagcctggggggtctctgaaactctcctgtgtagcctctggaaccgacttcagtatcaattttgtgcgctggtaccgtcagcgtccagggaagcagcgcgagtgggtcgcaggatttactgcgaatggtgatacaaactatccagactccatgaaggggcgattcaccatttccagagacaacgccaagaatacggtgtatctacagataaacagcctgaaatctgaggacacggccgtctattattgctatatgttagataattggggccaggggacccaggtcaccgtctcctcagcggccgcagaacaaaaactcatctcagaagaggatctgaatggggccgcacatcaccaccatcaccatgggagctag

SEQ ID NO: 65 - DNA, 31 bp, synthetic construct
  source 1..31: mol_type = other DNA
atatatgaattcggctcgggacggaggacgc

SEQ ID NO: 66 - DNA, 36 bp, synthetic construct
  source 1..36: mol_type = other DNA
ttaattgtcgacagaactcattgtcccaaccgtcac

SEQ ID NO: 67 - protein, 8 aa, synthetic construct
GTDFSLNF

SEQ ID NO: 68 - protein, 136 aa, synthetic construct
EVQLVESGGGVVQPGGSLKLSCVASGTDFSLNFIRWYRQAPGKQREFVAGFTATGNTNYADSMKGRFTISRDNTKNAVYLQIDSLKPEDTAVYYCYMLDKWGQGTQVTVSSAAAEQKLISEEDLNGAAHHHHHHGS

SEQ ID NO: 69 - protein, 8 aa, synthetic construct
GTDFSINY

SEQ ID NO: 70 - protein, 136 aa, synthetic construct
EVQLVESGGGVVQPGGSLKLSCVASGTDFSINYIRWYRQAPGKQREFVAGFTATGNTNYADSMKGRFTISRDNTKNAVYLQIDSLKPEDTAVYYCYMLDKWGQGTQVTVSSAAAEQKLISEEDLNGAAHHHHHHGS

SEQ ID NO: 71 - protein, 7 aa, synthetic construct
ITATGNT

SEQ ID NO: 72 - protein, 136 aa, synthetic construct
EVQLVESGGGVVQPGGSLKLSCVASGTDFSINFIRWYRQAPGKQREFVAGITATGNTNYADSMKGRFTISRDNTKNAVYLQIDSLKPEDTAVYYCYMLDKWGQGTQVTVSSAAAEQKLISEEDLNGAAHHHHHHGS

SEQ ID NO: 73 - protein, 7 aa, synthetic construct
FSATGNT

SEQ ID NO: 74 - protein, 136 aa, synthetic construct
EVQLVESGGGVVQPGGSLKLSCVASGTDFSINFIRWYRQAPGKQREFVAGFSATGNTNYADSMKGRFTISRDNTKNAVYLQIDSLKPEDTAVYYCYMLDKWGQGTQVTVSSAAAEQKLISEEDLNGAAHHHHHHGS

SEQ ID NO: 75 - protein, 7 aa, synthetic construct
FTATGNS

SEQ ID NO: 76 - protein, 136 aa, synthetic construct
EVQLVESGGGVVQPGGSLKLSCVASGTDFSINFIRWYRQAPGKQREFVAGFTATGNSNYADSMKGRFTISRDNTKNAVYLQIDSLKPEDTAVYYCYMLDKWGQGTQVTVSSAAAEQKLISEEDLNGAAHHHHHHGS

SEQ ID NO: 77 - protein, 5 aa, synthetic construct
FMLDK

SEQ ID NO: 78 - protein, 136 aa, synthetic construct
EVQLVESGGGVVQPGGSLKLSCVASGTDFSINFIRWYRQAPGKQREFVAGFTATGNTNYADSMKGRFTISRDNTKNAVYLQIDSLKPEDTAVYYCFMLDKWGQGTQVTVSSAAAEQKLISEEDLNGAAHHHHHHGS

SEQ ID NO: 79 - protein, 5 aa, synthetic construct
YILDK

SEQ ID NO: 80 - protein, 136 aa, synthetic construct
EVQLVESGGGVVQPGGSLKLSCVASGTDFSINFIRWYRQAPGKQREFVAGFTATGNTNYADSMKGRFTISRDNTKNAVYLQIDSLKPEDTAVYYCYILDKWGQGTQVTVSSAAAEQKLISEEDLNGAAHHHHHHGS

SEQ ID NO: 81 - protein, 5 aa, synthetic construct
YMIDK

SEQ ID NO: 82 - protein, 136 aa, synthetic construct
EVQLVESGGGVVQPGGSLKLSCVASGTDFSINFIRWYRQAPGKQREFVAGFTATGNTNYADSMKGRFTISRDNTKNAVYLQIDSLKPEDTAVYYCYMIDKWGQGTQVTVSSAAAEQKLISEEDLNGAAHHHHHHGS

SEQ ID NO: 83 - protein, 5 aa, synthetic construct
YMVDK

SEQ ID NO: 84 - protein, 136 aa, synthetic construct
EVQLVESGGGVVQPGGSLKLSCVASGTDFSINFIRWYRQAPGKQREFVAGFTATGNTNYADSMKGRFTISRDNTKNAVYLQIDSLKPEDTAVYYCYMVDKWGQGTQVTVSSAAAEQKLISEEDLNGAAHHHHHHGS

SEQ ID NO: 85 - protein, 5 aa, synthetic construct
YMLEK

SEQ ID NO: 86 - protein, 136 aa, synthetic construct
EVQLVESGGGVVQPGGSLKLSCVASGTDFSINFIRWYRQAPGKQREFVAGFTATGNTNYADSMKGRFTISRDNTKNAVYLQIDSLKPEDTAVYYCYMLEKWGQGTQVTVSSAAAEQKLISEEDLNGAAHHHHHHGS

SEQ ID NO: 87 - protein, 136 aa, synthetic construct
EVQLVESGGGVVQPGGSLRLSCAASGTDFSINFMSWVRQAPGKGLEWVAGFTATGNTNYADSVKGRFTISRDNAKNTLYLQMNSLRPEDTAVYYCYMLDKWGQGTQVTVSSAAAEQKLISEEDLNGAAHHHHHHGS

SEQ ID NO: 88 - protein, 136 aa, synthetic construct
EVQLVESGGGVVQPGGSLRLSCAASGTDFSINFIRWVRQAPGKQREFVAGFTATGNTNYADSVKGRFTISRDNAKNTLYLQMNSLRPEDTAVYYCYMLDKWGQGTQVTVSSAAAEQKLISEEDLNGAAHHHHHHGS

SEQ ID NO: 89 - protein, 136 aa, synthetic construct
EVQLVESGGGVVQPGGSLRLSCAASGTDFSINFMHWVRQAPGKGLEWVAGFTATGNTNYADSVKGRFTISRDNAKNTLYLQMNSLRPEDTAVYYCYMLDKWGQGTQVTVSSAAAEQKLISEEDLNGAAHHHHHHGS

SEQ ID NO: 90 - protein, 136 aa, synthetic construct
EVQLVESGGGVVQPGGSLRLSCAASGTDFSINFMSWVRQAPGKQREFVAGFTATGNTNYADSVKGRFTISRDNAKNTLYLQMNSLRPEDTAVYYCYMLDKWGQGTQVTVSSAAAEQKLISEEDLNGAAHHHHHHGS

SEQ ID NO: 91 - protein, 136 aa, synthetic construct
EVQLVESGGGVVQPGGSLRLSCAASGTDFSINFIRWVRQAPGKGLEWVAGFTATGNTNYADSVKGRFTISRDNAKNTLYLQMNSLRPEDTAVYYCYMLDKWGQGTQVTVSSAAAEQKLISEEDLNGAAHHHHHHGS

SEQ ID NO: 92 - protein, 136 aa, synthetic construct
EVQLVESGGGVVQPGGSLRLSCAASGTDFSINFIHWVRQAPGKGLEWVAGFTATGNTNYADSVKGRFTISRDNAKNTLYLQMNSLRPEDTAVYYCYMLDKWGQGTQVTVSSAAAEQKLISEEDLNGAAHHHHHHGS

SEQ ID NO: 93 - protein, 558 aa, synthetic construct
QVQLQQSGPELVRPGVSVKISCKGSGYTFTDYAMHWVKQSHAKSLEWIGVISTKYGKTNYNQKFKGKATMTVDKSSSTAYMELARLTSEDSAIYYCARGDDGYSWGQGTSVTVSSAKTTPPSVYPLAPGSAAQTNSMVTLGCLVKGYFPEPVTVTWNSGSLSSGVHTFPAVLQSDLYTLSSSVTVPSSTWPSETVTCNVAHPASSTKVDKKIVPRDCGCKPCICTVPEVSSVFIFPPKPKDVLTITLTPKVTCVVVDISKDDPEVQFSWFVDDVEVHTAQTQPREEQFNSTFRSVSELPIMHQDWLNGKEFKCRVNSAAFPAPIEKTISKTKGRPKAPQVYTIPPPKEQMAKDKVSLTCMITDFFPEDITVEWQWNGQPAENYKNTQPIMDTDGSYFVYSKLNVQKSNWEAGNTFTCSVLHEGLHNHHTEKSLSHSPGGGGGMAEVQLVESGGGVVQPGGSLKLSCVASGTDFSINFIRWYRQAPGKQREFVAGFTATGNTNYADSMKGRFTISRDNTKNAVYLQIDSLKPEDTAVYYCYMLDKWGQGTQVTVSSAAA

SEQ ID NO: 94 - protein, 343 aa, synthetic construct
DVVMTQTPLSLPVSLGDQASISCRSGQSLVHSNGNTYLHWYLQKPGQSPKLLIYTVSNRFSGVPDRFSGSGSGSDFTLKISRVEAEDLGVYFCSQNTFVPWTFGGGTKLEIKRADAAPTVSIFPPSSEQLTSGGASVVCFLNNFYPKDINVKWKIDGSERQNGVLNSWTDQDSKDSTYSMSSTLTLTKDEYERHNSYTCEATHKTSTSPIVKSFNRNECSGSGGGGGMAEVQLVESGGGVVQPGGSLKLSCVASGTDFSINFIRWYRQAPGKQREFVAGFTATGNTNYADSMKGRFTISRDNTKNAVYLQIDSLKPEDTAVYYCYMLDKWGQGTQVTVSSAAA

SEQ ID NO: 95 - DNA, 411 bp, synthetic construct
  source 1..411: mol_type = other DNA
gaggtgcagctggtggagtctgggggaggcgtggtgcagcctggggggtctctaaaactctcctgcgtagcctcgggaacggacttcagtctgaattttatacgctggtaccgccaggctccagggaagcagcgcgagttcgtcgcaggatttactgcgactggtaacacaaactatgcagactccatgaaggggcgattcaccatctccagagacaacaccaagaacgcggtgtatctgcaaatagacagcctgaaacctgaggacacggccgtgtattactgctatatgttggacaagtggggccaggggacccaggtcaccgtctcctcagcggccgcagaacaaaaactcatctcagaagaggatctgaatggggccgcacatcaccaccatcaccatgggagctag

SEQ ID NO: 96 - DNA, 411 bp, synthetic construct
  source 1..411: mol_type = other DNA
gaggtgcagctggtggagtctgggggaggcgtggtgcagcctggggggtctctaaaactctcctgcgtagcctcgggaacggacttcagtatcaattacatacgctggtaccgccaggctccagggaagcagcgcgagttcgtcgcaggatttactgcgactggtaacacaaactatgcagactccatgaaggggcgattcaccatctccagagacaacaccaagaacgcggtgtatctgcaaatagacagcctgaaacctgaggacacggccgtgtattactgctatatgttggacaagtggggccaggggacccaggtcaccgtctcctcagcggccgcagaacaaaaactcatctcagaagaggatctgaatggggccgcacatcaccaccatcaccatgggagctag

SEQ ID NO: 97 - DNA, 411 bp, synthetic construct
  source 1..411: mol_type = other DNA
gaggtgcagctggtggagtctgggggaggcgtggtgcagcctggggggtctctaaaactctcctgcgtagcctcgggaacggacttcagtatcaattttatacgctggtaccgccaggctccagggaagcagcgcgagttcgtcgcaggaattactgcgactggtaacacaaactatgcagactccatgaaggggcgattcaccatctccagagacaacaccaagaacgcggtgtatctgcaaatagacagcctgaaacctgaggacacggccgtgtattactgctatatgttggacaagtggggccaggggacccaggtcaccgtctcctcagcggccgcagaacaaaaactcatctcagaagaggatctgaatggggccgcacatcaccaccatcaccatgggagctag

SEQ ID NO: 98 - DNA, 411 bp, synthetic construct
  source 1..411: mol_type = other DNA
gaggtgcagctggtggagtctgggggaggcgtggtgcagcctggggggtctctaaaactctcctgcgtagcctcgggaacggacttcagtatcaattttatacgctggtaccgccaggctccagggaagcagcgcgagttcgtcgcaggattttcagcgactggtaacacaaactatgcagactccatgaaggggcgattcaccatctccagagacaacaccaagaacgcggtgtatctgcaaatagacagcctgaaacctgaggacacggccgtgtattactgctatatgttggacaagtggggccaggggacccaggtcaccgtctcctcagcggccgcagaacaaaaactcatctcagaagaggatctgaatggggccgcacatcaccaccatcaccatgggagctag

SEQ ID NO: 99 - DNA, 411 bp, synthetic construct
  source 1..411: mol_type = other DNA
gaggtgcagctggtggagtctgggggaggcgtggtgcagcctggggggtctctaaaactctcctgcgtagcctcgggaacggacttcagtatcaattttatacgctggtaccgccaggctccagggaagcagcgcgagttcgtcgcaggatttactgcgactggtaactcaaactatgcagactccatgaaggggcgattcaccatctccagagacaacaccaagaacgcggtgtatctgcaaatagacagcctgaaacctgaggacacggccgtgtattactgctatatgttggacaagtggggccaggggacccaggtcaccgtctcctcagcggccgcagaacaaaaactcatctcagaagaggatctgaatggggccgcacatcaccaccatcaccatgggagctag

SEQ ID NO: 100 - DNA, 411 bp, synthetic construct
  source 1..411: mol_type = other DNA
gaggtgcagctggtggagtctgggggaggcgtggtgcagcctggggggtctctaaaactctcctgcgtagcctcgggaacggacttcagtatcaattttatacgctggtaccgccaggctccagggaagcagcgcgagttcgtcgcaggatttactgcgactggtaacacaaactatgcagactccatgaaggggcgattcaccatctccagagacaacaccaagaacgcggtgtatctgcaaatagacagcctgaaacctgaggacacggccgtgtattactgctttatgttggacaagtggggccaggggacccaggtcaccgtctcctcagcggccgcagaacaaaaactcatctcagaagaggatctgaatggggccgcacatcaccaccatcaccatgggagctag

SEQ ID NO: 101 - DNA, 411 bp, synthetic construct
  source 1..411: mol_type = other DNA
gaggtgcagctggtggagtctgggggaggcgtggtgcagcctggggggtctctaaaactctcctgcgtagcctcgggaacggacttcagtatcaattttatacgctggtaccgccaggctccagggaagcagcgcgagttcgtcgcaggatttactgcgactggtaacacaaactatgcagactccatgaaggggcgattcaccatctccagagacaacaccaagaacgcggtgtatctgcaaatagacagcctgaaacctgaggacacggccgtgtattactgctatattttggacaagtggggccaggggacccaggtcaccgtctcctcagcggccgcagaacaaaaactcatctcagaagaggatctgaatggggccgcacatcaccaccatcaccatgggagctag

SEQ ID NO: 102 - DNA, 411 bp, synthetic construct
  source 1..411: mol_type = other DNA
gaggtgcagctggtggagtctgggggaggcgtggtgcagcctggggggtctctaaaactctcctgcgtagcctcgggaacggacttcagtatcaattttatacgctggtaccgccaggctccagggaagcagcgcgagttcgtcgcaggatttactgcgactggtaacacaaactatgcagactccatgaaggggcgattcaccatctccagagacaacaccaagaacgcggtgtatctgcaaatagacagcctgaaacctgaggacacggccgtgtattactgctatatgattgacaagtggggccaggggacccaggtcaccgtctcctcagcggccgcagaacaaaaactcatctcagaagaggatctgaatggggccgcacatcaccaccatcaccatgggagctag

SEQ ID NO: 103 - DNA, 411 bp, synthetic construct
  source 1..411: mol_type = other DNA
gaggtgcagctggtggagtctgggggaggcgtggtgcagcctggggggtctctaaaactctcctgcgtagcctcgggaacggacttcagtatcaattttatacgctggtaccgccaggctccagggaagcagcgcgagttcgtcgcaggatttactgcgactggtaacacaaactatgcagactccatgaaggggcgattcaccatctccagagacaacaccaagaacgcggtgtatctgcaaatagacagcctgaaacctgaggacacggccgtgtattactgctatatggtggacaagtggggccaggggacccaggtcaccgtctcctcagcggccgcagaacaaaaactcatctcagaagaggatctgaatggggccgcacatcaccaccatcaccatgggagctag

SEQ ID NO: 104 - DNA, 411 bp, synthetic construct
  source 1..411: mol_type = other DNA
gaggtgcagctggtggagtctgggggaggcgtggtgcagcctggggggtctctaaaactctcctgcgtagcctcgggaacggacttcagtatcaattttatacgctggtaccgccaggctccagggaagcagcgcgagttcgtcgcaggatttactgcgactggtaacacaaactatgcagactccatgaaggggcgattcaccatctccagagacaacaccaagaacgcggtgtatctgcaaatagacagcctgaaacctgaggacacggccgtgtattactgctatatgttggaaaagtggggccaggggacccaggtcaccgtctcctcagcggccgcagaacaaaaactcatctcagaagaggatctgaatggggccgcacatcaccaccatcaccatgggagctag

SEQ ID NO: 105 - DNA, 411 bp, synthetic construct
  source 1..411: mol_type = other DNA
gaggtgcagctggtggagtctgggggaggcgtggtgcagcctggggggtctctacgtctctcctgcgcagcctcgggaacggacttcagtatcaattttatgagctgggttcgccaggctccagggaagggtctggagtgggtcgcaggatttactgcgactggtaacacaaactatgcagactccgttaaggggcgattcaccatctccagagacaacgcaaagaacaccctgtatctgcaaatgaatagcctgcgtcctgaggacacggccgtgtattactgctatatgttggacaagtggggccaggggacccaggtcaccgtctcctcagcggccgcagaacaaaaactcatctcagaagaggatctgaatggggccgcacatcaccaccatcaccatgggagctag

SEQ ID NO: 106 - DNA, 411 bp, synthetic construct
  source 1..411: mol_type = other DNA
gaggtgcagctggtggagtctgggggaggcgtggtgcagcctggggggtctctacgtctctcctgcgcagcctcgggaacggacttcagtatcaattttatacgctgggttcgccaggctccagggaagcagcgcgagttcgtcgcaggatttactgcgactggtaacacaaactatgcagactccgttaaggggcgattcaccatctccagagacaacgcaaagaacaccctgtatctgcaaatgaatagcctgcgtcctgaggacacggccgtgtattactgctatatgttggacaagtggggccaggggacccaggtcaccgtctcctcagcggccgcagaacaaaaactcatctcagaagaggatctgaatggggccgcacatcaccaccatcaccatgggagctag

SEQ ID NO: 107 - DNA, 411 bp, synthetic construct
  source 1..411: mol_type = other DNA
gaggtgcagctggtggagtctgggggaggcgtggtgcagcctggggggtctctacgtctctcctgcgcagcctcgggaacggacttcagtatcaattttatgcattgggttcgccaggctccagggaagggtctggagtgggtcgcaggatttactgcgactggtaacacaaactatgcagactccgttaaggggcgattcaccatctccagagacaacgcaaagaacaccctgtatctgcaaatgaatagcctgcgtcctgaggacacggccgtgtattactgctatatgttggacaagtggggccaggggacccaggtcaccgtctcctcagcggccgcagaacaaaaactcatctcagaagaggatctgaatggggccgcacatcaccaccatcaccatgggagctag

SEQ ID NO: 108 - DNA, 411 bp, synthetic construct
  source 1..411: mol_type = other DNA
gaggtgcagctggtggagtctgggggaggcgtggtgcagcctggggggtctctacgtctctcctgcgcagcctcgggaacggacttcagtatcaattttatgagctgggttcgccaggctccagggaagcagcgcgagttcgtcgcaggatttactgcgactggtaacacaaactatgcagactccgttaaggggcgattcaccatctccagagacaacgcaaagaacaccctgtatctgcaaatgaatagcctgcgtcctgaggacacggccgtgtattactgctatatgttggacaagtggggccaggggacccaggtcaccgtctcctcagcggccgcagaacaaaaactcatctcagaagaggatctgaatggggccgcacatcaccaccatcaccatgggagctag

SEQ ID NO: 109 - DNA, 411 bp, synthetic construct
  source 1..411: mol_type = other DNA
gaggtgcagctggtggagtctgggggaggcgtggtgcagcctggggggtctctacgtctctcctgcgcagcctcgggaacggacttcagtatcaattttatacgctgggttcgccaggctccagggaagggtctggagtgggtcgcaggatttactgcgactggtaacacaaactatgcagactccgttaaggggcgattcaccatctccagagacaacgcaaagaacaccctgtatctgcaaatgaatagcctgcgtcctgaggacacggccgtgtattactgctatatgttggacaagtggggccaggggacccaggtcaccgtctcctcagcggccgcagaacaaaaactcatctcagaagaggatctgaatggggccgcacatcaccaccatcaccatgggagctag

SEQ ID NO: 110 - DNA, 411 bp, synthetic construct
  source 1..411: mol_type = other DNA
gaggtgcagctggtggagtctgggggaggcgtggtgcagcctggggggtctctacgtctctcctgcgcagcctcgggaacggacttcagtatcaattttatacattgggttcgccaggctccagggaagggtctggagtgggtcgcaggatttactgcgactggtaacacaaactatgcagactccgttaaggggcgattcaccatctccagagacaacgcaaagaacaccctgtatctgcaaatgaatagcctgcgtcctgaggacacggccgtgtattactgctatatgttggacaagtggggccaggggacccaggtcaccgtctcctcagcggccgcagaacaaaaactcatctcagaagaggatctgaatggggccgcacatcaccaccatcaccatgggagctag

SEQ ID NO: 111 - protein, 6 aa, synthetic construct
GGGLQR

SEQ ID NO: 112 - protein, 15 aa, synthetic construct
AAAHHHHHHGGGLQR

SEQ ID NO: 113 - protein, 7 aa, synthetic construct
WTATGNT

SEQ ID NO: 114 - protein, 136 aa, synthetic construct
EVQLVESGGGVVQPGGSLKLSCVASGTDFSINFIRWYRQAPGKQREFVAGWTATGNTNYADSMKGRFTISRDNTKNAVYLQIDSLKPEDTAVYYCYMLDKWGQGTQVTVSSAAAEQKLISEEDLNGAAHHHHHHGS

SEQ ID NO: 115 - protein, 7 aa, synthetic construct
YTATGNT

SEQ ID NO: 116 - protein, 136 aa, synthetic construct
EVQLVESGGGVVQPGGSLKLSCVASGTDFSINFIRWYRQAPGKQREFVAGYTATGNTNYADSMKGRFTISRDNTKNAVYLQIDSLKPEDTAVYYCYMLDKWGQGTQVTVSSAAAEQKLISEEDLNGAAHHHHHHGS

SEQ ID NO: 117 - protein, 5 aa, synthetic construct
HMLDK

SEQ ID NO: 118 - protein, 136 aa, synthetic construct
EVQLVESGGGVVQPGGSLKLSCVASGTDFSINFIRWYRQAPGKQREFVAGFTATGNTNYADSMKGRFTISRDNTKNAVYLQIDSLKPEDTAVYYCHMLDKWGQGTQVTVSSAAAEQKLISEEDLNGAAHHHHHHGS

SEQ ID NO: 119 - protein, 5 aa, synthetic construct
WMLDK

SEQ ID NO: 120 - protein, 136 aa, synthetic construct
EVQLVESGGGVVQPGGSLKLSCVASGTDFSINFIRWYRQAPGKQREFVAGFTATGNTNYADSMKGRFTISRDNTKNAVYLQIDSLKPEDTAVYYCWMLDKWGQGTQVTVSSAAAEQKLISEEDLNGAAHHHHHHGS

SEQ ID NO: 121 - protein, 5 aa, synthetic construct
YLLDK

SEQ ID NO: 122 - protein, 136 aa, synthetic construct
EVQLVESGGGVVQPGGSLKLSCVASGTDFSINFIRWYRQAPGKQREFVAGFTATGNTNYADSMKGRFTISRDNTKNAVYLQIDSLKPEDTAVYYCYLLDKWGQGTQVTVSSAAAEQKLISEEDLNGAAHHHHHHGS

SEQ ID NO: 123 - protein, 5 aa, synthetic construct
YVLDK

SEQ ID NO: 124 - protein, 136 aa, synthetic construct
EVQLVESGGGVVQPGGSLKLSCVASGTDFSINFIRWYRQAPGKQREFVAGFTATGNTNYADSMKGRFTISRDNTKNAVYLQIDSLKPEDTAVYYCYVLDKWGQGTQVTVSSAAAEQKLISEEDLNGAAHHHHHHGS

SEQ ID NO: 125 - protein, 8 aa, synthetic construct
GADFSINY

SEQ ID NO: 126 - protein, 136 aa, synthetic construct
EVQLVESGGGVVQPGGSLKLSCVASGADFSINYIRWYRQAPGKQREFVAGFTATGNTNYADSMKGRFTISRDNTKNAVYLQIDSLKPEDTAVYYCYMLDKWGQGTQVTVSSAAAEQKLISEEDLNGAAHHHHHHGS

SEQ ID NO: 127 - protein, 136 aa, synthetic construct
EVQLVESGGGVVQPGGSLKLSCVASGADFSINFIRWYRQAPGKQREFVAGFSATGNTNYADSMKGRFTISRDNTKNAVYLQIDSLKPEDTAVYYCYMLDKWGQGTQVTVSSAAAEQKLISEEDLNGAAHHHHHHGS

SEQ ID NO: 128 - protein, 7 aa, synthetic construct
FTATGHT

SEQ ID NO: 129 - protein, 136 aa, synthetic construct
EVQLVESGGGVVQPGGSLKLSCVASGADFSINFIRWYRQAPGKQREFVAGFTATGHTNYADSMKGRFTISRDNTKNAVYLQIDSLKPEDTAVYYCYMLDKWGQGTQVTVSSAAAEQKLISEEDLNGAAHHHHHHGS

SEQ ID NO: 130 - protein, 136 aa, synthetic construct
EVQLVESGGGVVQPGGSLKLSCVASGTDFSINFIRWVRQAPGKGLEWVAGFTATGNTNYADSMKGRFTISRDNTKNALYLQIDSLRPEDTAVYYCYMLDKWGQGTQVTVSSAAAEQKLISEEDLNGAAHHHHHHGS

SEQ ID NO: 131 - protein, 136 aa, synthetic construct
EVQLVESGGGVVQPGGSLRLSCAASGTDFSINFIRWVRQAPGKGLEWVAGFTATGNTNYADSVKGRFTISRDNTKNTLYLQIDSLRPEDTAVYYCYMLDKWGQGTQVTVSSAAAEQKLISEEDLNGAAHHHHHHGS

SEQ ID NO: 132 - protein, 136 aa, synthetic construct
EVQLVESGGGVVQPGGSLRLSCAASGTDFSINFIRWYRQAPGKGLEFVAGFTATGNTNYADSVKGRFTISRDNAKNTLYLQMNSLRPEDTAVYYCYMLDKWGQGTQVTVSSAAAEQKLISEEDLNGAAHHHHHHGS

SEQ ID NO: 133 - protein, 136 aa, synthetic construct
EVQLVESGGGVVQPGGSLKLSCAASGTDFSINFIRWVRQAPGKGLEWVAGFTATGNTNYADSVKGRFTISRDNTKNTLYLQINSLRPEDTAVYYCYMLDKWGQGTQVTVSSAAAEQKLISEEDLNGAAHHHHHHGS

SEQ ID NO: 134 - protein, 136 aa, synthetic construct
EVQLVESGGGVVQPGGSLRLSCAASGTDFSINFIRWVRQAPGKGLEWVAGFTATGNTNYADSMKGRFTISRDNTKNTLYLQMNSLRPEDTAVYYCYMLDKWGQGTQVTVSSAAAEQKLISEEDLNGAAHHHHHHGS

SEQ ID NO: 135 - protein, 136 aa, synthetic construct
EVQLVESGGGVVQPGGSLRLSCAASGTDFSINFIRWYRQAPGKGLEFVAGFTATGNTNYADSVKGRFTISRDNAKNTLYLQIDSLRPEDTAVYYCYMLDKWGQGTQVTVSSAAAEQKLISEEDLNGAAHHHHHHGS

SEQ ID NO: 136 - protein, 136 aa, synthetic construct
EVQLVESGGGVVQPGGSLRLSCAASGTDFSINFIRWYRQAPGKGLEFVAGFTATGNTNYADSVKGRFTISRDNTKNTLYLQMNSLRPEDTAVYYCYMLDKWGQGTQVTVSSAAAEQKLISEEDLNGAAHHHHHHGS

SEQ ID NO: 137 - protein, 136 aa, synthetic construct
EVQLVESGGGVVQPGGSLRLSCAASGTDFSINFIRWVRQAPGKGLEWVAGFTATGNTNYADSVKGRFTISRDNTKNALYLQMNSLRPEDTAVYYCYMLDKWGQGTQVTVSSAAAEQKLISEEDLNGAAHHHHHHGS

SEQ ID NO: 138 - protein, 136 aa, synthetic construct
EVQLVESGGGVVQPGGSLRLSCVASGTDFSINFIRWVRQAPGKGLEWVAGFTATGNTNYADSVKGRFTISRDNTKNTLYLQMDSLRPEDTAVYYCYMLDKWGQGTQVTVSSAAAEQKLISEEDLNGAAHHHHHHGS

SEQ ID NO: 139 - protein, 136 aa, synthetic construct
EVQLVESGGGLVQPGGSLRLSCAASGTDFSINFIRWYRQAPGKGLEFVAGFTATGNTNYADSVKGRFTISRDNSKNTLYLQMNSLRAEDTAVYYCYMLDKWGQGTLVTVSSAAAEQKLISEEDLNGAAHHHHHHGS

SEQ ID NO: 140 - protein, 136 aa, synthetic construct
EVQLVESGGGVVQPGGSLKLSCVASGTDFSINFIRWVRQAPGKGLEFVAGFTATGNTNYADSMKGRFTISRDNTKNALYLQIDSLRPEDTAVYYCYMLDKWGQGTQVTVSSAAAEQKLISEEDLNGAAHHHHHHGS

SEQ ID NO: 141 - protein, 136 aa, synthetic construct
EVQLVESGGGVVQPGGSLKLSCVASGTDFSINFIRWYRQAPGKGLEFVAGFTATGNTNYADSVKGRFTISRDNAKNTLYLQMNSLRPEDTAVYYCYMLDKWGQGTQVTVSSAAAEQKLISEEDLNGAAHHHHHHGS

SEQ ID NO: 142 - protein, 136 aa, synthetic construct
EVQLVESGGGVVQPGGSLRLSCAASGTDFSINFIRWYRQAPGKQREFVAGFTATGNTNYADSVKGRFTISRDNAKNTLYLQMNSLRPEDTAVYYCYMLDKWGQGTQVTVSSAAAEQKLISEEDLNGAAHHHHHHGS

SEQ ID NO: 143 - protein, 136 aa, synthetic construct
EVQLVESGGGVVQPGGSLRLSCAASGTDFSINFIRWYRQAPGKGLEFVAGFTATGNTNYADSVKGRFTISRDNAKNAVYLQMNSLRPEDTAVYYCYMLDKWGQGTQVTVSSAAAEQKLISEEDLNGAAHHHHHHGS

SEQ ID NO: 144 - protein, 136 aa, synthetic construct
EVQLVESGGGVVQPGGSLRLSCAASGTDFSINFIRWYRQAPGKGLEFVAGFTATGNTNYADSVKGRFTISRDNAKNTLYLQMNSLKPEDTAVYYCYMLDKWGQGTQVTVSSAAAEQKLISEEDLNGAAHHHHHHGS

SEQ ID NO: 145 - protein, 136 aa, synthetic construct
EVQLVESGGGVVQPGGSLRLSCAASGTDFSINFIRWYRQAPGKGREFVAGFTATGNTNYADSVKGRFTISRDNAKNTLYLQMNSLRPEDTAVYYCYMLDKWGQGTQVTVSSAAAEQKLISEEDLNGAAHHHHHHGS

SEQ ID NO: 146 - protein, 136 aa, synthetic construct; identical to SEQ ID NO: 88

SEQ ID NO: 147 - protein, 136 aa, synthetic construct
EVQLVESGGGVVQPGGSLRLSCAASGTDFSINFIRWYRQAPGKGLEFVAGFTATGNTNYADSMKGRFTISRDNAKNTLYLQMNSLRPEDTAVYYCYMLDKWGQGTQVTVSSAAAEQKLISEEDLNGAAHHHHHHGS

SEQ ID NO: 148 - protein, 136 aa, synthetic construct
EVQLVESGGGVVQPGGSLRLSCAASGTDFSINFIRWVRQAPGKGLEFVAGFTATGNTNYADSVKGRFTISRDNAKNTLYLQIDSLRPEDTAVYYCYMLDKWGQGTQVTVSSAAAEQKLISEEDLNGAAHHHHHHGS

SEQ ID NO: 149 - protein, 136 aa, synthetic construct
EVQLVESGGGVVQPGGSLRLSCAASGTDFSINFIRWYRQAPGKGLEWVAGFTATGNTNYADSVKGRFTISRDNAKNTLYLQIDSLRPEDTAVYYCYMLDKWGQGTQVTVSSAAAEQKLISEEDLNGAAHHHHHHGS

SEQ ID NO: 150 - protein, 5 aa, synthetic construct
AMADK

SEQ ID NO: 151 - protein, 136 aa, synthetic construct
EVQLVESGGGVVQPGGSLKLSCVASGTDFSINFIRWYRQAPGKQREFVAGFTATGNTNYADSMKGRFTISRDNTKNAVYLQIDSLKPEDTAVYYCAMADKWGQGTQVTVSSAAAEQKLISEEDLNGAAHHHHHHGS

SEQ ID NO: 152 - protein, 136 aa, synthetic construct
EVQLVESGGGVVQPGGSLRLSCAASGEIFSINFMRWYRQAPGKGLEWVAGFTRDGSTNYPDSVKGRFTISRDNAKNTVYLQMNSLRPEDTAVYYCYMLDTWGQGTQVTVSSAAAEQKLISEEDLNGAAHHHHHHGS

SEQ ID NO: 153 - protein, 136 aa, synthetic construct
EVQLVESGGGVVQPGGSLRLSCAASGTDFSINFIRWYRQAPGKGLEFVAGFSATGNTNYADSVKGRFTISRDNAKNAVYLQMNSLRPEDTAVYYCYMLDKWGQGTQVTVSSAAAEQKLISEEDLNGAAHHHHHHGS

SEQ ID NO: 154 - protein, 136 aa, synthetic construct
EVQLVESGGGVVQPGGSLRLSCAASGTDFSINFIRWYRQAPGKGLEFVAGFTATGNTNYADSVKGRFTISRDNAKNAVYLQMNSLRPEDTAVYYCYILDKWGQGTQVTVSSAAAEQKLISEEDLNGAAHHHHHHGS

SEQ ID NO: 155 - protein, 136 aa, synthetic construct
EVQLVESGGGVVQPGGSLRLSCAADGEIFSINFMRWYRQAPGKQREWVAGFTRDGSTNYPDSAKGRFTISRDNAKNTVYLQIDSLKPEDTAVYYCYMLDTWGQGTQVTVSSAAAEQKLISEEDLNGAAHHHHHHGS

SEQ ID NO: 156 - protein, 136 aa, synthetic construct
EVQLVESGGGVVQPGGSLRLSCAASGEIFSINFMRWYGQAPGKQREWVAGFTRDGSTNYPDSAKGRFTISRDNAKNTVYLQIDSLKPEDTAVYYCYMLDTWGQGTQVTVSSAAAEQKLISEEDLNGAAHHHHHHGS

SEQ ID NO: 157 - protein, 136 aa, synthetic construct
EVQLVESGGGVVQPGGSLRLSCAASGEIFSINFMRWYREAPGKQREWVAGFTRDGSTNYPDSAKGRFTISRDNAKNTVYLQIDSLKPEDTAVYYCYMLDTWGQGTQVTVSSAAAEQKLISEEDLNGAAHHHHHHGS

SEQ ID NO: 158 - protein, 136 aa, synthetic construct
EVQLVESGGGVVQPGGSLRLSCAASGEIFSINFMRWYRQAPIKQREWVAGFTRDGSTNYPDSAKGRFTISRDNAKNTVYLQIDSLKPEDTAVYYCYMLDTWGQGTQVTVSSAAAEQKLISEEDLNGAAHHHHHHGS

SEQ ID NO: 159 - protein, 136 aa, synthetic construct
EVQLVESGGGVVQPGGSLRLSCAASGEIFSINFMRWYRQAPGKIREWVAGFTRDGSTNYPDSAKGRFTISRDNAKNTVYLQIDSLKPEDTAVYYCYMLDTWGQGTQVTVSSAAAEQKLISEEDLNGAAHHHHHHGS

SEQ ID NO: 160 - protein, 7 aa, synthetic construct
FTRDGFT

SEQ ID NO: 161 - protein, 136 aa, synthetic construct
EVQLVESGGGVVQPGGSLRLSCAASGEIFSINFMRWYRQAPGKQREWVAGFTRDGFTNYPDSAKGRFTISRDNAKNTVYLQIDSLKPEDTAVYYCYMLDTWGQGTQVTVSSAAAEQKLISEEDLNGAAHHHHHHGS

SEQ ID NO: 162 - protein, 7 aa, synthetic construct
FTRDGYT

SEQ ID NO: 163 - protein, 136 aa, synthetic construct
EVQLVESGGGVVQPGGSLRLSCAASGEIFSINFMRWYRQAPGKQREWVAGFTRDGYTNYPDSAKGRFTISRDNAKNTVYLQIDSLKPEDTAVYYCYMLDTWGQGTQVTVSSAAAEQKLISEEDLNGAAHHHHHHGS

SEQ ID NO: 164 - protein, 7 aa, synthetic construct
FTRDGSL

SEQ ID NO: 165 - protein, 136 aa, synthetic construct
EVQLVESGGGVVQPGGSLRLSCAASGEIFSINFMRWYRQAPGKQREWVAGFTRDGSLNYPDSAKGRFTISRDNAKNTVYLQIDSLKPEDTAVYYCYMLDTWGQGTQVTVSSAAAEQKLISEEDLNGAAHHHHHHGS

SEQ ID NO: 166 - protein, 7 aa, synthetic construct
FTRDGSK

SEQ ID NO: 167 - protein, 136 aa, synthetic construct
EVQLVESGGGVVQPGGSLRLSCAASGEIFSINFMRWYRQAPGKQREWVAGFTRDGSKNYPDSAKGRFTISRDNAKNTVYLQIDSLKPEDTAVYYCYMLDTWGQGTQVTVSSAAAEQKLISEEDLNGAAHHHHHHGS

SEQ ID NO: 168 - protein, 142 aa, synthetic construct
EVQLVESGGGLVQPGGSLRLSCTASGGPIEQYPMGWFRRAPGKERNLVASISRSGDGTYYAISSVKGRFTISRDNAENTVFLQMNSLKPDDTAVYYCGAGINPTKIWGQGTQVTVSSAAAEQKLISEEDLNGAAHHHHHHGS

SEQ ID NO: 169 - protein, 9 aa, synthetic construct
FSRSGDGTY

SEQ ID NO: 170 - protein, 142 aa, synthetic construct
EVQLVESGGGLVQPGGSLRLSCTASGGPIEQYPMGWFRRAPGKERELVASFSRSGDGTYYAISSVKGRFTISRDNAENTVFLQMNSLKPDDTAVYYCGAGINPTKIWGQGTQVTVSSAAAEQKLISEEDLNGAAHHHHHHGS

SEQ ID NO: 171 - protein, 9 aa, synthetic construct
SSRSGDGTY

SEQ ID NO: 172 - protein, 142 aa, synthetic construct
EVQLVESGGGLVQPGGSLRLSCTASGGPIEQYPMGWFRRAPGKERELVASSSRSGDGTYYAISSVKGRFTISRDNAENTVFLQMNSLKPDDTAVYYCGAGINPTKIWGQGTQVTVSSAAAEQKLISEEDLNGAAHHHHHHGS

SEQ ID NO: 173 - protein, 142 aa, synthetic construct
EVQLVESGGGLVQPGGSLRLSCTASGGPIEQYPMGWFRRAPGKERESVASISRSGDGTYYAISSVKGRFTISRDNAENTVFLQMNSLKPDDTAVYYCGAGINPTKIWGQGTQVTVSSAAAEQKLISEEDLNGAAHHHHHHGS

SEQ ID NO: 174 - protein, 142 aa, synthetic construct
EVQLVESGGGLVQPGGSLRLSCTASGGPIEQYPMGWFRRAPGKERELQASISRSGDGTYYAISSVKGRFTISRDNAENTVFLQMNSLKPDDTAVYYCGAGINPTKIWGQGTQVTVSSAAAEQKLISEEDLNGAAHHHHHHGS

SEQ ID NO: 175 - protein, 8 aa, synthetic construct
GRPLSDYP

SEQ ID NO: 176 - protein, 8 aa, synthetic construct
ISRTGDGT

SEQ ID NO: 177 - protein, 9 aa, synthetic construct
GAGINPTKY

SEQ ID NO: 178 - protein, 141 aa, synthetic construct
QVQLVQSGGGLVQAGGSLTLSCTASGRPLSDYPMGWFRRAPEKERELVASISRTGDGTYYADGMRGRFTISRDNSENTVSLQMNNLKPEDTAVYYCGAGINPTKYWGQGTQVTVSSAAAEQKLISEEDLNGAAHHHHHHGS

SEQ ID NO: 179 - protein, 8 aa, synthetic construct
GRPISDYP

SEQ ID NO: 180 - protein, 9 aa, synthetic construct
GAGINPTRY

SEQ ID NO: 181 - protein, 141 aa, synthetic construct
EVQLVESGGGLVQAGGSLRLSCTASGRPISDYPMGWFRRAPGKDRELVASISRTGDGTYYANSMKERFTISRDNAQNTVSLQISSLKPEDTAVYYCGAGINPTRYWGQGTQVTVSSAAAEQKLISEEDLNGAAHHHHHHGS

SEQ ID NO: 182 - protein, 8 aa, synthetic construct
GFTFSAYA

SEQ ID NO: 183 - protein, 141 aa, synthetic construct
QVQLVQSGGGLVQPGGSLRLSCAASGFTFSAYAMSWVRQAPGKGRELVASISRTGDGTYYADGMKGRFTISRDNAENTVSLQINSLKPEDTAIYYCGAGINPTKYWGQGTQVTVSSAAAEQKLISEEDLNGAAHHHHHHGS

SEQ ID NO: 184 - protein, 8 aa, synthetic construct
GLPLSNYP

SEQ ID NO: 185 - protein, 142 aa, synthetic construct
EVQLVESGGGLVQAGDSLRLSCTASGLPLSNYPMGWFRRAPGKERELIASISRTGDGTYYADSSVKGRFTISRDNAENTVSLQMNSLKPEDTAVYYCGAGINPTKYWGQGTQVTVSSAAAEQKLISEEDLNGAAHHHHHHGS

SEQ ID NO: 186 - protein, 8 aa, synthetic construct
GSIFSDIT

SEQ ID NO: 187 - protein, 7 aa, synthetic construct
ISRSGSP

SEQ ID NO: 188 - protein, 5 aa, synthetic construct
YSRGY

SEQ ID NO: 189 - protein, 136 aa, synthetic construct
QVQLVQSGGGLVQAGGSLRLSCAASGSIFSDITLAWHRQIPGKEREWVAGISRSGSPSYRDSVKGRFTISRDNAKNTVFLQMNSLEPEDTGVYYCYSRGYWGQGTQVTVSSAAAEQKLISEEDLNGAAHHHHHHGS

SEQ ID NO: 190 - protein, 8 aa, synthetic construct
GRDFSDTS

SEQ ID NO: 191 - protein, 8 aa, synthetic construct
IRSGSTST

SEQ ID NO: 192 - protein, 5 aa, synthetic construct
YSKGY

SEQ ID NO: 193 - protein, 137 aa, synthetic construct
EVQLVQSGGGLVQAGGSLRLSCAASGRDFSDTSMAWHRQAPGKERLWVAGIRSGSTSTSYADSVKGRFTISRDDAKNTVYLQMDNLTPEDTAVYFCYSKGYWGQGTQVTVSSAAAEQKLISEEDLNGAAHHHHHHGS

SEQ ID NO: 194 - protein, 7 aa, synthetic construct
ESISIYG

SEQ ID NO: 195 - protein, 7 aa, synthetic construct
LKRNGLT

SEQ ID NO: 196 - protein, 9 aa, synthetic construct
NTALGSVLP

SEQ ID NO: 197 - protein, 139 aa, synthetic construct
EVQLVESGGGLVQPGESLRLSCTASESISIYGVGWYRQAPGEQRVLVAHLKRNGLTEYKDSVKGRFTISRDNARNTIYLEMKNLKPEDTAIYYCNTALGSVLPWGRGTQVTVSSAAAEQKLISEEDLNGAAHHHHHHGS

SEQ ID NO: 198 - protein, 7 aa, synthetic construct
ATFGGYS

SEQ ID NO: 199 - protein, 9 aa, synthetic construct
ITWNGGIIK

SEQ ID NO: 200 - protein, 21 aa, synthetic construct
AGDRTYYAGGYVPTSEREYAF

SEQ ID NO: 201 - protein, 8 aa, synthetic construct
GSIFLIND

SEQ ID NO: 202 - protein, 5 aa, synthetic construct
RGGST

SEQ ID NO: 203 - protein, 11 aa, synthetic construct
HRESGLGSSEY

SEQ ID NO: 204 - protein, 140 aa, synthetic construct
QVQLVQSGGGLVQAGGSLRLSCAASGSIFLINDMGWYRQAPGKQRELVAVRGGSTKYGDSVKGRFTISRDDAKNTVYLQMNSLKPEDTAVYYCHRESGLGSSEYWGQGTQVTVSSAAAEQKLISEEDLNGAAHHHHHHGS

SEQ ID NO: 205 - protein, 8 aa, synthetic construct
GRTVSNYR

SEQ ID NO: 206 - protein, 8 aa, synthetic construct
IAWAGGSL

SEQ ID NO: 207 - protein, 11 aa, synthetic construct
KGSRIFPTRDY

SEQ ID NO: 208 - protein, 143 aa, synthetic construct
EVQLVESGGGLVQAGGSLRLSCTASGRTVSNYRMGWFRQTPGKEREFVAAIAWAGGSLTYADSVKGRFTISRDNAKNTVYLQMNSLEPTDTAVYYCKGSRIFPTRDYWGKGTQVTVSSAAAEQKLISEEDLNGAAHHHHHHGS

SEQ ID NO: 209 - protein, 8 aa, synthetic construct
GFTFGSYV

SEQ ID NO: 210 - protein, 8 aa, synthetic construct
VSSGGGTT

SEQ ID NO: 211 - protein, 12 aa, synthetic construct
ATGRTGLGEGDH

SEQ ID NO: 212 - protein, 143 aa, synthetic construct
EVQLVESGGGLVQPGGSLRLSCAASGFTFGSYVMSWVRQAPGKGPEWVSTVSSGGGTTYYADSVKGRFTISRDNAQNTLYLQMNSLKPEDTAVYYCATGRTGLGEGDHRGQGTQVTSSAAAEQKLISEEDLNGAAHHHHHHGS

SEQ ID NO: 213 - protein, 111 aa, synthetic construct
EVQLVESGGGVVQPGGSLKLSCVASGTDFSINFIRWYRQAPGKQREFVAGFTATGNTNYADSMKGRFTISRDNTKNAVYLQIDSLKPEDTAVYYCYMLDKWGQGTQVTVSS

SEQ ID NO: 214 - protein, 111 aa, synthetic construct
EVQLVESGGGVVQPGGSLRLSCAASGEIFSINFMRWYRQAPGKQREWVAGFTRDGSTNYPDSAKGRFTISRDNAKNTVYLQIDSLKPEDTAVYYCYMLDTWGQGTQVTVSS

SEQ ID NO: 215 - protein, 117 aa, synthetic construct
EVQLVESGGGLVQPGGSLRLSCTASGGPIEQYPMGWFRRAPGKERELVASISRSGDGTYYAISSVKGRFTISRDNAENTVFLQMNSLKPDDTAVYYCGAGINPTKIWGQGTQVTVSS

SEQ ID NO: 216 - protein, 111 aa, synthetic construct
EVQLVESGGGEVQPGGSLKLSCVASGTDFSINFVRWYRQRPGKQREWVAGFTANGDTNYPDSMKGRFTISRDNAKNTVYLQINSLKSEDTAVYYCYMLDNWGQGTQVTVSS

SEQ ID NO: 217 - protein, 111 aa, synthetic construct
EVQLVESGGGVVQPGGSLKLSCVASGADFSINFIRWYRQAPGKQREFVAGFTATGNTNYADSMKGRFTISRDNTKNAVYLQIDSLKPEDTAVYYCYMLDKWGQGTQVTVSS

SEQ ID NO: 218 - protein, 111 aa, synthetic construct
EVQLVESGGGVVQPGGSLKLSCVASGTAFSINFIRWYRQAPGKQREFVAGFTATGNTNYADSMKGRFTISRDNTKNAVYLQIDSLKPEDTAVYYCYMLDKWGQGTQVTVSS

SEQ ID NO: 219 - protein, 111 aa, synthetic construct
EVQLVESGGGVVQPGGSLKLSCVASGTDFSINFIRWYRQAPGKQREFVAGFTAAGNTNYADSMKGRFTISRDNTKNAVYLQIDSLKPEDTAVYYCYMLDKWGQGTQVTVSS

SEQ ID NO: 220 - protein, 111 aa, synthetic construct
EVQLVESGGGVVQPGGSLKLSCVASGTDFSINFIRWYRQAPGKQREFVAGFTATGATNYADSMKGRFTISRDNTKNAVYLQIDSLKPEDTAVYYCYMLDKWGQGTQVTVSS

SEQ ID NO: 221 - protein, 111 aa, synthetic construct
EVQLVESGGGVVQPGGSLKLSCVASGTDFSINFIRWYRQAPGKQREFVAGFTATGNTNYADSMKGRFTISRDNTKNAVYLQIDSLKPEDTAVYYCAMLDKWGQGTQVTVSS

SEQ ID NO: 222 - protein, 111 aa, synthetic construct
EVQLVESGGGVVQPGGSLKLSCVASGTDFSINFIRWYRQAPGKQREFVAGFTATGNTNYADSMKGRFTISRDNTKNAVYLQIDSLKPEDTAVYYCYALDKWGQGTQVTVSS

SEQ ID NO: 223 - protein, 111 aa, synthetic construct
EVQLVESGGGVVQPGGSLKLSCVASGTDFSINFIRWYRQAPGKQREFVAGFTATGNTNYADSMKGRFTISRDNTKNAVYLQIDSLKPEDTAVYYCYMADKWGQGTQVTVSS

SEQ ID NO: 224 - protein, 111 aa, synthetic construct
EVQLVESGGGVVQPGGSLKLSCVASGTDFSINFIRWYRQAPGKQREFVAGFTATGNTNYADSMKGRFTISRDNTKNAVYLQIDSLKPEDTAVYYCYMLAKWGQGTQVTVSS

SEQ ID NO: 225 - protein, 111 aa, synthetic construct
EVQLVESGGGVVQPGGSLKLSCVASGTDFSINFIRWYRQAPGKQREFVAGFTATGNTNYADSMKGRFTISRDNTKNAVYLQIDSLKPEDTAVYYCYMLDAWGQGTQVTVSS

SEQ ID NO: 226 - protein, 111 aa, synthetic construct
EVQLVESGGGVVQPGGSLKLSCVASGTDFSLNFIRWYRQAPGKQREFVAGFTATGNTNYADSMKGRFTISRDNTKNAVYLQIDSLKPEDTAVYYCYMLDKWGQGTQVTVSS

SEQ ID NO: 227 - protein, 111 aa, synthetic construct
EVQLVESGGGVVQPGGSLKLSCVASGTDFSINYIRWYRQAPGKQREFVAGFTATGNTNYADSMKGRFTISRDNTKNAVYLQIDSLKPEDTAVYYCYMLDKWGQGTQVTVSS

SEQ ID NO: 228 - protein, 111 aa, synthetic construct
EVQLVESGGGVVQPGGSLKLSCVASGTDFSINFIRWYRQAPGKQREFVAGITATGNTNYADSMKGRFTISRDNTKNAVYLQIDSLKPEDTAVYYCYMLDKWGQGTQVTVSS

SEQ ID NO: 229 - protein, 111 aa, synthetic construct
EVQLVESGGGVVQPGGSLKLSCVASGTDFSINFIRWYRQAPGKQREFVAGFSATGNTNYADSMKGRFTISRDNTKNAVYLQIDSLKPEDTAVYYCYMLDKWGQGTQVTVSS

SEQ ID NO: 230 - protein, 111 aa, synthetic construct
EVQLVESGGGVVQPGGSLKLSCVASGTDFSINFIRWYRQAPGKQREFVAGFTATGNSNYADSMKGRFTISRDNTKNAVYLQIDSLKPEDTAVYYCYMLDKWGQGTQVTVSS

SEQ ID NO: 231 - protein, 111 aa, synthetic construct
EVQLVESGGGVVQPGGSLKLSCVASGTDFSINFIRWYRQAPGKQREFVAGFTATGNTNYADSMKGRFTISRDNTKNAVYLQIDSLKPEDTAVYYCFMLDKWGQGTQVTVSS

SEQ ID NO: 232 - protein, 111 aa, synthetic construct
EVQLVESGGGVVQPGGSLKLSCVASGTDFSINFIRWYRQAPGKQREFVAGFTATGNTNYADSMKGRFTISRDNTKNAVYLQIDSLKPEDTAVYYCYILDKWGQGTQVTVSS

SEQ ID NO: 233 - protein, 111 aa, synthetic construct
EVQLVESGGGVVQPGGSLKLSCVASGTDFSINFIRWYRQAPGKQREFVAGFTATGNTNYADSMKGRFTISRDNTKNAVYLQIDSLKPEDTAVYYCYMIDKWGQGTQVTVSS

SEQ ID NO: 234 - protein, 111 aa, synthetic construct
EVQLVESGGGVVQPGGSLKLSCVASGTDFSINFIRWYRQAPGKQREFVAGFTATGNTNYADSMKGRFTISRDNTKNAVYLQIDSLKPEDTAVYYCYMVDKWGQGTQVTVSS

SEQ ID NO: 235 - protein, 111 aa, synthetic construct
EVQLVESGGGVVQPGGSLKLSCVASGTDFSINFIRWYRQAPGKQREFVAGFTATGNTNYADSMKGRFTISRDNTKNAVYLQIDSLKPEDTAVYYCYMLEKWGQGTQVTVSS

SEQ ID NO: 236 - protein, 111 aa, synthetic construct
EVQLVESGGGVVQPGGSLRLSCAASGTDFSINFMSWVRQAPGKGLEWVAGFTATGNTNYADSVKGRFTISRDNAKNTLYLQMNSLRPEDTAVYYCYMLDKWGQGTQVTVSS

SEQ ID NO: 237 - protein, 111 aa, synthetic construct
EVQLVESGGGVVQPGGSLRLSCAASGTDFSINFIRWVRQAPGKQREFVAGFTATGNTNYADSVKGRFTISRDNAKNTLYLQMNSLRPEDTAVYYCYMLDKWGQGTQVTVSS

SEQ ID NO: 238 - protein, 111 aa, synthetic construct
EVQLVESGGGVVQPGGSLRLSCAASGTDFSINFMHWVRQAPGKGLEWVAGFTATGNTNYADSVKGRFTISRDNAKNTLYLQMNSLRPEDTAVYYCYMLDKWGQGTQVTVSS

SEQ ID NO: 239 - protein, 111 aa, synthetic construct
EVQLVESGGGVVQPGGSLRLSCAASGTDFSINFMSWVRQAPGKQREFVAGFTATGNTNYADSVKGRFTISRDNAKNTLYLQMNSLRPEDTAVYYCYMLDKWGQGTQVTVSS

SEQ ID NO: 240 - protein, 111 aa, synthetic construct
EVQLVESGGGVVQPGGSLRLSCAASGTDFSINFIRWVRQAPGKGLEWVAGFTATGNTNYADSVKGRFTISRDNAKNTLYLQMNSLRPEDTAVYYCYMLDKWGQGTQVTVSS

SEQ ID NO: 241 - protein, 111 aa, synthetic construct
EVQLVESGGGVVQPGGSLRLSCAASGTDFSINFIHWVRQAPGKGLEWVAGFTATGNTNYADSVKGRFTISRDNAKNTLYLQMNSLRPEDTAVYYCYMLDKWGQGTQVTVSS

SEQ ID NO: 242 - protein, 111 aa, synthetic construct
EVQLVESGGGVVQPGGSLKLSCVASGHDFSINFIRWYRQAPGKQREFVAGFTATGNTNYADSMKGRFTISRDNTKNAVYLQIDSLKPEDTAVYYCYMLDKWGQGTQVTVSS

SEQ ID NO: 243 - protein, 111 aa, synthetic construct
EVQLVESGGGVVQPGGSLKLSCVASGTDFSINFIRWYRQAPGKQREFVAGWTATGNTNYADSMKGRFTISRDNTKNAVYLQIDSLKPEDTAVYYCYMLDKWGQGTQVTVSS

SEQ ID NO: 244 - protein, 111 aa, synthetic construct
EVQLVESGGGVVQPGGSLKLSCVASGTDFSINFIRWYRQAPGKQREFVAGYTATGNTNYADSMKGRFTISRDNTKNAVYLQIDSLKPEDTAVYYCYMLDKWGQGTQVTVSS

SEQ ID NO: 245 - protein, 111 aa, synthetic construct
EVQLVESGGGVVQPGGSLKLSCVASGTDFSINFIRWYRQAPGKQREFVAGFTATGNTNYADSMKGRFTISRDNTKNAVYLQIDSLKPEDTAVYYCHMLDKWGQGTQVTVSS

SEQ ID NO: 246 - protein, 111 aa, synthetic construct
EVQLVESGGGVVQPGGSLKLSCVASGTDFSINFIRWYRQAPGKQREFVAGFTATGNTNYADSMKGRFTISRDNTKNAVYLQIDSLKPEDTAVYYCWMLDKWGQGTQVTVSS

SEQ ID NO: 247 - protein, 111 aa, synthetic construct
EVQLVESGGGVVQPGGSLKLSCVASGTDFSINFIRWYRQAPGKQREFVAGFTATGNTNYADSMKGRFTISRDNTKNAVYLQIDSLKPEDTAVYYCYLLDKWGQGTQVTVSS

SEQ ID NO: 248 - protein, 111 aa, synthetic construct
EVQLVESGGGVVQPGGSLKLSCVASGTDFSINFIRWYRQAPGKQREFVAGFTATGNTNYADSMKGRFTISRDNTKNAVYLQIDSLKPEDTAVYYCYVLDKWGQGTQVTVSS

SEQ ID NO: 249 - protein, 111 aa, synthetic construct
EVQLVESGGGVVQPGGSLKLSCVASGADFSINYIRWYRQAPGKQREFVAGFTATGNTNYADSMKGRFTISRDNTKNAVYLQIDSLKPEDTAVYYCYMLDKWGQGTQVTVSS

SEQ ID NO: 250 - protein, 111 aa, synthetic construct
EVQLVESGGGVVQPGGSLKLSCVASGADFSINFIRWYRQAPGKQREFVAGFSATGNTNYADSMKGRFTISRDNTKNAVYLQIDSLKPEDTAVYYCYMLDKWGQGTQVTVSS

SEQ ID NO: 251 - protein, 111 aa, synthetic construct
EVQLVESGGGVVQPGGSLKLSCVASGADFSINFIRWYRQAPGKQREFVAGFTATGHTNYADSMKGRFTISRDNTKNAVYLQIDSLKPEDTAVYYCYMLDKWGQGTQVTVSS

SEQ ID NO: 252 - protein, 111 aa, synthetic construct
EVQLVESGGGVVQPGGSLKLSCVASGTDFSINFIRWVRQAPGKGLEWVAGFTATGNTNYADSMKGRFTISRDNTKNALYLQIDSLRPEDTAVYYCYMLDKWGQGTQVTVSS

SEQ ID NO: 253 - protein, 111 aa, synthetic construct
EVQLVESGGGVVQPGGSLRLSCAASGTDFSINFIRWVRQAPGKGLEWVAGFTATGNTNYADSVKGRFTISRDNTKNTLYLQIDSLRPEDTAVYYCYMLDKWGQGTQVTVSS

SEQ ID NO: 254 - protein, 111 aa, synthetic construct
EVQLVESGGGVVQPGGSLRLSCAASGTDFSINFIRWYRQAPGKGLEFVAGFTATGNTNYADSVKGRFTISRDNAKNTLYLQMNSLRPEDTAVYYCYMLDKWGQGTQVTVSS

SEQ ID NO: 255 - protein, 111 aa, synthetic construct
EVQLVESGGGVVQPGGSLKLSCAASGTDFSINFIRWVRQAPGKGLEWVAGFTATGNTNYADSVKGRFTISRDNTKNTLYLQINSLRPEDTAVYYCYMLDKWGQGTQVTVSS

SEQ ID NO: 256 - protein, 111 aa, synthetic construct
EVQLVESGGGVVQPGGSLRLSCAASGTDFSINFIRWVRQAPGKGLEWVAGFTATGNTNYADSMKGRFTISRDNTKNTLYLQMNSLRPEDTAVYYCYMLDKWGQGTQVTVSS

SEQ ID NO: 257 - protein, 111 aa, synthetic construct
EVQLVESGGGVVQPGGSLRLSCAASGTDFSINFIRWYRQAPGKGLEFVAGFTATGNTNYADSVKGRFTISRDNAKNTLYLQIDSLRPEDTAVYYCYMLDKWGQGTQVTVSS

SEQ ID NO: 258 - protein, 111 aa, synthetic construct
EVQLVESGGGVVQPGGSLRLSCAASGTDFSINFIRWYRQAPGKGLEFVAGFTATGNTNYADSVKGRFTISRDNTKNTLYLQMNSLRPEDTAVYYCYMLDKWGQGTQVTVSS

SEQ ID NO: 259 - protein, 111 aa, synthetic construct
EVQLVESGGGVVQPGGSLRLSCAASGTDFSINFIRWVRQAPGKGLEWVAGFTATGNTNYADSVKGRFTISRDNTKNALYLQMNSLRPEDTAVYYCYMLDKWGQGTQVTVSS

SEQ ID NO: 260 - protein, 111 aa, synthetic construct
EVQLVESGGGVVQPGGSLRLSCVASGTDFSINFIRWVRQAPGKGLEWVAGFTATGNTNYADSVKGRFTISRDNTKNTLYLQMDSLRPEDTAVYYCYMLDKWGQGTQVTVSS

SEQ ID NO: 261 - protein, 111 aa, synthetic construct
EVQLVESGGGLVQPGGSLRLSCAASGTDFSINFIRWYRQAPGKGLEFVAGFTATGNTNYADSVKGRFTISRDNSKNTLYLQMNSLRAEDTAVYYCYMLDKWGQGTLVTVSS

SEQ ID NO: 262 - protein, 111 aa, synthetic construct
EVQLVESGGGVVQPGGSLKLSCVASGTDFSINFIRWVRQAPGKGLEFVAGFTATGNTNYADSMKGRFTISRDNTKNALYLQIDSLRPEDTAVYYCYMLDKWGQGTQVTVSS

SEQ ID NO: 263 - protein, 111 aa, synthetic construct
EVQLVESGGGVVQPGGSLKLSCVASGTDFSINFIRWYRQAPGKGLEFVAGFTATGNTNYADSVKGRFTISRDNAKNTLYLQMNSLRPEDTAVYYCYMLDKWGQGTQVTVSS

SEQ ID NO: 264 - protein, 111 aa, synthetic construct
EVQLVESGGGVVQPGGSLRLSCAASGTDFSINFIRWYRQAPGKQREFVAGFTATGNTNYADSVKGRFTISRDNAKNTLYLQMNSLRPEDTAVYYCYMLDKWGQGTQVTVSS

SEQ ID NO: 265 - protein, 111 aa, synthetic construct
EVQLVESGGGVVQPGGSLRLSCAASGTDFSINFIRWYRQAPGKGLEFVAGFTATGNTNYADSVKGRFTISRDNAKNAVYLQMNSLRPEDTAVYYCYMLDKWGQGTQVTVSS

SEQ ID NO: 266 - protein, 111 aa, synthetic construct
EVQLVESGGGVVQPGGSLRLSCAASGTDFSINFIRWYRQAPGKGLEFVAGFTATGNTNYADSVKGRFTISRDNAKNTLYLQMNSLKPEDTAVYYCYMLDKWGQGTQVTVSS

SEQ ID NO: 267 - protein, 111 aa, synthetic construct
EVQLVESGGGVVQPGGSLRLSCAASGTDFSINFIRWYRQAPGKGREFVAGFTATGNTNYADSVKGRFTISRDNAKNTLYLQMNSLRPEDTAVYYCYMLDKWGQGTQVTVSS

SEQ ID NO: 268 - protein, 111 aa, synthetic construct; identical to SEQ ID NO: 237

SEQ ID NO: 269 - protein, 111 aa, synthetic construct
EVQLVESGGGVVQPGGSLRLSCAASGTDFSINFIRWYRQAPGKGLEFVAGFTATGNTNYADSMKGRFTISRDNAKNTLYLQMNSLRPEDTAVYYCYMLDKWGQGTQVTVSS

SEQ ID NO: 270 - protein, 111 aa, synthetic construct
EVQLVESGGGVVQPGGSLRLSCAASGTDFSINFIRWVRQAPGKGLEFVAGFTATGNTNYADSVKGRFTISRDNAKNTLYLQIDSLRPEDTAVYYCYMLDKWGQGTQVTVSS

SEQ ID NO: 271 - protein, 111 aa, synthetic construct
EVQLVESGGGVVQPGGSLRLSCAASGTDFSINFIRWYRQAPGKGLEWVAGFTATGNTNYADSVKGRFTISRDNAKNTLYLQIDSLRPEDTAVYYCYMLDKWGQGTQVTVSS

SEQ ID NO: 272 - protein, 111 aa, synthetic construct
EVQLVESGGGVVQPGGSLKLSCVASGTDFSINFIRWYRQAPGKQREFVAGFTATGNTNYADSMKGRFTISRDNTKNAVYLQIDSLKPEDTAVYYCAMADKWGQGTQVTVSS

SEQ ID NO: 273 - protein, 111 aa, synthetic construct
EVQLVESGGGVVQPGGSLRLSCAASGEIFSINFMRWYRQAPGKGLEWVAGFTRDGSTNYPDSVKGRFTISRDNAKNTVYLQMNSLRPEDTAVYYCYMLDTWGQGTQVTVSS

SEQ ID NO: 274 - protein, 111 aa, synthetic construct
EVQLVESGGGVVQPGGSLRLSCAASGTDFSINFIRWYRQAPGKGLEFVAGFSATGNTNYADSVKGRFTISRDNAKNAVYLQMNSLRPEDTAVYYCYMLDKWGQGTQVTVSS

SEQ ID NO: 275 - protein, 111 aa, synthetic construct
EVQLVESGGGVVQPGGSLRLSCAASGTDFSINFIRWYRQAPGKGLEFVAGFTATGNTNYADSVKGRFTISRDNAKNAVYLQMNSLRPEDTAVYYCYILDKWGQGTQVTVSS

SEQ ID NO: 276 - protein, 111 aa, synthetic construct
EVQLVESGGGVVQPGGSLRLSCAADGEIFSINFMRWYRQAPGKQREWVAGFTRDGSTNYPDSAKGRFTISRDNAKNTVYLQIDSLKPEDTAVYYCYMLDTWGQGTQVTVSS

SEQ ID NO: 277 - protein, 111 aa, synthetic construct
EVQLVESGGGVVQPGGSLRLSCAASGEIFSINFMRWYGQAPGKQREWVAGFTRDGSTNYPDSAKGRFTISRDNAKNTVYLQIDSLKPEDTAVYYCYMLDTWGQGTQVTVSS

SEQ ID NO: 278 - protein, 111 aa, synthetic construct
EVQLVESGGGVVQPGGSLRLSCAASGEIFSINFMRWYREAPGKQREWVAGFTRDGSTNYPDSAKGRFTISRDNAKNTVYLQIDSLKPEDTAVYYCYMLDTWGQGTQVTVSS

SEQ ID NO: 279 - protein, 111 aa, synthetic construct
EVQLVESGGGVVQPGGSLRLSCAASGEIFSINFMRWYRQAPIKQREWVAGFTRDGSTNYPDSAKGRFTISRDNAKNTVYLQIDSLKPEDTAVYYCYMLDTWGQGTQVTVSS

SEQ ID NO: 280 - protein, 111 aa, synthetic construct
EVQLVESGGGVVQPGGSLRLSCAASGEIFSINFMRWYRQAPGKIREWVAGFTRDGSTNYPDSAKGRFTISRDNAKNTVYLQIDSLKPEDTAVYYCYMLDTWGQGTQVTVSS

SEQ ID NO: 281 - protein, 111 aa, synthetic construct
EVQLVESGGGVVQPGGSLRLSCAASGEIFSINFMRWYRQAPGKQREWVAGFTRDGFTNYPDSAKGRFTISRDNAKNTVYLQIDSLKPEDTAVYYCYMLDTWGQGTQVTVSS

SEQ ID NO: 282 - protein, 111 aa, synthetic construct
EVQLVESGGGVVQPGGSLRLSCAASGEIFSINFMRWYRQAPGKQREWVAGFTRDGYTNYPDSAKGRFTISRDNAKNTVYLQIDSLKPEDTAVYYCYMLDTWGQGTQVTVSS

SEQ ID NO: 283 - protein, 111 aa, synthetic construct
EVQLVESGGGVVQPGGSLRLSCAASGEIFSINFMRWYRQAPGKQREWVAGFTRDGSLNYPDSAKGRFTISRDNAKNTVYLQIDSLKPEDTAVYYCYMLDTWGQGTQVTVSS

SEQ ID NO: 284 - protein, 111 aa, synthetic construct
EVQLVESGGGVVQPGGSLRLSCAASGEIFSINFMRWYRQAPGKQREWVAGFTRDGSKNYPDSAKGRFTISRDNAKNTVYLQIDSLKPEDTAVYYCYMLDTWGQGTQVTVSS

SEQ ID NO: 285 - protein, 117 aa, synthetic construct
EVQLVESGGGLVQPGGSLRLSCTASGGPIEQYPMGWFRRAPGKERNLVASISRSGDGTYYAISSVKGRFTISRDNAENTVFLQMNSLKPDDTAVYYCGAGINPTKIWGQGTQVTVSS

SEQ ID NO: 286 - protein, 117 aa, synthetic construct
EVQLVESGGGLVQPGGSLRLSCTASGGPIEQYPMGWFRRAPGKERELVASFSRSGDGTYYAISSVKGRFTISRDNAENTVFLQMNSLKPDDTAVYYCGAGINPTKIWGQGTQVTVSS

SEQ ID NO: 287 - protein, 117 aa, synthetic construct
EVQLVESGGGLVQPGGSLRLSCTASGGPIEQYPMGWFRRAPGKERELVASSSRSGDGTYYAISSVKGRFTISRDNAENTVFLQMNSLKPDDTAVYYCGAGINPTKIWGQGTQVTVSS

SEQ ID NO: 288 - protein, 117 aa, synthetic construct
EVQLVESGGGLVQPGGSLRLSCTASGGPIEQYPMGWFRRAPGKERESVASISRSGDGTYYAISSVKGRFTISRDNAENTVFLQMNSLKPDDTAVYYCGAGINPTKIWGQGTQVTVSS

SEQ ID NO: 289 - protein, 117 aa, synthetic construct
EVQLVESGGGLVQPGGSLRLSCTASGGPIEQYPMGWFRRAPGKERELQASISRSGDGTYYAISSVKGRFTISRDNAENTVFLQMNSLKPDDTAVYYCGAGINPTKIWGQGTQVTVSS

SEQ ID NO: 290 - protein, 116 aa, synthetic construct
QVQLVQSGGGLVQAGGSLTLSCTASGRPLSDYPMGWFRRAPEKERELVASISRTGDGTYYADGMRGRFTISRDNSENTVSLQMNNLKPEDTAVYYCGAGINPTKYWGQGTQVTVSS

SEQ ID NO: 291 - protein, 116 aa, synthetic construct
EVQLVESGGGLVQAGGSLRLSCTASGRPISDYPMGWFRRAPGKDRELVASISRTGDGTYYANSMKERFTISRDNAQNTVSLQISSLKPEDTAVYYCGAGINPTRYWGQGTQVTVSS

SEQ ID NO: 292 - protein, 116 aa, synthetic construct
QVQLVQSGGGLVQPGGSLRLSCAASGFTFSAYAMSWVRQAPGKGRELVASISRTGDGTYYADGMKGRFTISRDNAENTVSLQINSLKPEDTAIYYCGAGINPTKYWGQGTQVTVSS

SEQ ID NO: 293 - protein, 117 aa, synthetic construct
EVQLVESGGGLVQAGDSLRLSCTASGLPLSNYPMGWFRRAPGKERELIASISRTGDGTYYADSSVKGRFTISRDNAENTVSLQMNSLKPEDTAVYYCGAGINPTKYWGQGTQVTVSS

SEQ ID NO: 294 - protein, 111 aa, synthetic construct
QVQLVQSGGGLVQAGGSLRLSCAASGSIFSDITLAWHRQIPGKEREWVAGISRSGSPSYRDSVKGRFTISRDNAKNTVFLQMNSLEPEDTGVYYCYSRGYWGQGTQVTVSS

SEQ ID NO: 295 - protein, 112 aa, synthetic construct
EVQLVQSGGGLVQAGGSLRLSCAASGRDFSDTSMAWHRQAPGKERLWVAGIRSGSTSTSYADSVKGRFTISRDDAKNTVYLQMDNLTPEDTAVYFCYSKGYWGQGTQVTVSS

SEQ ID NO: 296 - protein, 114 aa, synthetic construct
EVQLVESGGGLVQPGESLRLSCTASESISIYGVGWYRQAPGEQRVLVAHLKRNGLTEYKDSVKGRFTISRDNARNTIYLEMKNLKPEDTAIYYCNTALGSVLPWGRGTQVTVSS

SEQ ID NO: 297 - protein, 128 aa, synthetic construct
EVQLVESGGGLVQPGGSLRLSCVSSATFGGYSMGWFRQAPGKEREFVAAITWNGGIIKDYADGVMGRFTISRNSALNTVYLQMDSLKSTDTGVYVCAGDRTYYAGGYVPTSEREYAFWGQGTQVTVSS

SEQ ID NO: 298 - protein, 115 aa, synthetic construct
QVQLVQSGGGLVQAGGSLRLSCAASGSIFLINDMGWYRQAPGKQRELVAVRGGSTKYGDSVKGRFTISRDDAKNTVYLQMNSLKPEDTAVYYCHRESGLGSSEYWGQGTQVTVSS

SEQ ID NO: 299 - protein, 118 aa, synthetic construct
EVQLVESGGGLVQAGGSLRLSCTASGRTVSNYRMGWFRQTPGKEREFVAAIAWAGGSLTYADSVKGRFTISRDNAKNTVYLQMNSLEPTDTAVYYCKGSRIFPTRDYWGKGTQVTVSS

SEQ ID NO: 300 - protein, 118 aa, synthetic construct
EVQLVESGGGLVQPGGSLRLSCAASGFTFGSYVMSWVRQAPGKGPEWVSTVSSGGGTTYYADSVKGRFTISRDNAQNTLYLQMNSLKPEDTAVYYCATGRTGLGEGDHRGQGTQVTSS

SEQ ID NO: 301 - DNA, 333 bp, synthetic construct
  source 1..333: mol_type = other DNA
gaggtgcagctggtggagtctgggggaggcgtggtgcagcctggggggtctctaaaactctcctgcgtagcctcgggaacggacttcagtatcaattttatacgctggtaccgccaggctccagggaagcagcgcgagttcgtcgcaggatttactgcgactggtaacacaaactatgcagactccatgaaggggcgattcaccatctccagagacaacaccaagaacgcggtgtatctgcaaatagacagcctgaaacctgaggacacggccgtgtattactgctatatgttggacaagtggggccaggggacccaggtcaccgtctcctca

SEQ ID NO: 302 - DNA, 333 bp, synthetic construct
  source 1..333: mol_type = other DNA
gaggtgcagctggtggagtctgggggaggcgtggtgcagcctggggggtctctaaaactctcctgcgtagcctcgggagcggacttcagtatcaattttatacgctggtaccgccaggctccagggaagcagcgcgagttcgtcgcaggatttactgcgactggtaacacaaactatgcagactccatgaaggggcgattcaccatctccagagacaacaccaagaacgcggtgtatctgcaaatagacagcctgaaacctgaggacacggccgtgtattactgctatatgttggacaagtggggccaggggacccaggtcaccgtctcctca

SEQ ID NO: 303 - DNA, 333 bp, synthetic construct
  source 1..333: mol_type = other DNA
gaggtgcagctggtggagtctgggggaggcgtggtgcagcctggggggtctctaaaactctcctgcgtagcctcgggaacggcgttcagtatcaattttatacgctggtaccgccaggctccagggaagcagcgcgagttcgtcgcaggatttactgcgactggtaacacaaactatgcagactccatgaaggggcgattcaccatctccagagacaacaccaagaacgcggtgtatctgcaaatagacagcctgaaacctgaggacacggccgtgtattactgctatatgttggacaagtggggccaggggacccaggtcaccgtctcctca

SEQ ID NO: 304 - DNA, 333 bp, synthetic construct
  source 1..333: mol_type = other DNA
gaggtgcagctggtggagtctgggggaggcgtggtgcagcctggggggtctctaaaactctcctgcgtagcctcgggaacggacttcagtatcaattttatacgctggtaccgccaggctccagggaagcagcgcgagttcgtcgcaggatttactgcggcgggtaacacaaactatgcagactccatgaaggggcgattcaccatctccagagacaacaccaagaacgcggtgtatctgcaaatagacagcctgaaacctgaggacacggccgtgtattactgctatatgttggacaagtggggccaggggacccaggtcaccgtctcctca

SEQ ID NO: 305 - DNA, 333 bp, synthetic construct
  source 1..333: mol_type = other DNA
gaggtgcagctggtggagtctgggggaggcgtggtgcagcctggggggtctctaaaactctcctgcgtagcctcgggaacggacttcagtatcaattttatacgctggtaccgccaggctccagggaagcagcgcgagttcgtcgcaggatttactgcgactggtgcgacaaactatgcagactccatgaaggggcgattcaccatctccagagacaacaccaagaacgcggtgtatctgcaaatagacagcctgaaacctgaggacacggccgtgtattactgctatatgttggacaagtggggccaggggacccaggtcaccgtctcctca

SEQ ID NO: 306 - DNA, 333 bp, synthetic construct
  source 1..333: mol_type = other DNA
gaggtgcagctggtggagtctgggggaggcgtggtgcagcctggggggtctctaaaactctcctgcgtagcctcgggaacggacttcagtatcaattttatacgctggtaccgccaggctccagggaagcagcgcgagttcgtcgcaggatttactgcgactggtaacacaaactatgcagactccatgaaggggcgattcaccatctccagagacaacaccaagaacgcggtgtatctgcaaatagacagcctgaaacctgaggacacggccgtgtattactgcgcgatgttggacaagtggggccaggggacccaggtcaccgtctcctca

SEQ ID NO: 307 - DNA, 333 bp, synthetic construct
  source 1..333: mol_type = other DNA
gaggtgcagctggtggagtctgggggaggcgtggtgcagcctggggggtctctaaaactctcctgcgtagcctcgggaacggacttcagtatcaattttatacgctggtaccgccaggctccagggaagcagcgcgagttcgtcgcaggatttactgcgactggtaacacaaactatgcagactccatgaaggggcgattcaccatctccagagacaacaccaagaacgcggtgtatctgcaaatagacagcctgaaacctgaggacacggccgtgtattactgctatgcgttggacaagtggggccaggggacccaggtcaccgtctcctca

SEQ ID NO: 308 - DNA, 333 bp, synthetic construct
  source 1..333: mol_type = other DNA
gaggtgcagctggtggagtctgggggaggcgtggtgcagcctggggggtctctaaaactctcctgcgtagcctcgggaacggacttcagtatcaattttatacgctggtaccgccaggctccagggaagcagcgcgagttcgtcgcaggatttactgcgactggtaacacaaactatgcagactccatgaaggggcgattcaccatctccagagacaacaccaagaacgcggtgtatctgcaaatagacagcctgaaacctgaggacacggccgtgtattactgctatatggcggacaagtggggccaggggacccaggtcaccgtctcctca

SEQ ID NO: 309 - DNA, 333 bp, synthetic construct
  source 1..333: mol_type = other DNA
gaggtgcagctggtggagtctgggggaggcgtggtgcagcctggggggtctctaaaactctcctgcgtagcctcgggaacggacttcagtatcaattttatacgctggtaccgccaggctccagggaagcagcgcgagttcgtcgcaggatttactgcgactggtaacacaaactatgcagactccatgaaggggcgattcaccatctccagagacaacaccaagaacgcggtgtatctgcaaatagacagcctgaaacctgaggacacggccgtgtattactgctatatgttggcgaagtggggccaggggacccaggtcaccgtctcctca

SEQ ID NO: 310 - DNA, 333 bp, synthetic construct
  source 1..333: mol_type = other DNA
gaggtgcagctggtggagtctgggggaggcgtggtgcagcctggggggtctctaaaactctcctgcgtagcctcgggaacggacttcagtatcaattttatacgctggtaccgccaggctccagggaagcagcgcgagttcgtcgcaggatttactgcgactggtaacacaaactatgcagactccatgaaggggcgattcaccatctccagagacaacaccaagaacgcggtgtatctgcaaatagacagcctgaaacctgaggacacggccgtgtattactgctatatgttggacgcgtggggccaggggacccaggtcaccgtctcctca

SEQ ID NO: 311 - DNA, 333 bp, synthetic construct
  source 1..333: mol_type = other DNA
gaggtgcagctggtggagtctgggggaggcgtggtgcagcctggggggtctctgagactctcctgtgcagcctctggagagatcttcagtatcaattttatgcgctggtaccgccaggctccagggaagcagcgcgagtgggtcgcaggttttactagggatggaagcacaaactatccagactccgcgaagggccgattcaccatctctagagacaacgccaagaacacggtgtatctgcaaatagacagcctgaaacctgaggacacggccgtctattattgttatatgttggacacctggggccaggggacccaggtcactgtctcctca

SEQ ID NO: 312 - DNA, 351 bp, synthetic construct
  source 1..351: mol_type = other DNA
gaggtgcagctggtggagtctgggggaggcttggtgcagcctgggggttctctgagactctcctgtacagcctctggaggccccatcgagcagtatcccatgggctggttccgccgggccccaggaaaggagcgtgaattggtagcaagtattagccgaagtggagatggcacatactatgcaatctcttccgtgaagggccgattcaccatctctagagacaacgccgagaacacggtatttctgcaaatgaacagcctgaaacctgacgacacggccgtttattactgtggggctggtataaacccaaccaagatctggggccaggggacccaggtcaccgtctcctca

SEQ ID NO: 313 - DNA, 333 bp, synthetic construct
  source 1..333: mol_type = other DNA
gaggtgcagctggtggagtctgggggaggcgaggtgcagcctggggggtctctgaaactctcctgtgtagcctctggaaccgacttcagtatcaattttgtgcgctggtaccgtcagcgtccagggaagcagcgcgagtgggtcgcaggatttactgcgaatggtgatacaaactatccagactccatgaaggggcgattcaccatttccagagacaacgccaagaatacggtgtatctacagataaacagcctgaaatctgaggacacggccgtctattattgctatatgttagataattggggccaggggacccaggtcaccgtctcctca

SEQ ID NO: 314 - DNA, 333 bp, synthetic construct
  source 1..333: mol_type = other DNA
gaggtgcagctggtggagtctgggggaggcgtggtgcagcctggggggtctctaaaactctcctgcgtagcctcgggaacggacttcagtctgaattttatacgctggtaccgccaggctccagggaagcagcgcgagttcgtcgcaggatttactgcgactggtaacacaaactatgcagactccatgaaggggcgattcaccatctccagagacaacaccaagaacgcggtgtatctgcaaatagacagcctgaaacctgaggacacggccgtgtattactgctatatgttggacaagtggggccaggggacccaggtcaccgtctcctca

SEQ ID NO: 315 - DNA, 333 bp, synthetic construct
  source 1..333: mol_type = other DNA
gaggtgcagctggtggagtctgggggaggcgtggtgcagcctggggggtctctaaaactctcctgcgtagcctcgggaacggacttcagtatcaattacatacgctggtaccgccaggctccagggaagcagcgcgagttcgtcgcaggatttactgcgactggtaacacaaactatgcagactccatgaaggggcgattcaccatctccagagacaacaccaagaacgcggtgtatctgcaaatagacagcctgaaacctgaggacacggccgtgtattactgctatatgttggacaagtggggccaggggacccaggtcaccgtctcctca

SEQ ID NO: 316 - DNA, 333 bp, synthetic construct
  source 1..333: mol_type = other DNA
gaggtgcagctggtggagtctgggggaggcgtggtgcagcctggggggtctctaaaactctcctgcgtagcctcgggaacggacttcagtatcaattttatacgctggtaccgccaggctccagggaagcagcgcgagttcgtcgcaggaattactgcgactggtaacacaaactatgcagactccatgaaggggcgattcaccatctccagagacaacaccaagaacgcggtgtatctgcaaatagacagcctgaaacctgaggacacggccgtgtattactgctatatgttggacaagtggggccaggggacccaggtcaccgtctcctca

SEQ ID NO: 317 - DNA, 333 bp, synthetic construct
  source 1..333: mol_type = other DNA
gaggtgcagctggtggagtctgggggaggcgtggtgcagcctggggggtctctaaaactctcctgcgtagcctcgggaacggacttcagtatcaattttatacgctggtaccgccaggctccagggaagcagcgcgagttcgtcgcaggattttcagcgactggtaacacaaactatgcagactccatgaaggggcgattcaccatctccagagacaacaccaagaacgcggtgtatctgcaaatagacagcctgaaacctgaggacacggccgtgtattactgctatatgttggacaagtggggccaggggacccaggtcaccgtctcctca

SEQ ID NO: 318 - DNA, 333 bp, synthetic construct
  source 1..333: mol_type = other DNA
gaggtgcagctggtggagtctgggggaggcgtggtgcagcctggggggtctctaaaactctcctgcgtagcctcgggaacggacttcagtatcaattttatacgctggtaccgccaggctccagggaagcagcgcgagttcgtcgcaggatttactgcgactggtaactcaaactatgcagactccatgaaggggcgattcaccatctccagagacaacaccaagaacgcggtgtatctgcaaatagacagcctgaaacctgaggacacggccgtgtattactgctatatgttggacaagtggggccaggggacccaggtcaccgtctcctca

SEQ ID NO: 319 - DNA, 333 bp, synthetic construct
  source 1..333: mol_type = other DNA
gaggtgcagctggtggagtctgggggaggcgtggtgcagcctggggggtctctaaaactctcctgcgtagcctcgggaacggacttcagtatcaattttatacgctggtaccgccaggctccagggaagcagcgcgagttcgtcgcaggatttactgcgactggtaacacaaactatgcagactccatgaaggggcgattcaccatctccagagacaacaccaagaacgcggtgtatctgcaaatagacagcctgaaacctgaggacacggccgtgtattactgctttatgttggacaagtggggccaggggacccaggtcaccgtctcctca

SEQ ID NO: 320 - DNA, 333 bp, synthetic construct
  source 1..333: mol_type = other DNA
gaggtgcagctggtggagtctgggggaggcgtggtgcagcctggggggtctctaaaactctcctgcgtagcctcgggaacggacttcagtatcaattttatacgctggtaccgccaggctccagggaagcagcgcgagttcgtcgcaggatttactgcgactggtaacacaaactatgcagactccatgaaggggcgattcaccatctccagagacaacaccaagaacgcggtgtatctgcaaatagacagcctgaaacctgaggacacggccgtgtattactgctatattttggacaagtggggccaggggacccaggtcaccgtctcctca

SEQ ID NO: 321 - DNA, 333 bp, synthetic construct
  source 1..333: mol_type = other DNA
gaggtgcagctggtggagtctgggggaggcgtggtgcagcctggggggtctctaaaactctcctgcgtagcctcgggaacggacttcagtatcaattttatacgctggtaccgccaggctccagggaagcagcgcgagttcgtcgcaggatttactgcgactggtaacacaaactatgcagactccatgaaggggcgattcaccatctccagagacaacaccaagaacgcggtgtatctgcaaatagacagcctgaaacctgaggacacggccgtgtattactgctatatgattgacaagtggggccaggggacccaggtcaccgtctcctca

SEQ ID NO: 322 - DNA, 333 bp, synthetic construct
  source 1..333: mol_type = other DNA
gaggtgcagctggtggagtctgggggaggcgtggtgcagcctggggggtctctaaaactctcctgcgtagcctcgggaacggacttcagtatcaattttatacgctggtaccgccaggctccagggaagcagcgcgagttcgtcgcaggatttactgcgactggtaacacaaactatgcagactccatgaaggggcgattcaccatctccagagacaacaccaagaacgcggtgtatctgcaaatagacagcctgaaacctgaggacacggccgtgtattactgctatatggtggacaagtggggccaggggacccaggtcaccgtctcctca

SEQ ID NO: 323 - DNA, 333 bp, synthetic construct
  source 1..333: mol_type = other DNA
gaggtgcagctggtggagtctgggggaggcgtggtgcagcctggggggtctctaaaactctcctgcgtagcctcgggaacggacttcagtatcaattttatacgctggtaccgccaggctccagggaagcagcgcgagttcgtcgcaggatttactgcgactggtaacacaaactatgcagactccatgaaggggcgattcaccatctccagagacaacaccaagaacgcggtgtatctgcaaatagacagcctgaaacctgaggacacggccgtgtattactgctatatgttggaaaagtggggccaggggacccaggtcaccgtctcctca

SEQ ID NO: 324 - DNA, 333 bp, synthetic construct
  source 1..333: mol_type = other DNA
gaggtgcagctggtggagtctgggggaggcgtggtgcagcctggggggtctctacgtctctcctgcgcagcctcgggaacggacttcagtatcaattttatgagctgggttcgccaggctccagggaagggtctggagtgggtcgcaggatttactgcgactggtaacacaaactatgcagactccgttaaggggcgattcaccatctccagagacaacgcaaagaacaccctgtatctgcaaatgaatagcctgcgtcctgaggacacggccgtgtattactgctatatgttggacaagtggggccaggggacccaggtcaccgtctcctca

SEQ ID NO: 325 - DNA, 333 bp, synthetic construct
  source 1..333: mol_type = other DNA
gaggtgcagctggtggagtctgggggaggcgtggtgcagcctggggggtctctacgtctctcctgcgcagcctcgggaacggacttcagtatcaattttatacgctgggttcgccaggctccagggaagcagcgcgagttcgtcgcaggatttactgcgactggtaacacaaactatgcagactccgttaaggggcgattcaccatctccagagacaacgcaaagaacaccctgtatctgcaaatgaatagcctgcgtcctgaggacacggccgtgtattactgctatatgttggacaagtggggccaggggacccaggtcaccgtctcctca

SEQ ID NO: 326 - DNA, 333 bp, synthetic construct
  source 1..333: mol_type = other DNA
gaggtgcagctggtggagtctgggggaggcgtggtgcagcctggggggtctctacgtctctcctgcgcagcctcgggaacggacttcagtatcaattttatgcattgggttcgccaggctccagggaagggtctggagtgggtcgcaggatttactgcgactggtaacacaaactatgcagactccgttaaggggcgattcaccatctccagagacaacgcaaagaacaccctgtatctgcaaatgaatagcctgcgtcctgaggacacggccgtgtattactgctatatgttggacaagtggggccaggggacccaggtcaccgtctcctca

SEQ ID NO: 327 - DNA, 333 bp, synthetic construct
  source 1..333: mol_type = other DNA
gaggtgcagctggtggagtctgggggaggcgtggtgcagcctggggggtctctacgtctctcctgcgcagcctcgggaacggacttcagtatcaattttatgagctgggttcgccaggctccagggaagcagcgcgagttcgtcgcaggatttactgcgactggtaacacaaactatgcagactccgttaaggggcgattcaccatctccagagacaacgcaaagaacaccctgtatctgcaaatgaatagcctgcgtcctgaggacacggccgtgtattactgctatatgttggacaagtggggccaggggacccaggtcaccgtctcctca

SEQ ID NO: 328 - DNA, 333 bp, synthetic construct
  source 1..333: mol_type = other DNA
gaggtgcagctggtggagtctgggggaggcgtggtgcagcctggggggtctctacgtctctcctgcgcagcctcgggaacggacttcagtatcaattttatacgctgggttcgccaggctccagggaagggtctggagtgggtcgcaggatttactgcgactggtaacacaaactatgcagactccgttaaggggcgattcaccatctccagagacaacgcaaagaacaccctgtatctgcaaatgaatagcctgcgtcctgaggacacggccgtgtattactgctatatgttggacaagtggggccaggggacccaggtcaccgtctcctca

SEQ ID NO: 329 - DNA, 333 bp, synthetic construct
  source 1..333: mol_type = other DNA
gaggtgcagctggtggagtctgggggaggcgtggtgcagcctggggggtctctacgtctctcctgcgcagcctcgggaacggacttcagtatcaattttatacattgggttcgccaggctccagggaagggtctggagtgggtcgcaggatttactgcgactggtaacacaaactatgcagactccgttaaggggcgattcaccatctccagagacaacgcaaagaacaccctgtatctgcaaatgaatagcctgcgtcctgaggacacggccgtgtattactgctatatgttggacaagtggggccaggggacccaggtcaccgtctcctca

SEQ ID NO: 330 - DNA, 78 bp, synthetic construct
  source 1..78: mol_type = other DNA
gcggccgcagaacaaaaactcatctcagaagaggatctgaatggggccgcacatcaccaccatcaccatgggagctag

SEQ ID NO: 331 - protein, 25 aa, synthetic construct
EVQLVESGGGVVQPGGSLKLSCAAS

SEQ ID NO: 332 - protein, 25 aa, synthetic construct [sequence omitted]

SEQ ID NO: 333 - protein, 25 aa, synthetic construct
EVQLVESGGGVVQPGGSLRLSCAAD

SEQ ID NO: 334 - protein, 25 aa, synthetic construct
QVQLVQSGGGLVQAGGSLTLSCTAS

SEQ ID NO: 335 - protein, 25 aa, synthetic construct
EVQLVESGGGLVQAGGSLRLSCTAS

SEQ ID NO: 336 - protein, 25 aa, synthetic construct
QVQLVQSGGGLVQPGGSLRLSCAAS

SEQ ID NO: 337 - protein, 25 aa, synthetic construct
EVQLVESGGGLVQAGDSLRLSCTAS

SEQ ID NO: 338 - protein, 25 aa, synthetic construct
QVQLVQSGGGLVQAGGSLRLSCAAS

SEQ ID NO: 339 - protein, 25 aa, synthetic construct
EVQLVQSGGGLVQAGGSLRLSCAAS

SEQ ID NO: 340 - protein, 25 aa, synthetic construct
EVQLVESGGGLVQPGESLRLSCTAS

SEQ ID NO: 341 - protein, 25 aa, synthetic construct
EVQLVESGGGLVQPGGSLRLSCVSS

SEQ ID NO: 342 - protein, 17 aa, synthetic construct
IRWVRQAPGKGLEWVAG

SEQ ID NO: 343 - protein, 17 aa, synthetic construct
IRWYRQAPGKGLEFVAG

SEQ ID NO: 344 - protein, 17 aa, synthetic construct
IRWVRQAPGKGLEFVAG

SEQ ID NO: 345 - protein, 17 aa, synthetic construct
IRWYRQAPGKGREFVAG

SEQ ID NO: 346 - protein, 17 aa, synthetic construct
IRWVRQAPGKQREFVAG

SEQ ID NO: 347 - protein, 17 aa, synthetic construct
IRWYRQAPGKGLEWVAG

SEQ ID NO: 348 - protein, 17 aa, synthetic construct
MRWYRQAPGKGLEWVAG

SEQ ID NO: 349 - protein, 17 aa, synthetic construct
MRWYGQAPGKQREWVAG

SEQ ID NO: 350 - protein, 17 aa, synthetic construct
MRWYREAPGKQREWVAG

SEQ ID NO: 351 - protein, 17 aa, synthetic construct
MRWYRQAPIKQREWVAG

SEQ ID NO: 352 - protein, 17 aa, synthetic construct
MRWYRQAPGKIREWVAG

SEQ ID NO: 353 - protein, 17 aa, synthetic construct
MGWFRRAPGKERNLVAS

SEQ ID NO: 354 - protein, 17 aa, synthetic construct
MGWFRRAPGKERESVAS

SEQ ID NO: 355 - protein, 17 aa, synthetic construct
MGWFRRAPGKERELQAS

SEQ ID NO: 356 - protein, 17 aa, synthetic construct
MGWFRRAPEKERELVAS

SEQ ID NO: 357 - protein, 17 aa, synthetic construct
MGWFRRAPGKDRELVAS

SEQ ID NO: 358 - protein, 17 aa, synthetic construct
MSWVRQAPGKGRELVAS

SEQ ID NO: 359 - protein, 17 aa, synthetic construct
MGWFRRAPGKERELIAS

SEQ ID NO: 360 - protein, 17 aa, synthetic construct
LAWHRQIPGKEREWVAG

SEQ ID NO: 361 - protein, 17 aa, synthetic construct
MAWHRQAPGKERLWVAG

SEQ ID NO: 362 - protein, 17 aa, synthetic construct
VGWYRQAPGEQRVLVAH

SEQ ID NO: 363 - protein, 17 aa, synthetic construct
MGWFRQAPGKEREFVAA

SEQ ID NO: 364 - protein, 17 aa, synthetic construct
MGWYRQAPGKQRELVAV

SEQ ID NO: 365 - protein, 17 aa, synthetic construct
MGWFRQTPGKEREFVAA

SEQ ID NO: 366 - protein, 38 aa, synthetic construct
NYADSMKGRFTISRDNTKNALYLQIDSLRPEDTAVYYC

SEQ ID NO: 367 - protein, 38 aa, synthetic construct
NYADSVKGRFTISRDNTKNTLYLQIDSLRPEDTAVYYC

SEQ ID NO: 368 - protein, 38 aa, synthetic construct
NYADSVKGRFTISRDNAKNTLYLQMNSLRPEDTAVYYC

SEQ ID NO: 369 - protein, 38 aa, synthetic construct
NYADSVKGRFTISRDNTKNTLYLQINSLRPEDTAVYYC

SEQ ID NO: 370 - protein, 38 aa, synthetic construct
NYADSMKGRFTISRDNTKNTLYLQMNSLRPEDTAVYYC

SEQ ID NO: 371 - protein, 38 aa, synthetic construct
NYADSVKGRFTISRDNAKNTLYLQIDSLRPEDTAVYYC

SEQ ID NO: 372 - protein, 38 aa, synthetic construct
NYADSVKGRFTISRDNTKNTLYLQMNSLRPEDTAVYYC

SEQ ID NO: 373 - protein, 38 aa, synthetic construct
NYADSVKGRFTISRDNTKNALYLQMNSLRPEDTAVYYC

SEQ ID NO: 374 - protein, 38 aa, synthetic construct
NYADSVKGRFTISRDNTKNTLYLQMDSLRPEDTAVYYC

SEQ ID NO: 375 - protein, 38 aa, synthetic construct
NYADSVKGRFTISRDNSKNTLYLQMNSLRAEDTAVYYC

SEQ ID NO: 376 - protein, 38 aa, synthetic construct
NYADSVKGRFTISRDNAKNAVYLQMNSLRPEDTAVYYC

SEQ ID NO: 377 - protein, 38 aa, synthetic construct
NYADSVKGRFTISRDNAKNTLYLQMNSLKPEDTAVYYC

SEQ ID NO: 378 - protein, 38 aa, synthetic construct
NYADSMKGRFTISRDNAKNTLYLQMNSLRPEDTAVYYC

SEQ ID NO: 379 - protein, 38 aa, synthetic construct
NYPDSVKGRFTISRDNAKNTVYLQMNSLRPEDTAVYYC

SEQ ID NO: 380 - protein, 38 aa, synthetic construct
YYADGMRGRFTISRDNSENTVSLQMNNLKPEDTAVYYC

SEQ ID NO: 381 - protein, 38 aa, synthetic construct
YYANSMKERFTISRDNAQNTVSLQISSLKPEDTAVYYC

SEQ ID NO: 382 - protein, 38 aa, synthetic construct
YYADGMKGRFTISRDNAENTVSLQINSLKPEDTAIYYC

SEQ ID NO: 383 - protein, 39 aa, synthetic construct
YYADSSVKGRFTISRDNAENTVSLQMNSLKPEDTAVYYC

SEQ ID NO: 384 - protein, 38 aa, synthetic construct
SYRDSVKGRFTISRDNAKNTVFLQMNSLEPEDTGVYYC

SEQ ID NO: 385 - protein, 38 aa, synthetic construct
SYADSVKGRFTISRDDAKNTVYLQMDNLTPEDTAVYFC

SEQ ID NO: 386 - protein, 38 aa, synthetic construct
EYKDSVKGRFTISRDNARNTIYLEMKNLKPEDTAIYYC

SEQ ID NO: 387 - protein, 38 aa, synthetic construct
DYADGVMGRFTISRNSALNTVYLQMDSLKSTDTGVYVC

SEQ ID NO: 388 - protein, 38 aa, synthetic construct
KYGDSVKGRFTISRDDAKNTVYLQMNSLKPEDTAVYYC

SEQ ID NO: 389 - protein, 38 aa, synthetic construct
TYADSVKGRFTISRDNAKNTVYLQMNSLEPTDTAVYYC

SEQ ID NO: 390 - protein, 11 aa, synthetic construct
WGQGTLVTVSS

SEQ ID NO: 391 - protein, 11 aa, synthetic construct
WGKGTQVTVSS

SEQ ID NO: 392 - protein, 8 aa, synthetic construct
GHDFSINF

SEQ ID NO: 393 - protein, 136 aa, synthetic construct
EVQLVESGGGVVQPGGSLKLSCVASGHDFSINFIRWYRQAPGKQREFVAGFTATGNTNYADSMKGRFTISRDNTKNAVYLQIDSLKPEDTAVYYCYMLDKWGQGTQVTVSSAAAEQKLISEEDLNGAAHHHHHHGS

SEQ ID NO: 394 - protein, 10 aa, synthetic construct
EQKLISEEDL

SEQ ID NO: 395 - protein, 6 aa, synthetic construct
HHHHHH

SEQ ID NO: 396 - protein, 8 aa, synthetic construct
HHHHHHHH

SEQ ID NO: 397 - protein, 9 aa, synthetic construct
YPYDVPDYA

SEQ ID NO: 398 - protein, 8 aa, synthetic construct
DYKDDDDK

SEQ ID NO: 399 - protein, 12 aa, synthetic construct
GGGGSCHHHHHH

SEQ ID NO: 400 - protein, 25 aa, synthetic construct
EVQLVESGGGVVQPGGSLRLSCVAS

SEQ ID NO: 401 - protein, 7 aa, synthetic construct
GGGGLQR

SEQ ID NO: 402 - protein, 8 aa, synthetic construct
GGGGGLQR

SEQ ID NO: 403 - protein, 9 aa, synthetic construct
GGGGGGLQR

SEQ ID NO: 404 - protein, 10 aa, synthetic construct
GGGGGGGLQR

SEQ ID NO: 405 - DNA, 20 bp, synthetic construct
  source 1..20: mol_type = other DNA
  misc_feature 1: note = linker (conjugation handle)
  misc_feature 1..20: note = phosphorothioate internucleosidic linkage
  modified_base 17: mod_base = OTHER; note = 2'-O-methoxyethyl-5-methyl-cytidine
  modified_base 1..5: mod_base = OTHER; note = 2'-O-methoxyethyl
  modified_base 16: mod_base = OTHER; note = 2'-O-methoxyethyl
  modified_base 18..20: mod_base = OTHER; note = 2'-O-methoxyethyl
  modified_base 6..15: mod_base = OTHER; note = oligodeoxynucleotides
gggagttacttgccaacttg

SEQ ID NO: 406 - protein, 16 aa, synthetic construct
AAAHHHHHHGGGGLQR

SEQ ID NO: 407 - protein, 17 aa, synthetic construct
AAAHHHHHHGGGGGLQR

SEQ ID NO: 408 - protein, 18 aa, synthetic construct
AAAHHHHHHGGGGGGLQR

SEQ ID NO: 409 - protein, 19 aa, synthetic construct
AAAHHHHHHGGGGGGGLQR

SEQ ID NO: 410 - protein, 8 aa, synthetic construct
DEIFSINF

SEQ ID NO: 411 - protein, 136 aa, synthetic construct
EVQLVESGGGVVQPGGSLRLSCAASDEIFSINFMRWYRQAPGKQREWVAGFTRDGSTNYPDSAKGRFTISRDNAKNTVYLQIDSLKPEDTAVYYCYMLDTWGQGTQVTVSSAAAEQKLISEEDLNGAAHHHHHHGS

SEQ ID NO: 412 - protein, 111 aa, synthetic construct
EVQLVESGGGVVQPGGSLRLSCAASDEIFSINFMRWYRQAPGKQREWVAGFTRDGSTNYPDSAKGRFTISRDNAKNTVYLQIDSLKPEDTAVYYCYMLDTWGQGTQVTVSS

SEQ ID NO: 413 - protein, 8 aa, synthetic construct
GEIFYINF

SEQ ID NO: 414 - protein, 136 aa, synthetic construct
EVQLVESGGGVVQPGGSLRLSCAASGEIFYINFMRWYRQAPGKQREWVAGFTRDGSTNYPDSAKGRFTISRDNAKNTVYLQIDSLKPEDTAVYYCYMLDTWGQGTQVTVSSAAAEQKLISEEDLNGAAHHHHHHGS

SEQ ID NO: 415 - protein, 111 aa, synthetic construct
EVQLVESGGGVVQPGGSLRLSCAASGEIFYINFMRWYRQAPGKQREWVAGFTRDGSTNYPDSAKGRFTISRDNAKNTVYLQIDSLKPEDTAVYYCYMLDTWGQGTQVTVSS

SEQ ID NO: 416 - protein, 7 aa, synthetic construct
FTRLGST

SEQ ID NO: 417 - protein, 136 aa, synthetic construct
EVQLVESGGGVVQPGGSLRLSCAASGEIFSINFMRWYRQAPGKQREWVAGFTRLGSTNYPDSAKGRFTISRDNAKNTVYLQIDSLKPEDTAVYYCYMLDTWGQGTQVTVSSAAAEQKLISEEDLNGAAHHHHHHGS

SEQ ID NO: 418 - protein, 111 aa, synthetic construct
EVQLVESGGGVVQPGGSLRLSCAASGEIFSINFMRWYRQAPGKQREWVAGFTRLGSTNYPDSAKGRFTISRDNAKNTVYLQIDSLKPEDTAVYYCYMLDTWGQGTQVTVSS

SEQ ID NO: 419 - protein, 7 aa, synthetic construct
FTRDDST

SEQ ID NO: 420 - protein, 136 aa, synthetic construct
EVQLVESGGGVVQPGGSLRLSCAASGEIFSINFMRWYRQAPGKQREWVAGFTRDDSTNYPDSAKGRFTISRDNAKNTVYLQIDSLKPEDTAVYYCYMLDTWGQGTQVTVSSAAAEQKLISEEDLNGAAHHHHHHGS

SEQ ID NO: 421 - protein, 111 aa, synthetic construct
EVQLVESGGGVVQPGGSLRLSCAASGEIFSINFMRWYRQAPGKQREWVAGFTRDDSTNYPDSAKGRFTISRDNAKNTVYLQIDSLKPEDTAVYYCYMLDTWGQGTQVTVSS

SEQ ID NO: 422 - protein, 136 aa, synthetic construct
EVQLVESGGGVVQPGGSLRLSCAASGEIFSINFMRWYRQAPGKQREQVAGFTRDGSTNYPDSAKGRFTISRDNAKNTVYLQIDSLKPEDTAVYYCYMLDTWGQGTQVTVSSAAAEQKLISEEDLNGAAHHHHHHGS

SEQ ID NO: 423 - protein, 111 aa, synthetic construct
EVQLVESGGGVVQPGGSLRLSCAASGEIFSINFMRWYRQAPGKQREQVAGFTRDGSTNYPDSAKGRFTISRDNAKNTVYLQIDSLKPEDTAVYYCYMLDTWGQGTQVTVSS

SEQ ID NO: 424 - protein, 136 aa, synthetic construct
EVQLVESGGGVVQPGGSLRLSCAASGEIFSINFMRWYRQAPGKQREFVAGFTRDGSTNYPDSAKGRFTISRDNAKNTVYLQIDSLKPEDTAVYYCYMLDTWGQGTQVTVSSAAAEQKLISEEDLNGAAHHHHHHGS

SEQ ID NO: 425 - protein, 111 aa, synthetic construct
EVQLVESGGGVVQPGGSLRLSCAASGEIFSINFMRWYRQAPGKQREFVAGFTRDGSTNYPDSAKGRFTISRDNAKNTVYLQIDSLKPEDTAVYYCYMLDTWGQGTQVTVSS

SEQ ID NO: 426 - protein, 8 aa, synthetic construct
GEIHSINF

SEQ ID NO: 427 - protein, 136 aa, synthetic construct
EVQLVESGGGVVQPGGSLRLSCAASGEIHSINFMRWYRQAPGKQREWVAGFTRDGSTNYPDSAKGRFTISRDNAKNTVYLQIDSLKPEDTAVYYCYMLDTWGQGTQVTVSSAAAEQKLISEEDLNGAAHHHHHHGS

SEQ ID NO: 428 - protein, 111 aa, synthetic construct
EVQLVESGGGVVQPGGSLRLSCAASGEIHSINFMRWYRQAPGKQREWVAGFTRDGSTNYPDSAKGRFTISRDNAKNTVYLQIDSLKPEDTAVYYCYMLDTWGQGTQVTVSS

SEQ ID NO: 429 - protein, 136 aa, synthetic construct
EVQLVESGGGVVQPGGSLRLSCAASGEIFSINFMRWYRQAPGKQRHWVAGFTRDGSTNYPDSAKGRFTISRDNAKNTVYLQIDSLKPEDTAVYYCYMLDTWGQGTQVTVSSAAAEQKLISEEDLNGAAHHHHHHGS

SEQ ID NO: 430 - protein, 111 aa, synthetic construct
EVQLVESGGGVVQPGGSLRLSCAASGEIFSINFMRWYRQAPGKQRHWVAGFTRDGSTNYPDSAKGRFTISRDNAKNTVYLQIDSLKPEDTAVYYCYMLDTWGQGTQVTVSS

SEQ ID NO: 431 - protein, 7 aa, synthetic construct
FTRDGSH

SEQ ID NO: 432 - protein, 136 aa, synthetic construct
EVQLVESGGGVVQPGGSLRLSCAASGEIFSINFMRWYRQAPGKQREWVAGFTRDGSHNYPDSAKGRFTISRDNAKNTVYLQIDSLKPEDTAVYYCYMLDTWGQGTQVTVSSAAAEQKLISEEDLNGAAHHHHHHGS

SEQ ID NO: 433 - protein, 111 aa, synthetic construct
EVQLVESGGGVVQPGGSLRLSCAASGEIFSINFMRWYRQAPGKQREWVAGFTRDGSHNYPDSAKGRFTISRDNAKNTVYLQIDSLKPEDTAVYYCYMLDTWGQGTQVTVSS

SEQ ID NO: 434 - protein, 8 aa, synthetic construct
GEIFSINN

SEQ ID NO: 435 - protein, 136 aa, synthetic construct
EVQLVESGGGVVQPGGSLRLSCAASGEIFSINNMRWYRQAPGKQREWVAGFTRDGSTNYPDSAKGRFTISRDNAKNTVYLQIDSLKPEDTAVYYCYMLDTWGQGTQVTVSSAAAEQKLISEEDLNGAAHHHHHHGS

SEQ ID NO: 436 - protein, 111 aa, synthetic construct
EVQLVESGGGVVQPGGSLRLSCAASGEIFSINNMRWYRQAPGKQREWVAGFTRDGSTNYPDSAKGRFTISRDNAKNTVYLQIDSLKPEDTAVYYCYMLDTWGQGTQVTVSS

SEQ ID NO: 437 - protein, 8 aa, synthetic construct
GEIFSINQ

SEQ ID NO: 438 - protein, 136 aa, synthetic construct
EVQLVESGGGVVQPGGSLRLSCAASGEIFSINQMRWYRQAPGKQREWVAGFTRDGSTNYPDSAKGRFTISRDNAKNTVYLQIDSLKPEDTAVYYCYMLDTWGQGTQVTVSSAAAEQKLISEEDLNGAAHHHHHHGS

SEQ ID NO: 439 - protein, 111 aa, synthetic construct
EVQLVESGGGVVQPGGSLRLSCAASGEIFSINQMRWYRQAPGKQREWVAGFTRDGSTNYPDSAKGRFTISRDNAKNTVYLQIDSLKPEDTAVYYCYMLDTWGQGTQVTVSS

SEQ ID NO: 440 - protein, 136 aa, synthetic construct
EVQLVESGGGVVQPGGSLRLSCAASGEIFSINFMIWYRQAPGKQREWVAGFTRDGSTNYPDSAKGRFTISRDNAKNTVYLQIDSLKPEDTAVYYCYMLDTWGQGTQVTVSSAAAEQKLISEEDLNGAAHHHHHHGS

SEQ ID NO: 441 - protein, 111 aa, synthetic construct
EVQLVESGGGVVQPGGSLRLSCAASGEIFSINFMIWYRQAPGKQREWVAGFTRDGSTNYPDSAKGRFTISRDNAKNTVYLQIDSLKPEDTAVYYCYMLDTWGQGTQVTVSS

SEQ ID NO: 442 - protein, 136 aa, synthetic construct
EVQLVESGGGVVQPGGSLRLSCAASGEIFSINFMEWYRQAPGKQREWVAGFTRDGSTNYPDSAKGRFTISRDNAKNTVYLQIDSLKPEDTAVYYCYMLDTWGQGTQVTVSSAAAEQKLISEEDLNGAAHHHHHHGS

SEQ ID NO: 443 - protein, 111 aa, synthetic construct
EVQLVESGGGVVQPGGSLRLSCAASGEIFSINFMEWYRQAPGKQREWVAGFTRDGSTNYPDSAKGRFTISRDNAKNTVYLQIDSLKPEDTAVYYCYMLDTWGQGTQVTVSS

SEQ ID NO: 444 - protein, 136 aa, synthetic construct
EVQLVESGGGVVQPGGSLRLSCAASGEIFSINFMRWYRQAPGKQREWVAAFTRDGSTNYPDSAKGRFTISRDNAKNTVYLQIDSLKPEDTAVYYCYMLDTWGQGTQVTVSSAAAEQKLISEEDLNGAAHHHHHHGS

SEQ ID NO: 445 - protein, 111 aa, synthetic construct
EVQLVESGGGVVQPGGSLRLSCAASGEIFSINFMRWYRQAPGKQREWVAAFTRDGSTNYPDSAKGRFTISRDNAKNTVYLQIDSLKPEDTAVYYCYMLDTWGQGTQVTVSS

SEQ ID NO: 446 - protein, 136 aa, synthetic construct
EVQLVESGGGVVQPGGSLRLSCAASGEIFSINFMRWYRQAPGKQREWVAKFTRDGSTNYPDSAKGRFTISRDNAKNTVYLQIDSLKPEDTAVYYCYMLDTWGQGTQVTVSSAAAEQKLISEEDLNGAAHHHHHHGS

SEQ ID NO: 447 - protein, 111 aa, synthetic construct
EVQLVESGGGVVQPGGSLRLSCAASGEIFSINFMRWYRQAPGKQREWVAKFTRDGSTNYPDSAKGRFTISRDNAKNTVYLQIDSLKPEDTAVYYCYMLDTWGQGTQVTVSS

SEQ ID NO: 448 - protein, 136 aa, synthetic construct
EVQLVESGGGVVQPGGSLRLSCAASGEIFSINFMRWYRQAPGKQREWVAGFTRDGSTVYPDSAKGRFTISRDNAKNTVYLQIDSLKPEDTAVYYCYMLDTWGQGTQVTVSSAAAEQKLISEEDLNGAAHHHHHHGS

SEQ ID NO: 449 - protein, 111 aa, synthetic construct
EVQLVESGGGVVQPGGSLRLSCAASGEIFSINFMRWYRQAPGKQREWVAGFTRDGSTVYPDSAKGRFTISRDNAKNTVYLQIDSLKPEDTAVYYCYMLDTWGQGTQVTVSS

SEQ ID NO: 450 - protein, 136 aa, synthetic construct
EVQLVESGGGVVQPGGSLRLSCAASGEIFSINFMRWYRQAPGKQREWVAGFTRDGSTFYPDSAKGRFTISRDNAKNTVYLQIDSLKPEDTAVYYCYMLDTWGQGTQVTVSSAAAEQKLISEEDLNGAAHHHHHHGS

SEQ ID NO: 451 - protein, 111 aa, synthetic construct
EVQLVESGGGVVQPGGSLRLSCAASGEIFSINFMRWYRQAPGKQREWVAGFTRDGSTFYPDSAKGRFTISRDNAKNTVYLQIDSLKPEDTAVYYCYMLDTWGQGTQVTVSS

SEQ ID NO: 452 - protein, 5 aa, synthetic construct
YMADT

SEQ ID NO: 453 - protein, 136 aa, synthetic construct
EVQLVESGGGVVQPGGSLRLSCAASGEIFSINFMRWYRQAPGKQREWVAGFTRDGSTNYPDSAKGRFTISRDNAKNTVYLQIDSLKPEDTAVYYCYMADTWGQGTQVTVSSAAAEQKLISEEDLNGAAHHHHHHGS

SEQ ID NO: 454 - protein, 111 aa, synthetic construct
EVQLVESGGGVVQPGGSLRLSCAASGEIFSINFMRWYRQAPGKQREWVAGFTRDGSTNYPDSAKGRFTISRDNAKNTVYLQIDSLKPEDTAVYYCYMADTWGQGTQVTVSS

SEQ ID NO: 455 - protein, 5 aa, synthetic construct
YMQDT

SEQ ID NO: 456 - protein, 136 aa, synthetic construct
EVQLVESGGGVVQPGGSLRLSCAASGEIFSINFMRWYRQAPGKQREWVAGFTRDGSTNYPDSAKGRFTISRDNAKNTVYLQIDSLKPEDTAVYYCYMQDTWGQGTQVTVSSAAAEQKLISEEDLNGAAHHHHHHGS

SEQ ID NO: 457 - protein, 111 aa, synthetic construct
EVQLVESGGGVVQPGGSLRLSCAASGEIFSINFMRWYRQAPGKQREWVAGFTRDGSTNYPDSAKGRFTISRDNAKNTVYLQIDSLKPEDTAVYYCYMQDTWGQGTQVTVSS

SEQ ID NO: 458 - protein, 17 aa, synthetic construct
MRWYRQAPGKQREQVAG

SEQ ID NO: 459 - protein, 17 aa, synthetic construct
MRWYRQAPGKQREFVAG

SEQ ID NO: 460 - protein, 17 aa, synthetic construct
MRWYRQAPGKQRHWVAG

SEQ ID NO: 461 - protein, 17 aa, synthetic construct
MIWYRQAPGKQREWVAG

SEQ ID NO: 462 - protein, 17 aa, synthetic construct
MEWYRQAPGKQREWVAG

SEQ ID NO: 463 - protein, 17 aa, synthetic construct
MRWYRQAPGKQREWVAA

SEQ ID NO: 464 - protein, 17 aa, synthetic construct
MRWYRQAPGKQREWVAK

SEQ ID NO: 465 - RNA, 21 nt, synthetic construct
  source 1..21: mol_type = other RNA
  modified_base 7: mod_base = OTHER; note = 2'-deoxy-2'-fluoro
  modified_base 9..11: mod_base = OTHER; note = 2'-deoxy-2'-fluoro
  misc_feature 21: note = linker (conjugation handle)
  misc_feature 1..3: note = phosphorothioate internucleosidic linkage
  modified_base 1: mod_base = cm
  modified_base 2: mod_base = OTHER; note = 2'-O-methyl
  modified_base 3..6: mod_base = um
  modified_base 8: mod_base = OTHER; note = 2'-O-methyl
  modified_base 12: mod_base = um
  modified_base 13: mod_base = cm
  modified_base 14: mod_base = OTHER; note = 2'-O-methyl
  modified_base 15: mod_base = cm
  modified_base 16: mod_base = um
  modified_base 17: mod_base = cm
  modified_base 18: mod_base = um
  modified_base 19..21: mod_base = OTHER; note = 2'-O-methyl
cattttaatcctcactctaaa

SEQ ID NO: 466 - RNA, 23 nt, synthetic construct
  source 1..23: mol_type = other RNA
  modified_base 2: mod_base = OTHER; note = 2'-deoxy-2'-fluoro
  modified_base 6: mod_base = OTHER; note = 2'-deocy-2'-fluoro
  modified_base 8..9: mod_base = OTHER; note = 2'-deoxy-2'-fluoro
  modified_base 14: mod_base = OTHER; note = 2'-deoxy-2'-fluoro
  modified_base 16: mod_base = OTHER; note = 2'-deoxy-2'-fluoro
  misc_feature 1..3: note = phosphorothioate internucleosidic linkage
  misc_feature 21..23: note = phosphorothioate internucleosidic linkage
  modified_base 10..13: mod_base = OTHER; note = 2'-O-methyl
  modified_base 1: mod_base = um
  modified_base 3: mod_base = um
  modified_base 4: mod_base = OTHER; note = 2'-O-methyl
  modified_base 5: mod_base = gm
  modified_base 7: mod_base = gm
  modified_base 10: mod_base = OTHER; note = 2'-O-methyl
  modified_base 11..12: mod_base = gm
  modified_base 13: mod_base = OTHER; note = 2'-O-methyl
  modified_base 15: mod_base = um
  modified_base 17..18: mod_base = OTHER; note = 2'-O-methyl
  modified_base 19: mod_base = gm
  modified_base 20: mod_base = um
  modified_base 21: mod_base = gm
  modified_base 22: mod_base = OTHER; note = 2'-O-methyl
  modified_base 23: mod_base = gm
tttagagtgaggattaaaatgag

SEQ ID NO: 467 - RNA, 23 nt, synthetic construct
  source 1..23: mol_type = other RNA
  modified_base 7: mod_base = OTHER; note = 2'-deoxy-2'-fluoro
  modified_base 9..11: mod_base = OTHER; note = 2'-deoxy-2'-fluoro
  misc_feature 21: note = linker (conjugation handle)
  misc_feature 1..3: note = phosphorothioate internucleosidic linkage
  modified_base 1: mod_base = cm
  modified_base 2: mod_base = OTHER; note = 2'-O-methyl
  modified_base 3..6: mod_base = um
  modified_base 8: mod_base = OTHER; note = 2'-O-methyl
  modified_base 12: mod_base = um
  modified_base 13: mod_base = cm
  modified_base 14: mod_base = OTHER; note = 2'-O-methyl
  modified_base 15: mod_base = cm
  modified_base 16: mod_base = um
  modified_base 17: mod_base = cm
  modified_base 18: mod_base = um
  modified_base 19..21: mod_base = OTHER; note = 2'-O-methyl
  modified_base 22..23: mod_base = OTHER; note = deoxythymidine
cattttaatcctcactctaaatt

SEQ ID NO: 468 - RNA, 23 nt, synthetic construct
  source 1..23: mol_type = other RNA
  modified_base 2: mod_base = OTHER; note = 2'-deoxy-2'-fluoro
  modified_base 6: mod_base = OTHER; note = 2'-deocy-2'-fluoro
  modified_base 8..9: mod_base = OTHER; note = 2'-deoxy-2'-fluoro
  modified_base 14: mod_base = OTHER; note = 2'-deoxy-2'-fluoro
  modified_base 16: mod_base = OTHER; note = 2'-deoxy-2'-fluoro
  misc_feature 1..3: note = phosphorothioate internucleosidic linkage
  misc_feature 21..23: note = phosphorothioate internucleosidic linkage
  modified_base 10..13: mod_base = OTHER; note = 2'-O-methyl
  modified_base 1: mod_base = um
  modified_base 3: mod_base = um
  modified_base 4: mod_base = OTHER; note = 2'-O-methyl
  modified_base 5: mod_base = gm
  modified_base 7: mod_base = gm
  modified_base 10: mod_base = OTHER; note = 2'-O-methyl
  modified_base 11..12: mod_base = gm
  modified_base 13: mod_base = OTHER; note = 2'-O-methyl
  modified_base 15: mod_base = um
  modified_base 17..18: mod_base = OTHER; note = 2'-O-methyl
  modified_base 19: mod_base = gm
  modified_base 20: mod_base = um
  modified_base 21: mod_base = gm
  modified_base 22: mod_base = OTHER; note = 2'-O-methyl
  modified_base 23: mod_base = gm
tttagagtgaggattaaaatgag

SEQ ID NO: 469 - DNA, 411 bp, synthetic construct
  source 1..411: mol_type = other DNA
gaggtgcagctggtggagtctgggggaggcgtggtgcagcctggggggtctctaaaactctcctgcgtagcctcgggacatgacttcagtatcaattttatacgctggtaccgccaggctccagggaagcagcgcgagttcgtcgcaggatttactgcgactggtaacacaaactatgcagactccatgaaggggcgattcaccatctccagagacaacaccaagaacgcggtgtatctgcaaatagacagcctgaaacctgaggacacggccgtgtattactgctatatgttggacaagtggggccaggggacccaggtcaccgtctcctcagcggccgcagaacaaaaactcatctcagaagaggatctgaatggggccgcacatcaccaccatcaccatgggagctag

SEQ ID NO: 470 - DNA, 411 bp, synthetic construct
  source 1..411: mol_type = other DNA
gaggtgcagctggtggagtctgggggaggcgtggtgcagcctggggggtctctaaaactctcctgcgtagcctcgggaacggacttcagtatcaattttatacgctggtaccgccaggctccagggaagcagcgcgagttcgtcgcaggatggactgcgactggtaacacaaactatgcagactccatgaaggggcgattcaccatctccagagacaacaccaagaacgcggtgtatctgcaaatagacagcctgaaacctgaggacacggccgtgtattactgctatatgttggacaagtggggccaggggacccaggtcaccgtctcctcagcggccgcagaacaaaaactcatctcagaagaggatctgaatggggccgcacatcaccaccatcaccatgggagctag

SEQ ID NO: 471 - DNA, 411 bp, synthetic construct
  source 1..411: mol_type = other DNA
gaggtgcagctggtggagtctgggggaggcgtggtgcagcctggggggtctctaaaactctcctgcgtagcctcgggaacggacttcagtatcaattttatacgctggtaccgccaggctccagggaagcagcgcgagttcgtcgcaggatatactgcgactggtaacacaaactatgcagactccatgaaggggcgattcaccatctccagagacaacaccaagaacgcggtgtatctgcaaatagacagcctgaaacctgaggacacggccgtgtattactgctatatgttggacaagtggggccaggggacccaggtcaccgtctcctcagcggccgcagaacaaaaactcatctcagaagaggatctgaatggggccgcacatcaccaccatcaccatgggagctag

SEQ ID NO: 472 - DNA, 411 bp, synthetic construct
  source 1..411: mol_type = other DNA
gaggtgcagctggtggagtctgggggaggcgtggtgcagcctggggggtctctaaaactctcctgcgtagcctcgggaacggacttcagtatcaattttatacgctggtaccgccaggctccagggaagcagcgcgagttcgtcgcaggatttactgcgactggtaacacaaactatgcagactccatgaaggggcgattcaccatctccagagacaacaccaagaacgcggtgtatctgcaaatagacagcctgaaacctgaggacacggccgtgtattactgccatatgttggacaagtggggccaggggacccaggtcaccgtctcctcagcggccgcagaacaaaaactcatctcagaagaggatctgaatggggccgcacatcaccaccatcaccatgggagctag

SEQ ID NO: 473 - DNA, 411 bp, synthetic construct
  source 1..411: mol_type = other DNA
gaggtgcagctggtggagtctgggggaggcgtggtgcagcctggggggtctctaaaactctcctgcgtagcctcgggaacggacttcagtatcaattttatacgctggtaccgccaggctccagggaagcagcgcgagttcgtcgcaggatttactgcgactggtaacacaaactatgcagactccatgaaggggcgattcaccatctccagagacaacaccaagaacgcggtgtatctgcaaatagacagcctgaaacctgaggacacggccgtgtattactgctggatgttggacaagtggggccaggggacccaggtcaccgtctcctcagcggccgcagaacaaaaactcatctcagaagaggatctgaatggggccgcacatcaccaccatcaccatgggagctag

SEQ ID NO: 474 - DNA, 411 bp, synthetic construct
  source 1..411: mol_type = other DNA
gaggtgcagctggtggagtctgggggaggcgtggtgcagcctggggggtctctaaaactctcctgcgtagcctcgggaacggacttcagtatcaattttatacgctggtaccgccaggctccagggaagcagcgcgagttcgtcgcaggatttactgcgactggtaacacaaactatgcagactccatgaaggggcgattcaccatctccagagacaacaccaagaacgcggtgtatctgcaaatagacagcctgaaacctgaggacacggccgtgtattactgctatctgttggacaagtggggccaggggacccaggtcaccgtctcctcagcggccgcagaacaaaaactcatctcagaagaggatctgaatggggccgcacatcaccaccatcaccatgggagctag

SEQ ID NO: 475 - DNA, 411 bp, synthetic construct
  source 1..411: mol_type = other DNA
gaggtgcagctggtggagtctgggggaggcgtggtgcagcctggggggtctctaaaactctcctgcgtagcctcgggaacggacttcagtatcaattttatacgctggtaccgccaggctccagggaagcagcgcgagttcgtcgcaggatttactgcgactggtaacacaaactatgcagactccatgaaggggcgattcaccatctccagagacaacaccaagaacgcggtgtatctgcaaatagacagcctgaaacctgaggacacggccgtgtattactgctatgttttggacaagtggggccaggggacccaggtcaccgtctcctcagcggccgcagaacaaaaactcatctcagaagaggatctgaatggggccgcacatcaccaccatcaccatgggagctag

SEQ ID NO: 476 - DNA, 411 bp, synthetic construct
  source 1..411: mol_type = other DNA
gaggtgcagctggtggagtctgggggaggcgtggtgcagcctggggggtctctaaaactctcctgcgtagcctcgggagcggacttcagtatcaattatatacgctggtaccgccaggctccagggaagcagcgcgagttcgtcgcaggatttactgcgactggtaacacaaactatgcagactccatgaaggggcgattcaccatctccagagacaacaccaagaacgcggtgtatctgcaaatagacagcctgaaacctgaggacacggccgtgtattactgctatatgttggacaagtggggccaggggacccaggtcaccgtctcctcagcggccgcagaacaaaaactcatctcagaagaggatctgaatggggccgcacatcaccaccatcaccatgggagctag

SEQ ID NO: 477 - DNA, 411 bp, synthetic construct
  source 1..411: mol_type = other DNA
gaggtgcagctggtggagtctgggggaggcgtggtgcagcctggggggtctctaaaactctcctgcgtagcctcgggagcggacttcagtatcaattttatacgctggtaccgccaggctccagggaagcagcgcgagttcgtcgcaggatttagcgcgactggtaacacaaactatgcagactccatgaaggggcgattcaccatctccagagacaacaccaagaacgcggtgtatctgcaaatagacagcctgaaacctgaggacacggccgtgtattactgctatatgttggacaagtggggccaggggacccaggtcaccgtctcctcagcggccgcagaacaaaaactcatctcagaagaggatctgaatggggccgcacatcaccaccatcaccatgggagctag

SEQ ID NO: 478 - DNA, 411 bp, synthetic construct
  source 1..411: mol_type = other DNA
gaggtgcagctggtggagtctgggggaggcgtggtgcagcctggggggtctctaaaactctcctgcgtagcctcgggagcggacttcagtatcaattttatacgctggtaccgccaggctccagggaagcagcgcgagttcgtcgcaggatttactgcgactggtcatacaaactatgcagactccatgaaggggcgattcaccatctccagagacaacaccaagaacgcggtgtatctgcaaatagacagcctgaaacctgaggacacggccgtgtattactgctatatgttggacaagtggggccaggggacccaggtcaccgtctcctcagcggccgcagaacaaaaactcatctcagaagaggatctgaatggggccgcacatcaccaccatcaccatgggagctag

SEQ ID NO: 479 - DNA, 411 bp, synthetic construct
  source 1..411: mol_type = other DNA
gaggtgcagctggtggagtctgggggaggcgtggtgcagcctggggggtctctacgtctctcctgcgcagcctcgggaacggacttcagtatcaattttatacgctgggttcgccaggctccagggaagggtctggagtgggtcgcaggatttactgcgactggtaacacaaactatgcagactccgttaaggggcgattcaccatctccagagacaacaccaagaacaccctgtatctgcaaatagacagcctgcgtcctgaggacacggccgtgtattactgctatatgttggacaagtggggccaggggacccaggtcaccgtctcctcagcggccgcagaacaaaaactcatctcagaagaggatctgaatggggccgcacatcaccaccatcaccatgggagctag

SEQ ID NO: 480 - DNA, 411 bp, synthetic construct
  source 1..411: mol_type = other DNA
gaggtgcagctggtggagtctgggggaggcgtggtgcagcctggggggtctctacgtctctcctgcgcagcctcgggaacggacttcagtatcaattttatacgctggtaccgccaggctccagggaagggtctggagttcgtcgcaggatttactgcgactggtaacacaaactatgcagactccgttaaggggcgattcaccatctccagagacaacgcaaagaacaccctgtatctgcaaatgaatagcctgcgtcctgaggacacggccgtgtattactgctatatgttggacaagtggggccaggggacccaggtcaccgtctcctcagcggccgcagaacaaaaactcatctcagaagaggatctgaatggggccgcacatcaccaccatcaccatgggagctag

SEQ ID NO: 481 - DNA, 411 bp, synthetic construct
  source 1..411: mol_type = other DNA
gaggtgcagctggtggagtctgggggaggcgtggtgcagcctggggggtctctaaaactctcctgcgcagcctcgggaacggacttcagtatcaattttatacgctgggttcgccaggctccagggaagggtctggagtgggtcgcaggatttactgcgactggtaacacaaactatgcagactccgttaaggggcgattcaccatctccagagacaacaccaagaacaccctgtatctgcaaataaatagcctgcgtcctgaggacacggccgtgtattactgctatatgttggacaagtggggccaggggacccaggtcaccgtctcctcagcggccgcagaacaaaaactcatctcagaagaggatctgaatggggccgcacatcaccaccatcaccatgggagctag

SEQ ID NO: 482 - DNA, 411 bp, synthetic construct
  source 1..411: mol_type = other DNA
gaggtgcagctggtggagtctgggggaggcgtggtgcagcctggggggtctctacgtctctcctgcgcagcctcgggaacggacttcagtatcaattttatacgctgggttcgccaggctccagggaagggtctggagtgggtcgcaggatttactgcgactggtaacacaaactatgcagactccatgaaggggcgattcaccatctccagagacaacaccaagaacaccctgtatctgcaaatgaatagcctgcgtcctgaggacacggccgtgtattactgctatatgttggacaagtggggccaggggacccaggtcaccgtctcctcagcggccgcagaacaaaaactcatctcagaagaggatctgaatggggccgcacatcaccaccatcaccatgggagctag

SEQ ID NO: 483 - DNA, 411 bp, synthetic construct
  source 1..411: mol_type = other DNA
gaggtgcagctggtggagtctgggggaggcgtggtgcagcctggggggtctctacgtctctcctgcgcagcctcgggaacggacttcagtatcaattttatacgctggtaccgccaggctccagggaagggtctggagttcgtcgcaggatttactgcgactggtaacacaaactatgcagactccgttaaggggcgattcaccatctccagagacaacgcaaagaacaccctgtatctgcaaatagacagcctgcgtcctgaggacacggccgtgtattactgctatatgttggacaagtggggccaggggacccaggtcaccgtctcctcagcggccgcagaacaaaaactcatctcagaagaggatctgaatggggccgcacatcaccaccatcaccatgggagctag

SEQ ID NO: 484 - DNA, 411 bp, synthetic construct
  source 1..411: mol_type = other DNA
gaggtgcagctggtggagtctgggggaggcgtggtgcagcctggggggtctctacgtctctcctgcgcagcctcgggaacggacttcagtatcaattttatacgctggtaccgccaggctccagggaagggtctggagttcgtcgcaggatttactgcgactggtaacacaaactatgcagactccgttaaggggcgattcaccatctccagagacaacaccaagaacaccctgtatctgcaaatgaatagcctgcgtcctgaggacacggccgtgtattactgctatatgttggacaagtggggccaggggacccaggtcaccgtctcctcagcggccgcagaacaaaaactcatctcagaagaggatctgaatggggccgcacatcaccaccatcaccatgggagctag

SEQ ID NO: 485 - DNA, 411 bp, synthetic construct
  source 1..411: mol_type = other DNA
gaggtgcagctggtggagtctgggggaggcgtggtgcagcctggggggtctctacgtctctcctgcgcagcctcgggaacggacttcagtatcaattttatacgctgggttcgccaggctccagggaagggtctggagtgggtcgcaggatttactgcgactggtaacacaaactatgcagactccgttaaggggcgattcaccatctccagagacaacaccaagaacgcgctgtatctgcaaatgaatagcctgcgtcctgaggacacggccgtgtattactgctatatgttggacaagtggggccaggggacccaggtcaccgtctcctcagcggccgcagaacaaaaactcatctcagaagaggatctgaatggggccgcacatcaccaccatcaccatgggagctag

SEQ ID NO: 486 - DNA, 411 bp, synthetic construct
  source 1..411: mol_type = other DNA
gaggtgcagctggtggagtctgggggaggcgtggtgcagcctggggggtctctacgtctctcctgcgtagcctcgggaacggacttcagtatcaattttatacgctgggttcgccaggctccagggaagggtctggagtgggtcgcaggatttactgcgactggtaacacaaactatgcagactccgttaaggggcgattcaccatctccagagacaacaccaagaacaccctgtatctgcaaatggacagcctgcgtcctgaggacacggccgtgtattactgctatatgttggacaagtggggccaggggacccaggtcaccgtctcctcagcggccgcagaacaaaaactcatctcagaagaggatctgaatggggccgcacatcaccaccatcaccatgggagctag

SEQ ID NO: 487 - DNA, 411 bp, synthetic construct
  source 1..411: mol_type = other DNA
gaggtgcagctggtggagtctgggggaggcctggtgcagcctggggggtctctacgtctctcctgcgcagcctcgggaacggacttcagtatcaattttatacgctggtaccgccaggctccagggaagggtctggagttcgtcgcaggatttactgcgactggtaacacaaactatgcagactccgttaaggggcgattcaccatctccagagacaacagcaagaacaccctgtatctgcaaatgaatagcctgcgtgcagaggacacggccgtgtattactgctatatgttggacaagtggggccaggggaccctggtcaccgtctcctcagcggccgcagaacaaaaactcatctcagaagaggatctgaatggggccgcacatcaccaccatcaccatgggagctag

SEQ ID NO: 488 - DNA, 411 bp, synthetic construct
  source 1..411: mol_type = other DNA
gaggtgcagctggtggagtctgggggaggcgtggtgcagcctggggggtctctaaaactctcctgcgtagcctcgggaacggacttcagtatcaattttatacgctgggttcgccaggctccagggaagggtctggagttcgtcgcaggatttactgcgactggtaacacaaactatgcagactccatgaaggggcgattcaccatctccagagacaacaccaagaacgcgctgtatctgcaaatagacagcctgcgtcctgaggacacggccgtgtattactgctatatgttggacaagtggggccaggggacccaggtcaccgtctcctcagcggccgcagaacaaaaactcatctcagaagaggatctgaatggggccgcacatcaccaccatcaccatgggagctag

SEQ ID NO: 489 - DNA, 411 bp, synthetic construct
  source 1..411: mol_type = other DNA
gaggtgcagctggtggagtctgggggaggcgtggtgcagcctggggggtctctaaaactctcctgcgtagcctcgggaacggacttcagtatcaattttatacgctggtaccgccaggctccagggaagggtctggagttcgtcgcaggatttactgcgactggtaacacaaactatgcagactccgttaaggggcgattcaccatctccagagacaacgcaaagaacaccctgtatctgcaaatgaatagcctgcgtcctgaggacacggccgtgtattactgctatatgttggacaagtggggccaggggacccaggtcaccgtctcctcagcggccgcagaacaaaaactcatctcagaagaggatctgaatggggccgcacatcaccaccatcaccatgggagctag

SEQ ID NO: 490 - DNA, 411 bp, synthetic construct
  source 1..411: mol_type = other DNA
gaggtgcagctggtggagtctgggggaggcgtggtgcagcctggggggtctctacgtctctcctgcgcagcctcgggaacggacttcagtatcaattttatacgctggtaccgccaggctccagggaagcagcgcgagttcgtcgcaggatttactgcgactggtaacacaaactatgcagactccgttaaggggcgattcaccatctccagagacaacgcaaagaacaccctgtatctgcaaatgaatagcctgcgtcctgaggacacggccgtgtattactgctatatgttggacaagtggggccaggggacccaggtcaccgtctcctcagcggccgcagaacaaaaactcatctcagaagaggatctgaatggggccgcacatcaccaccatcaccatgggagctag

SEQ ID NO: 491 - DNA, 411 bp, synthetic construct
  source 1..411: mol_type = other DNA
gaggtgcagctggtggagtctgggggaggcgtggtgcagcctggggggtctctacgtctctcctgcgcagcctcgggaacggacttcagtatcaattttatacgctggtaccgccaggctccagggaagggtctggagttcgtcgcaggatttactgcgactggtaacacaaactatgcagactccgttaaggggcgattcaccatctccagagacaacgcaaagaacgcggtgtatctgcaaatgaatagcctgcgtcctgaggacacggccgtgtattactgctatatgttggacaagtggggccaggggacccaggtcaccgtctcctcagcggccgcagaacaaaaactcatctcagaagaggatctgaatggggccgcacatcaccaccatcaccatgggagctag

SEQ ID NO: 492 - DNA, 411 bp, synthetic construct
  source 1..411: mol_type = other DNA
gaggtgcagctggtggagtctgggggaggcgtggtgcagcctggggggtctctacgtctctcctgcgcagcctcgggaacggacttcagtatcaattttatacgctggtaccgccaggctccagggaagggtctggagttcgtcgcaggatttactgcgactggtaacacaaactatgcagactccgttaaggggcgattcaccatctccagagacaacgcaaagaacaccctgtatctgcaaatgaatagcctgaaacctgaggacacggccgtgtattactgctatatgttggacaagtggggccaggggacccaggtcaccgtctcctcagcggccgcagaacaaaaactcatctcagaagaggatctgaatggggccgcacatcaccaccatcaccatgggagctag

SEQ ID NO: 493 - DNA, 411 bp, synthetic construct
  source 1..411: mol_type = other DNA
gaggtgcagctggtggagtctgggggaggcgtggtgcagcctggggggtctctacgtctctcctgcgcagcctcgggaacggacttcagtatcaattttatacgctggtaccgccaggctccagggaagggtcgcgagttcgtcgcaggatttactgcgactggtaacacaaactatgcagactccgttaaggggcgattcaccatctccagagacaacgcaaagaacaccctgtatctgcaaatgaatagcctgcgtcctgaggacacggccgtgtattactgctatatgttggacaagtggggccaggggacccaggtcaccgtctcctcagcggccgcagaacaaaaactcatctcagaagaggatctgaatggggccgcacatcaccaccatcaccatgggagctag

SEQ ID NO: 494 - DNA, 411 bp, synthetic construct; identical to SEQ ID NO: 106
  source 1..411: mol_type = other DNA

SEQ ID NO: 495 - DNA, 411 bp, synthetic construct
  source 1..411: mol_type = other DNA
gaggtgcagctggtggagtctgggggaggcgtggtgcagcctggggggtctctacgtctctcctgcgcagcctcgggaacggacttcagtatcaattttatacgctggtaccgccaggctccagggaagggtctggagttcgtcgcaggatttactgcgactggtaacacaaactatgcagactccatgaaggggcgattcaccatctccagagacaacgcaaagaacaccctgtatctgcaaatgaatagcctgcgtcctgaggacacggccgtgtattactgctatatgttggacaagtggggccaggggacccaggtcaccgtctcctcagcggccgcagaacaaaaactcatctcagaagaggatctgaatggggccgcacatcaccaccatcaccatgggagctag

SEQ ID NO: 496 - DNA, 411 bp, synthetic construct
  source 1..411: mol_type = other DNA
gaggtgcagctggtggagtctgggggaggcgtggtgcagcctggggggtctctacgtctctcctgcgcagcctcgggaacggacttcagtatcaattttatacgctgggttcgccaggctccagggaagggtctggagttcgtcgcaggatttactgcgactggtaacacaaactatgcagactccgttaaggggcgattcaccatctccagagacaacgcaaagaacaccctgtatctgcaaatagacagcctgcgtcctgaggacacggccgtgtattactgctatatgttggacaagtggggccaggggacccaggtcaccgtctcctcagcggccgcagaacaaaaactcatctcagaagaggatctgaatggggccgcacatcaccaccatcaccatgggagctag

SEQ ID NO: 497 - DNA, 411 bp, synthetic construct
  source 1..411: mol_type = other DNA
gaggtgcagctggtggagtctgggggaggcgtggtgcagcctggggggtctctacgtctctcctgcgcagcctcgggaacggacttcagtatcaattttatacgctggtaccgccaggctccagggaagggtctggagtgggtcgcaggatttactgcgactggtaacacaaactatgcagactccgttaaggggcgattcaccatctccagagacaacgcaaagaacaccctgtatctgcaaatagacagcctgcgtcctgaggacacggccgtgtattactgctatatgttggacaagtggggccaggggacccaggtcaccgtctcctcagcggccgcagaacaaaaactcatctcagaagaggatctgaatggggccgcacatcaccaccatcaccatgggagctag

SEQ ID NO: 498 - DNA, 411 bp, synthetic construct
  source 1..411: mol_type = other DNA
gaggtgcagctggtggagtctgggggaggcgtggtgcagcctggggggtctctaaaactctcctgcgtagcctcgggaacggacttcagtatcaattttatacgctggtaccgccaggctccagggaagcagcgcgagttcgtcgcaggatttactgcgactggtaacacaaactatgcagactccatgaaggggcgattcaccatctccagagacaacaccaagaacgcggtgtatctgcaaatagacagcctgaaacctgaggacacggccgtgtattactgcgcgatggcggacaagtggggccaggggacccaggtcaccgtctcctcagcggccgcagaacaaaaactcatctcagaagaggatctgaatggggccgcacatcaccaccatcaccatgggagctag

SEQ ID NO: 499 - DNA, 411 bp, synthetic construct
  source 1..411: mol_type = other DNA
gaggtgcagctggtggagtctgggggaggcgtggtgcagcctggggggtctctgagactctcctgtgcagcctctggagagatcttcagtatcaattttatgcgctggtaccgccaggctccagggaagggtctggagtgggtcgcaggttttactagggatggaagcacaaactatccagactccgttaagggccgattcaccatctctagagacaacgccaagaacacggtgtatctgcaaatgaatagcctgcgtcctgaggacacggccgtctattattgttatatgttggacacctggggccaggggacccaggtcactgtctcctcagcggccgcagaacaaaaactcatctcagaagaggatctgaatggggccgcacatcaccaccatcaccatgggagctag

SEQ ID NO: 500 - DNA, 411 bp, synthetic construct
  source 1..411: mol_type = other DNA
gaggtgcagctggtggagtctgggggaggcgtggtgcagcctggggggtctctacgtctctcctgcgcagcctcgggaacggacttcagtatcaattttatacgctggtaccgccaggctccagggaagggtctggagttcgtcgcaggattttcagcgactggtaacacaaactatgcagactccgttaaggggcgattcaccatctccagagacaacgcaaagaacgcggtgtatctgcaaatgaatagcctgcgtcctgaggacacggccgtgtattactgctatatgttggacaagtggggccaggggacccaggtcaccgtctcctcagcggccgcagaacaaaaactcatctcagaagaggatctgaatggggccgcacatcaccaccatcaccatgggagctag

SEQ ID NO: 501 - DNA, 411 bp, synthetic construct
  source 1..411: mol_type = other DNA
gaggtgcagctggtggagtctgggggaggcgtggtgcagcctggggggtctctacgtctctcctgcgcagcctcgggaacggacttcagtatcaattttatacgctggtaccgccaggctccagggaagggtctggagttcgtcgcaggatttactgcgactggtaacacaaactatgcagactccgttaaggggcgattcaccatctccagagacaacgcaaagaacgcggtgtatctgcaaatgaatagcctgcgtcctgaggacacggccgtgtattactgctatattttggacaagtggggccaggggacccaggtcaccgtctcctcagcggccgcagaacaaaaactcatctcagaagaggatctgaatggggccgcacatcaccaccatcaccatgggagctag

SEQ ID NO: 502 - DNA, 411 bp, synthetic construct
  source 1..411: mol_type = other DNA
gaggtgcagctggtggagtctgggggaggcgtggtgcagcctggggggtctctgagactctcctgtgcagccgatggagagatcttcagtatcaattttatgcgctggtaccgccaggctccagggaagcagcgcgagtgggtcgcaggttttactagggatggaagcacaaactatccagactccgcgaagggccgattcaccatctctagagacaacgccaagaacacggtgtatctgcaaatagacagcctgaaacctgaggacacggccgtctattattgttatatgttggacacctggggccaggggacccaggtcactgtctcctcagcggccgcagaacaaaaactcatctcagaagaggatctgaatggggccgcacatcaccaccatcaccatgggagctag

SEQ ID NO: 503 - DNA, 411 bp, synthetic construct
  source 1..411: mol_type = other DNA
gaggtgcagctggtggagtctgggggaggcgtggtgcagcctggggggtctctgagactctcctgtgcagcctctggagagatcttcagtatcaattttatgcgctggtacggccaggctccagggaagcagcgcgagtgggtcgcaggttttactagggatggaagcacaaactatccagactccgcgaagggccgattcaccatctctagagacaacgccaagaacacggtgtatctgcaaatagacagcctgaaacctgaggacacggccgtctattattgttatatgttggacacctggggccaggggacccaggtcactgtctcctcagcggccgcagaacaaaaactcatctcagaagaggatctgaatggggccgcacatcaccaccatcaccatgggagctag

SEQ ID NO: 504 - DNA, 411 bp, synthetic construct
  source 1..411: mol_type = other DNA
gaggtgcagctggtggagtctgggggaggcgtggtgcagcctggggggtctctgagactctcctgtgcagcctctggagagatcttcagtatcaattttatgcgctggtaccgcgaagctccagggaagcagcgcgagtgggtcgcaggttttactagggatggaagcacaaactatccagactccgcgaagggccgattcaccatctctagagacaacgccaagaacacggtgtatctgcaaatagacagcctgaaacctgaggacacggccgtctattattgttatatgttggacacctggggccaggggacccaggtcactgtctcctcagcggccgcagaacaaaaactcatctcagaagaggatctgaatggggccgcacatcaccaccatcaccatgggagctag

SEQ ID NO: 505 - DNA, 411 bp, synthetic construct
  source 1..411: mol_type = other DNA
gaggtgcagctggtggagtctgggggaggcgtggtgcagcctggggggtctctgagactctcctgtgcagcctctggagagatcttcagtatcaattttatgcgctggtaccgccaggctccaattaagcagcgcgagtgggtcgcaggttttactagggatggaagcacaaactatccagactccgcgaagggccgattcaccatctctagagacaacgccaagaacacggtgtatctgcaaatagacagcctgaaacctgaggacacggccgtctattattgttatatgttggacacctggggccaggggacccaggtcactgtctcctcagcggccgcagaacaaaaactcatctcagaagaggatctgaatggggccgcacatcaccaccatcaccatgggagctag

SEQ ID NO: 506 - DNA, 411 bp, synthetic construct
  source 1..411: mol_type = other DNA
gaggtgcagctggtggagtctgggggaggcgtggtgcagcctggggggtctctgagactctcctgtgcagcctctggagagatcttcagtatcaattttatgcgctggtaccgccaggctccagggaagattcgcgagtgggtcgcaggttttactagggatggaagcacaaactatccagactccgcgaagggccgattcaccatctctagagacaacgccaagaacacggtgtatctgcaaatagacagcctgaaacctgaggacacggccgtctattattgttatatgttggacacctggggccaggggacccaggtcactgtctcctcagcggccgcagaacaaaaactcatctcagaagaggatctgaatggggccgcacatcaccaccatcaccatgggagctag

SEQ ID NO: 507 - DNA, 411 bp, synthetic construct
  source 1..411: mol_type = other DNA
gaggtgcagctggtggagtctgggggaggcgtggtgcagcctggggggtctctgagactctcctgtgcagcctctggagagatcttcagtatcaattttatgcgctggtaccgccaggctccagggaagcagcgcgagtgggtcgcaggttttactagggatggatttacaaactatccagactccgcgaagggccgattcaccatctctagagacaacgccaagaacacggtgtatctgcaaatagacagcctgaaacctgaggacacggccgtctattattgttatatgttggacacctggggccaggggacccaggtcactgtctcctcagcggccgcagaacaaaaactcatctcagaagaggatctgaatggggccgcacatcaccaccatcaccatgggagctag

SEQ ID NO: 508 - DNA, 411 bp, synthetic construct
  source 1..411: mol_type = other DNA
gaggtgcagctggtggagtctgggggaggcgtggtgcagcctggggggtctctgagactctcctgtgcagcctctggagagatcttcagtatcaattttatgcgctggtaccgccaggctccagggaagcagcgcgagtgggtcgcaggttttactagggatggatatacaaactatccagactccgcgaagggccgattcaccatctctagagacaacgccaagaacacggtgtatctgcaaatagacagcctgaaacctgaggacacggccgtctattattgttatatgttggacacctggggccaggggacccaggtcactgtctcctcagcggccgcagaacaaaaactcatctcagaagaggatctgaatggggccgcacatcaccaccatcaccatgggagctag

SEQ ID NO: 509 - DNA, 411 bp, synthetic construct
  source 1..411: mol_type = other DNA
gaggtgcagctggtggagtctgggggaggcgtggtgcagcctggggggtctctgagactctcctgtgcagcctctggagagatcttcagtatcaattttatgcgctggtaccgccaggctccagggaagcagcgcgagtgggtcgcaggttttactagggatggaagcctgaactatccagactccgcgaagggccgattcaccatctctagagacaacgccaagaacacggtgtatctgcaaatagacagcctgaaacctgaggacacggccgtctattattgttatatgttggacacctggggccaggggacccaggtcactgtctcctcagcggccgcagaacaaaaactcatctcagaagaggatctgaatggggccgcacatcaccaccatcaccatgggagctag

SEQ ID NO: 510 - DNA, 411 bp, synthetic construct
  source 1..411: mol_type = other DNA
gaggtgcagctggtggagtctgggggaggcgtggtgcagcctggggggtctctgagactctcctgtgcagcctctggagagatcttcagtatcaattttatgcgctggtaccgccaggctccagggaagcagcgcgagtgggtcgcaggttttactagggatggaagcaaaaactatccagactccgcgaagggccgattcaccatctctagagacaacgccaagaacacggtgtatctgcaaatagacagcctgaaacctgaggacacggccgtctattattgttatatgttggacacctggggccaggggacccaggtcactgtctcctcagcggccgcagaacaaaaactcatctcagaagaggatctgaatggggccgcacatcaccaccatcaccatgggagctag

SEQ ID NO: 511 - DNA, 411 bp, synthetic construct
  source 1..411: mol_type = other DNA
gaggtgcagctggtggagtctgggggaggcgtggtgcagcctggggggtctctgagactctcctgtgcagcctctgatgagatcttcagtatcaattttatgcgctggtaccgccaggctccagggaagcagcgcgagtgggtcgcaggttttactagggatggaagcacaaactatccagactccgcgaagggccgattcaccatctctagagacaacgccaagaacacggtgtatctgcaaatagacagcctgaaacctgaggacacggccgtctattattgttatatgttggacacctggggccaggggacccaggtcactgtctcctcagcggccgcagaacaaaaactcatctcagaagaggatctgaatggggccgcacatcaccaccatcaccatgggagctag

SEQ ID NO: 512 - DNA, 411 bp, synthetic construct
  source 1..411: mol_type = other DNA
gaggtgcagctggtggagtctgggggaggcgtggtgcagcctggggggtctctgagactctcctgtgcagcctctggagagatcttctatatcaattttatgcgctggtaccgccaggctccagggaagcagcgcgagtgggtcgcaggttttactagggatggaagcacaaactatccagactccgcgaagggccgattcaccatctctagagacaacgccaagaacacggtgtatctgcaaatagacagcctgaaacctgaggacacggccgtctattattgttatatgttggacacctggggccaggggacccaggtcactgtctcctcagcggccgcagaacaaaaactcatctcagaagaggatctgaatggggccgcacatcaccaccatcaccatgggagctag

SEQ ID NO: 513 - DNA, 411 bp, synthetic construct
  source 1..411: mol_type = other DNA
gaggtgcagctggtggagtctgggggaggcgtggtgcagcctggggggtctctgagactctcctgtgcagcctctggagagatcttcagtatcaattttatgcgctggtaccgccaggctccagggaagcagcgcgagtgggtcgcaggttttactaggctgggaagcacaaactatccagactccgcgaagggccgattcaccatctctagagacaacgccaagaacacggtgtatctgcaaatagacagcctgaaacctgaggacacggccgtctattattgttatatgttggacacctggggccaggggacccaggtcactgtctcctcagcggccgcagaacaaaaactcatctcagaagaggatctgaatggggccgcacatcaccaccatcaccatgggagctag

SEQ ID NO: 514 - DNA, 411 bp, synthetic construct
  source 1..411: mol_type = other DNA
gaggtgcagctggtggagtctgggggaggcgtggtgcagcctggggggtctctgagactctcctgtgcagcctctggagagatcttcagtatcaattttatgcgctggtaccgccaggctccagggaagcagcgcgagtgggtcgcaggttttactagggatgatagcacaaactatccagactccgcgaagggccgattcaccatctctagagacaacgccaagaacacggtgtatctgcaaatagacagcctgaaacctgaggacacggccgtctattattgttatatgttggacacctggggccaggggacccaggtcactgtctcctcagcggccgcagaacaaaaactcatctcagaagaggatctgaatggggccgcacatcaccaccatcaccatgggagctag

SEQ ID NO: 515 - DNA, 411 bp, synthetic construct
  source 1..411: mol_type = other DNA
gaggtgcagctggtggagtctgggggaggcgtggtgcagcctggggggtctctgagactctcctgtgcagcctctggagagatcttcagtatcaattttatgcgctggtaccgccaggctccagggaagcagcgcgagcaggtcgcaggttttactagggatggaagcacaaactatccagactccgcgaagggccgattcaccatctctagagacaacgccaagaacacggtgtatctgcaaatagacagcctgaaacctgaggacacggccgtctattattgttatatgttggacacctggggccaggggacccaggtcactgtctcctcagcggccgcagaacaaaaactcatctcagaagaggatctgaatggggccgcacatcaccaccatcaccatgggagctag

SEQ ID NO: 516 - DNA, 411 bp, synthetic construct
  source 1..411: mol_type = other DNA
gaggtgcagctggtggagtctgggggaggcgtggtgcagcctggggggtctctgagactctcctgtgcagcctctggagagatcttcagtatcaattttatgcgctggtaccgccaggctccagggaagcagcgcgagtttgtcgcaggttttactagggatggaagcacaaactatccagactccgcgaagggccgattcaccatctctagagacaacgccaagaacacggtgtatctgcaaatagacagcctgaaacctgaggacacggccgtctattattgttatatgttggacacctggggccaggggacccaggtcactgtctcctcagcggccgcagaacaaaaactcatctcagaagaggatctgaatggggccgcacatcaccaccatcaccatgggagctag

SEQ ID NO: 517 - DNA, 411 bp, synthetic construct
  source 1..411: mol_type = other DNA
gaggtgcagctggtggagtctgggggaggcgtggtgcagcctggggggtctctgagactctcctgtgcagcctctggagagatccatagtatcaattttatgcgctggtaccgccaggctccagggaagcagcgcgagtgggtcgcaggttttactagggatggaagcacaaactatccagactccgcgaagggccgattcaccatctctagagacaacgccaagaacacggtgtatctgcaaatagacagcctgaaacctgaggacacggccgtctattattgttatatgttggacacctggggccaggggacccaggtcactgtctcctcagcggccgcagaacaaaaactcatctcagaagaggatctgaatggggccgcacatcaccaccatcaccatgggagctag

SEQ ID NO: 518 - DNA, 411 bp, synthetic construct
  source 1..411: mol_type = other DNA
gaggtgcagctggtggagtctgggggaggcgtggtgcagcctggggggtctctgagactctcctgtgcagcctctggagagatcttcagtatcaattttatgcgctggtaccgccaggctccagggaagcagcgccattgggtcgcaggttttactagggatggaagcacaaactatccagactccgcgaagggccgattcaccatctctagagacaacgccaagaacacggtgtatctgcaaatagacagcctgaaacctgaggacacggccgtctattattgttatatgttggacacctggggccaggggacccaggtcactgtctcctcagcggccgcagaacaaaaactcatctcagaagaggatctgaatggggccgcacatcaccaccatcaccatgggagctag

SEQ ID NO: 519 - DNA, 411 bp, synthetic construct
  source 1..411: mol_type = other DNA
gaggtgcagctggtggagtctgggggaggcgtggtgcagcctggggggtctctgagactctcctgtgcagcctctggagagatcttcagtatcaattttatgcgctggtaccgccaggctccagggaagcagcgcgagtgggtcgcaggttttactagggatggaagccataactatccagactccgcgaagggccgattcaccatctctagagacaacgccaagaacacggtgtatctgcaaatagacagcctgaaacctgaggacacggccgtctattattgttatatgttggacacctggggccaggggacccaggtcactgtctcctcagcggccgcagaacaaaaactcatctcagaagaggatctgaatggggccgcacatcaccaccatcaccatgggagctag

SEQ ID NO: 520 - DNA, 411 bp, synthetic construct
  source 1..411: mol_type = other DNA
gaggtgcagctggtggagtctgggggaggcgtggtgcagcctggggggtctctgagactctcctgtgcagcctctggagagatcttcagtatcaataacatgcgctggtaccgccaggctccagggaagcagcgcgagtgggtcgcaggttttactagggatggaagcacaaactatccagactccgcgaagggccgattcaccatctctagagacaacgccaagaacacggtgtatctgcaaatagacagcctgaaacctgaggacacggccgtctattattgttatatgttggacacctggggccaggggacccaggtcactgtctcctcagcggccgcagaacaaaaactcatctcagaagaggatctgaatggggccgcacatcaccaccatcaccatgggagctag

SEQ ID NO: 521 - DNA, 411 bp, synthetic construct
  source 1..411: mol_type = other DNA
gaggtgcagctggtggagtctgggggaggcgtggtgcagcctggggggtctctgagactctcctgtgcagcctctggagagatcttcagtatcaatcagatgcgctggtaccgccaggctccagggaagcagcgcgagtgggtcgcaggttttactagggatggaagcacaaactatccagactccgcgaagggccgattcaccatctctagagacaacgccaagaacacggtgtatctgcaaatagacagcctgaaacctgaggacacggccgtctattattgttatatgttggacacctggggccaggggacccaggtcactgtctcctcagcggccgcagaacaaaaactcatctcagaagaggatctgaatggggccgcacatcaccaccatcaccatgggagctag

SEQ ID NO: 522 - DNA, 411 bp, synthetic construct
  source 1..411: mol_type = other DNA
gaggtgcagctggtggagtctgggggaggcgtggtgcagcctggggggtctctgagactctcctgtgcagcctctggagagatcttcagtatcaattttatgatttggtaccgccaggctccagggaagcagcgcgagtgggtcgcaggttttactagggatggaagcacaaactatccagactccgcgaagggccgattcaccatctctagagacaacgccaagaacacggtgtatctgcaaatagacagcctgaaacctgaggacacggccgtctattattgttatatgttggacacctggggccaggggacccaggtcactgtctcctcagcggccgcagaacaaaaactcatctcagaagaggatctgaatggggccgcacatcaccaccatcaccatgggagctag

SEQ ID NO: 523 - DNA, 411 bp, synthetic construct
  source 1..411: mol_type = other DNA
gaggtgcagctggtggagtctgggggaggcgtggtgcagcctggggggtctctgagactctcctgtgcagcctctggagagatcttcagtatcaattttatggaatggtaccgccaggctccagggaagcagcgcgagtgggtcgcaggttttactagggatggaagcacaaactatccagactccgcgaagggccgattcaccatctctagagacaacgccaagaacacggtgtatctgcaaatagacagcctgaaacctgaggacacggccgtctattattgttatatgttggacacctggggccaggggacccaggtcactgtctcctcagcggccgcagaacaaaaactcatctcagaagaggatctgaatggggccgcacatcaccaccatcaccatgggagctag

SEQ ID NO: 524 - DNA, 411 bp, synthetic construct
  source 1..411: mol_type = other DNA
gaggtgcagctggtggagtctgggggaggcgtggtgcagcctggggggtctctgagactctcctgtgcagcctctggagagatcttcagtatcaattttatgcgctggtaccgccaggctccagggaagcagcgcgagtgggtcgcagcgtttactagggatggaagcacaaactatccagactccgcgaagggccgattcaccatctctagagacaacgccaagaacacggtgtatctgcaaatagacagcctgaaacctgaggacacggccgtctattattgttatatgttggacacctggggccaggggacccaggtcactgtctcctcagcggccgcagaacaaaaactcatctcagaagaggatctgaatggggccgcacatcaccaccatcaccatgggagctag

SEQ ID NO: 525 - DNA, 411 bp, synthetic construct
  source 1..411: mol_type = other DNA
gaggtgcagctggtggagtctgggggaggcgtggtgcagcctggggggtctctgagactctcctgtgcagcctctggagagatcttcagtatcaattttatgcgctggtaccgccaggctccagggaagcagcgcgagtgggtcgcaaaatttactagggatggaagcacaaactatccagactccgcgaagggccgattcaccatctctagagacaacgccaagaacacggtgtatctgcaaatagacagcctgaaacctgaggacacggccgtctattattgttatatgttggacacctggggccaggggacccaggtcactgtctcctcagcggccgcagaacaaaaactcatctcagaagaggatctgaatggggccgcacatcaccaccatcaccatgggagctag

SEQ ID NO: 526 - DNA, 411 bp, synthetic construct
  source 1..411: mol_type = other DNA
gaggtgcagctggtggagtctgggggaggcgtggtgcagcctggggggtctctgagactctcctgtgcagcctctggagagatcttcagtatcaattttatgcgctggtaccgccaggctccagggaagcagcgcgagtgggtcgcaggttttactagggatggaagcacagtgtatccagactccgcgaagggccgattcaccatctctagagacaacgccaagaacacggtgtatctgcaaatagacagcctgaaacctgaggacacggccgtctattattgttatatgttggacacctggggccaggggacccaggtcactgtctcctcagcggccgcagaacaaaaactcatctcagaagaggatctgaatggggccgcacatcaccaccatcaccatgggagctag

SEQ ID NO: 527 - DNA, 411 bp, synthetic construct
  source 1..411: mol_type = other DNA
gaggtgcagctggtggagtctgggggaggcgtggtgcagcctggggggtctctgagactctcctgtgcagcctctggagagatcttcagtatcaattttatgcgctggtaccgccaggctccagggaagcagcgcgagtgggtcgcaggttttactagggatggaagcacattttatccagactccgcgaagggccgattcaccatctctagagacaacgccaagaacacggtgtatctgcaaatagacagcctgaaacctgaggacacggccgtctattattgttatatgttggacacctggggccaggggacccaggtcactgtctcctcagcggccgcagaacaaaaactcatctcagaagaggatctgaatggggccgcacatcaccaccatcaccatgggagctag

SEQ ID NO: 528 - DNA, 411 bp, synthetic construct
  source 1..411: mol_type = other DNA
gaggtgcagctggtggagtctgggggaggcgtggtgcagcctggggggtctctgagactctcctgtgcagcctctggagagatcttcagtatcaattttatgcgctggtaccgccaggctccagggaagcagcgcgagtgggtcgcaggttttactagggatggaagcacaaactatccagactccgcgaagggccgattcaccatctctagagacaacgccaagaacacggtgtatctgcaaatagacagcctgaaacctgaggacacggccgtctattattgttatatggcggacacctggggccaggggacccaggtcactgtctcctcagcggccgcagaacaaaaactcatctcagaagaggatctgaatggggccgcacatcaccaccatcaccatgggagctag

SEQ ID NO: 529 - DNA, 411 bp, synthetic construct
  source 1..411: mol_type = other DNA
gaggtgcagctggtggagtctgggggaggcgtggtgcagcctggggggtctctgagactctcctgtgcagcctctggagagatcttcagtatcaattttatgcgctggtaccgccaggctccagggaagcagcgcgagtgggtcgcaggttttactagggatggaagcacaaactatccagactccgcgaagggccgattcaccatctctagagacaacgccaagaacacggtgtatctgcaaatagacagcctgaaacctgaggacacggccgtctattattgttatatgcaggacacctggggccaggggacccaggtcactgtctcctcagcggccgcagaacaaaaactcatctcagaagaggatctgaatggggccgcacatcaccaccatcaccatgggagctag

SEQ ID NO: 530 - DNA, 429 bp, synthetic construct
  source 1..429: mol_type = other DNA
gaggtgcagctggtggagtctgggggaggcttggtgcagcctgggggttctctgagactctcctgtacagcctctggaggccccatcgagcagtatcccatgggctggttccgccgggccccaggaaaggagcgtaacttggtagcaagtattagccgaagtggagatggcacatactatgcaatctcttccgtgaagggccgattcaccatctctagagacaacgccgagaacacggtatttctgcaaatgaacagcctgaaacctgacgacacggccgtttattactgtggggctggtataaacccaaccaagatctggggccaggggacccaggtcaccgtctcctcagcggccgcagaacaaaaactcatctcagaagaggatctgaatggggccgcacatcaccaccatcaccatgggagctag

SEQ ID NO: 531 - DNA, 429 bp, synthetic construct
  source 1..429: mol_type = other DNA
gaggtgcagctggtggagtctgggggaggcttggtgcagcctgggggttctctgagactctcctgtacagcctctggaggccccatcgagcagtatcccatgggctggttccgccgggccccaggaaaggagcgtgaattggtagcaagttttagccgaagtggagatggcacatactatgcaatctcttccgtgaagggccgattcaccatctctagagacaacgccgagaacacggtatttctgcaaatgaacagcctgaaacctgacgacacggccgtttattactgtggggctggtataaacccaaccaagatctggggccaggggacccaggtcaccgtctcctcagcggccgcagaacaaaaactcatctcagaagaggatctgaatggggccgcacatcaccaccatcaccatgggagctag

SEQ ID NO: 532 - DNA, 429 bp, synthetic construct
  source 1..429: mol_type = other DNA
gaggtgcagctggtggagtctgggggaggcttggtgcagcctgggggttctctgagactctcctgtacagcctctggaggccccatcgagcagtatcccatgggctggttccgccgggccccaggaaaggagcgtgaattggtagcaagttccagccgaagtggagatggcacatactatgcaatctcttccgtgaagggccgattcaccatctctagagacaacgccgagaacacggtatttctgcaaatgaacagcctgaaacctgacgacacggccgtttattactgtggggctggtataaacccaaccaagatctggggccaggggacccaggtcaccgtctcctcagcggccgcagaacaaaaactcatctcagaagaggatctgaatggggccgcacatcaccaccatcaccatgggagctag

SEQ ID NO: 533 - DNA, 429 bp, synthetic construct
  source 1..429: mol_type = other DNA
gaggtgcagctggtggagtctgggggaggcttggtgcagcctgggggttctctgagactctcctgtacagcctctggaggccccatcgagcagtatcccatgggctggttccgccgggccccaggaaaggagcgtgaaagcgtagcaagtattagccgaagtggagatggcacatactatgcaatctcttccgtgaagggccgattcaccatctctagagacaacgccgagaacacggtatttctgcaaatgaacagcctgaaacctgacgacacggccgtttattactgtggggctggtataaacccaaccaagatctggggccaggggacccaggtcaccgtctcctcagcggccgcagaacaaaaactcatctcagaagaggatctgaatggggccgcacatcaccaccatcaccatgggagctag

SEQ ID NO: 534 - DNA, 426 bp, synthetic construct
  source 1..426: mol_type = other DNA
caggtgcagctggtgcagtctgggggaggattggtgcaggctgggggctctctgacactctcctgtacagcctctggacgccccctcagtgactatcccatgggctggttccgccgggccccagaaaaggagcgtgaattggtagcgagtattagccgaactggagatggcacatactatgcagacggcatgaggggccgattcaccatctccagagacaacagcgagaacacggtgtctctgcaaatgaacaacctgaaacctgaggacacggccgtttattactgtggggctggtataaacccaaccaagtactggggccaggggacccaggtcaccgtctcctcagcggccgcagaacaaaaactcatctcagaagaggatctgaatggggccgcacatcaccaccatcaccatgggagctag

SEQ ID NO: 535 - DNA, 426 bp, synthetic construct
  source 1..426: mol_type = other DNA
gaggtgcagctggtggagtctgggggaggattggtgcaggctgggggctctctgagactctcctgtacagcctctggacgccccatcagtgactatcccatgggctggttccgccgggccccaggaaaggatcgtgaattggtagcaagtattagccgaactggagatggcacatactatgcaaactccatgaaggaacgattcaccatctccagagacaacgcccagaatacggtgtctctgcaaatttccagtctgaaacctgaggacacagccgtttattactgtggggctggaataaatccaaccaggtactggggccaggggacccaggtcactgtctcctcagcggccgcagaacaaaaactcatctcagaagaggatctgaatggggccgcacatcaccaccatcaccatgggagctag

SEQ ID NO: 536 - DNA, 426 bp, synthetic construct
  source 1..426: mol_type = other DNA
caggtgcagctggtgcagtctgggggaggtttggtgcagcctggggggtctctgagactctcctgtgcagcctctggattcaccttcagtgcctatgccatgagctgggtccgccaggctccaggaaaggggcgtgaactggtagcaagtattagccgaactggagacggcacatactatgcagacggcatgaagggccgattcaccatctccagagacaacgccgagaacacggtgtctctacaaattaacagcctgaaacctgaggacacggccatttattactgtggggctggtataaacccaaccaagtactggggccaggggacccaggtcaccgtctcctcagcggccgcagaacaaaaactcatctcagaagaggatctgaatggggccgcacatcaccaccatcaccatgggagctag

SEQ ID NO: 537 - DNA, 429 bp, synthetic construct
  source 1..429: mol_type = other DNA
gaggtgcagctggtggagtctgggggaggattggtgcaggctggggactctctgagactctcctgtacagcctctggactcccccttagcaactatcccatgggctggttccgccgggccccaggaaaggagcgtgaattgatagcaagtattagtcgtacgggagacggcacatattatgcagactcctccgtgaagggccgattcaccatctccagagacaacgccgagaacacggtgtctctgcaaatgaacagcctgaaacctgaggacacggccgtttattactgtggggctggtataaacccaaccaagtactggggccaggggacccaggtcaccgtctcctcagcggccgcagaacaaaaactcatctcagaagaggatctgaatggggccgcacatcaccaccatcaccatgggagctag

SEQ ID NO: 538 - DNA, 333 bp, synthetic construct
  source 1..333: mol_type = other DNA
gaggtgcagctggtggagtctgggggaggcgtggtgcagcctggggggtctctaaaactctcctgcgtagcctcgggacatgacttcagtatcaattttatacgctggtaccgccaggctccagggaagcagcgcgagttcgtcgcaggatttactgcgactggtaacacaaactatgcagactccatgaaggggcgattcaccatctccagagacaacaccaagaacgcggtgtatctgcaaatagacagcctgaaacctgaggacacggccgtgtattactgctatatgttggacaagtggggccaggggacccaggtcaccgtctcctca

SEQ ID NO: 539 - DNA, 333 bp, synthetic construct
  source 1..333: mol_type = other DNA
gaggtgcagctggtggagtctgggggaggcgtggtgcagcctggggggtctctaaaactctcctgcgtagcctcgggaacggacttcagtatcaattttatacgctggtaccgccaggctccagggaagcagcgcgagttcgtcgcaggatggactgcgactggtaacacaaactatgcagactccatgaaggggcgattcaccatctccagagacaacaccaagaacgcggtgtatctgcaaatagacagcctgaaacctgaggacacggccgtgtattactgctatatgttggacaagtggggccaggggacccaggtcaccgtctcctca

SEQ ID NO: 540 - DNA, 333 bp, synthetic construct
  source 1..333: mol_type = other DNA
gaggtgcagctggtggagtctgggggaggcgtggtgcagcctggggggtctctaaaactctcctgcgtagcctcgggaacggacttcagtatcaattttatacgctggtaccgccaggctccagggaagcagcgcgagttcgtcgcaggatatactgcgactggtaacacaaactatgcagactccatgaaggggcgattcaccatctccagagacaacaccaagaacgcggtgtatctgcaaatagacagcctgaaacctgaggacacggccgtgtattactgctatatgttggacaagtggggccaggggacccaggtcaccgtctcctca

SEQ ID NO: 541 - DNA, 333 bp, synthetic construct
  source 1..333: mol_type = other DNA
gaggtgcagctggtggagtctgggggaggcgtggtgcagcctggggggtctctaaaactctcctgcgtagcctcgggaacggacttcagtatcaattttatacgctggtaccgccaggctccagggaagcagcgcgagttcgtcgcaggatttactgcgactggtaacacaaactatgcagactccatgaaggggcgattcaccatctccagagacaacaccaagaacgcggtgtatctgcaaatagacagcctgaaacctgaggacacggccgtgtattactgccatatgttggacaagtggggccaggggacccaggtcaccgtctcctca

SEQ ID NO: 542 - DNA, 333 bp, synthetic construct
  source 1..333: mol_type = other DNA
gaggtgcagctggtggagtctgggggaggcgtggtgcagcctggggggtctctaaaactctcctgcgtagcctcgggaacggacttcagtatcaattttatacgctggtaccgccaggctccagggaagcagcgcgagttcgtcgcaggatttactgcgactggtaacacaaactatgcagactccatgaaggggcgattcaccatctccagagacaacaccaagaacgcggtgtatctgcaaatagacagcctgaaacctgaggacacggccgtgtattactgctggatgttggacaagtggggccaggggacccaggtcaccgtctcctca

SEQ ID NO: 543 - DNA, 333 bp, synthetic construct
  source 1..333: mol_type = other DNA
gaggtgcagctggtggagtctgggggaggcgtggtgcagcctggggggtctctaaaactctcctgcgtagcctcgggaacggacttcagtatcaattttatacgctggtaccgccaggctccagggaagcagcgcgagttcgtcgcaggatttactgcgactggtaacacaaactatgcagactccatgaaggggcgattcaccatctccagagacaacaccaagaacgcggtgtatctgcaaatagacagcctgaaacctgaggacacggccgtgtattactgctatctgttggacaagtggggccaggggacccaggtcaccgtctcctca

SEQ ID NO: 544 - DNA, 333 bp, synthetic construct
  source 1..333: mol_type = other DNA
gaggtgcagctggtggagtctgggggaggcgtggtgcagcctggggggtctctaaaactctcctgcgtagcctcgggaacggacttcagtatcaattttatacgctggtaccgccaggctccagggaagcagcgcgagttcgtcgcaggatttactgcgactggtaacacaaactatgcagactccatgaaggggcgattcaccatctccagagacaacaccaagaacgcggtgtatctgcaaatagacagcctgaaacctgaggacacggccgtgtattactgctatgttttggacaagtggggccaggggacccaggtcaccgtctcctca

SEQ ID NO: 545 - DNA, 333 bp, synthetic construct
  source 1..333: mol_type = other DNA
gaggtgcagctggtggagtctgggggaggcgtggtgcagcctggggggtctctaaaactctcctgcgtagcctcgggagcggacttcagtatcaattatatacgctggtaccgccaggctccagggaagcagcgcgagttcgtcgcaggatttactgcgactggtaacacaaactatgcagactccatgaaggggcgattcaccatctccagagacaacaccaagaacgcggtgtatctgcaaatagacagcctgaaacctgaggacacggccgtgtattactgctatatgttggacaagtggggccaggggacccaggtcaccgtctcctca

SEQ ID NO: 546 - DNA, 333 bp, synthetic construct
  source 1..333: mol_type = other DNA
gaggtgcagctggtggagtctgggggaggcgtggtgcagcctggggggtctctaaaactctcctgcgtagcctcgggagcggacttcagtatcaattttatacgctggtaccgccaggctccagggaagcagcgcgagttcgtcgcaggatttagcgcgactggtaacacaaactatgcagactccatgaaggggcgattcaccatctccagagacaacaccaagaacgcggtgtatctgcaaatagacagcctgaaacctgaggacacggccgtgtattactgctatatgttggacaagtggggccaggggacccaggtcaccgtctcctca

SEQ ID NO: 547 - DNA, 333 bp, synthetic construct
  source 1..333: mol_type = other DNA
gaggtgcagctggtggagtctgggggaggcgtggtgcagcctggggggtctctaaaactctcctgcgtagcctcgggagcggacttcagtatcaattttatacgctggtaccgccaggctccagggaagcagcgcgagttcgtcgcaggatttactgcgactggtcatacaaactatgcagactccatgaaggggcgattcaccatctccagagacaacaccaagaacgcggtgtatctgcaaatagacagcctgaaacctgaggacacggccgtgtattactgctatatgttggacaagtggggccaggggacccaggtcaccgtctcctca

SEQ ID NO: 548 - DNA, 333 bp, synthetic construct
  source 1..333: mol_type = other DNA
gaggtgcagctggtggagtctgggggaggcgtggtgcagcctggggggtctctacgtctctcctgcgcagcctcgggaacggacttcagtatcaattttatacgctgggttcgccaggctccagggaagggtctggagtgggtcgcaggatttactgcgactggtaacacaaactatgcagactccgttaaggggcgattcaccatctccagagacaacaccaagaacaccctgtatctgcaaatagacagcctgcgtcctgaggacacggccgtgtattactgctatatgttggacaagtggggccaggggacccaggtcaccgtctcctca

SEQ ID NO: 549 - DNA, 333 bp, synthetic construct
  source 1..333: mol_type = other DNA
gaggtgcagctggtggagtctgggggaggcgtggtgcagcctggggggtctctacgtctctcctgcgcagcctcgggaacggacttcagtatcaattttatacgctggtaccgccaggctccagggaagggtctggagttcgtcgcaggatttactgcgactggtaacacaaactatgcagactccgttaaggggcgattcaccatctccagagacaacgcaaagaacaccctgtatctgcaaatgaatagcctgcgtcctgaggacacggccgtgtattactgctatatgttggacaagtggggccaggggacccaggtcaccgtctcctca

SEQ ID NO: 550 - DNA, 333 bp, synthetic construct
  source 1..333: mol_type = other DNA
gaggtgcagctggtggagtctgggggaggcgtggtgcagcctggggggtctctaaaactctcctgcgcagcctcgggaacggacttcagtatcaattttatacgctgggttcgccaggctccagggaagggtctggagtgggtcgcaggatttactgcgactggtaacacaaactatgcagactccgttaaggggcgattcaccatctccagagacaacaccaagaacaccctgtatctgcaaataaatagcctgcgtcctgaggacacggccgtgtattactgctatatgttggacaagtggggccaggggacccaggtcaccgtctcctca

SEQ ID NO: 551 - DNA, 333 bp, synthetic construct
  source 1..333: mol_type = other DNA
gaggtgcagctggtggagtctgggggaggcgtggtgcagcctggggggtctctacgtctctcctgcgcagcctcgggaacggacttcagtatcaattttatacgctgggttcgccaggctccagggaagggtctggagtgggtcgcaggatttactgcgactggtaacacaaactatgcagactccatgaaggggcgattcaccatctccagagacaacaccaagaacaccctgtatctgcaaatgaatagcctgcgtcctgaggacacggccgtgtattactgctatatgttggacaagtggggccaggggacccaggtcaccgtctcctca

SEQ ID NO: 552 - DNA, 333 bp, synthetic construct
  source 1..333: mol_type = other DNA
gaggtgcagctggtggagtctgggggaggcgtggtgcagcctggggggtctctacgtctctcctgcgcagcctcgggaacggacttcagtatcaattttatacgctggtaccgccaggctccagggaagggtctggagttcgtcgcaggatttactgcgactggtaacacaaactatgcagactccgttaaggggcgattcaccatctccagagacaacgcaaagaacaccctgtatctgcaaatagacagcctgcgtcctgaggacacggccgtgtattactgctatatgttggacaagtggggccaggggacccaggtcaccgtctcctca

SEQ ID NO: 553 - DNA, 333 bp, synthetic construct
  source 1..333: mol_type = other DNA
gaggtgcagctggtggagtctgggggaggcgtggtgcagcctggggggtctctacgtctctcctgcgcagcctcgggaacggacttcagtatcaattttatacgctggtaccgccaggctccagggaagggtctggagttcgtcgcaggatttactgcgactggtaacacaaactatgcagactccgttaaggggcgattcaccatctccagagacaacaccaagaacaccctgtatctgcaaatgaatagcctgcgtcctgaggacacggccgtgtattactgctatatgttggacaagtggggccaggggacccaggtcaccgtctcctca

SEQ ID NO: 554 - DNA, 333 bp, synthetic construct
  source 1..333: mol_type = other DNA
gaggtgcagctggtggagtctgggggaggcgtggtgcagcctggggggtctctacgtctctcctgcgcagcctcgggaacggacttcagtatcaattttatacgctgggttcgccaggctccagggaagggtctggagtgggtcgcaggatttactgcgactggtaacacaaactatgcagactccgttaaggggcgattcaccatctccagagacaacaccaagaacgcgctgtatctgcaaatgaatagcctgcgtcctgaggacacggccgtgtattactgctatatgttggacaagtggggccaggggacccaggtcaccgtctcctca

SEQ ID NO: 555 - DNA, 333 bp, synthetic construct
  source 1..333: mol_type = other DNA
gaggtgcagctggtggagtctgggggaggcgtggtgcagcctggggggtctctacgtctctcctgcgtagcctcgggaacggacttcagtatcaattttatacgctgggttcgccaggctccagggaagggtctggagtgggtcgcaggatttactgcgactggtaacacaaactatgcagactccgttaaggggcgattcaccatctccagagacaacaccaagaacaccctgtatctgcaaatggacagcctgcgtcctgaggacacggccgtgtattactgctatatgttggacaagtggggccaggggacccaggtcaccgtctcctca

SEQ ID NO: 556 - DNA, 333 bp, synthetic construct
  source 1..333: mol_type = other DNA
gaggtgcagctggtggagtctgggggaggcctggtgcagcctggggggtctctacgtctctcctgcgcagcctcgggaacggacttcagtatcaattttatacgctggtaccgccaggctccagggaagggtctggagttcgtcgcaggatttactgcgactggtaacacaaactatgcagactccgttaaggggcgattcaccatctccagagacaacagcaagaacaccctgtatctgcaaatgaatagcctgcgtgcagaggacacggccgtgtattactgctatatgttggacaagtggggccaggggaccctggtcaccgtctcctca

SEQ ID NO: 557 - DNA, 333 bp, synthetic construct
  source 1..333: mol_type = other DNA
gaggtgcagctggtggagtctgggggaggcgtggtgcagcctggggggtctctaaaactctcctgcgtagcctcgggaacggacttcagtatcaattttatacgctgggttcgccaggctccagggaagggtctggagttcgtcgcaggatttactgcgactggtaacacaaactatgcagactccatgaaggggcgattcaccatctccagagacaacaccaagaacgcgctgtatctgcaaatagacagcctgcgtcctgaggacacggccgtgtattactgctatatgttggacaagtggggccaggggacccaggtcaccgtctcctca

SEQ ID NO: 558 - DNA, 333 bp, synthetic construct
  source 1..333: mol_type = other DNA
gaggtgcagctggtggagtctgggggaggcgtggtgcagcctggggggtctctaaaactctcctgcgtagcctcgggaacggacttcagtatcaattttatacgctggtaccgccaggctccagggaagggtctggagttcgtcgcaggatttactgcgactggtaacacaaactatgcagactccgttaaggggcgattcaccatctccagagacaacgcaaagaacaccctgtatctgcaaatgaatagcctgcgtcctgaggacacggccgtgtattactgctatatgttggacaagtggggccaggggacccaggtcaccgtctcctca

SEQ ID NO: 559 - DNA, 333 bp, synthetic construct
  source 1..333: mol_type = other DNA
gaggtgcagctggtggagtctgggggaggcgtggtgcagcctggggggtctctacgtctctcctgcgcagcctcgggaacggacttcagtatcaattttatacgctggtaccgccaggctccagggaagcagcgcgagttcgtcgcaggatttactgcgactggtaacacaaactatgcagactccgttaaggggcgattcaccatctccagagacaacgcaaagaacaccctgtatctgcaaatgaatagcctgcgtcctgaggacacggccgtgtattactgctatatgttggacaagtggggccaggggacccaggtcaccgtctcctca

SEQ ID NO: 560 - DNA, 333 bp, synthetic construct
  source 1..333: mol_type = other DNA
gaggtgcagctggtggagtctgggggaggcgtggtgcagcctggggggtctctacgtctctcctgcgcagcctcgggaacggacttcagtatcaattttatacgctggtaccgccaggctccagggaagggtctggagttcgtcgcaggatttactgcgactggtaacacaaactatgcagactccgttaaggggcgattcaccatctccagagacaacgcaaagaacgcggtgtatctgcaaatgaatagcctgcgtcctgaggacacggccgtgtattactgctatatgttggacaagtggggccaggggacccaggtcaccgtctcctca

SEQ ID NO: 561 - DNA, 333 bp, synthetic construct
  source 1..333: mol_type = other DNA
gaggtgcagctggtggagtctgggggaggcgtggtgcagcctggggggtctctacgtctctcctgcgcagcctcgggaacggacttcagtatcaattttatacgctggtaccgccaggctccagggaagggtctggagttcgtcgcaggatttactgcgactggtaacacaaactatgcagactccgttaaggggcgattcaccatctccagagacaacgcaaagaacaccctgtatctgcaaatgaatagcctgaaacctgaggacacggccgtgtattactgctatatgttggacaagtggggccaggggacccaggtcaccgtctcctca

SEQ ID NO: 562 - DNA, 333 bp, synthetic construct
  source 1..333: mol_type = other DNA
gaggtgcagctggtggagtctgggggaggcgtggtgcagcctggggggtctctacgtctctcctgcgcagcctcgggaacggacttcagtatcaattttatacgctggtaccgccaggctccagggaagggtcgcgagttcgtcgcaggatttactgcgactggtaacacaaactatgcagactccgttaaggggcgattcaccatctccagagacaacgcaaagaacaccctgtatctgcaaatgaatagcctgcgtcctgaggacacggccgtgtattactgctatatgttggacaagtggggccaggggacccaggtcaccgtctcctca

SEQ ID NO: 563 - DNA, 333 bp, synthetic construct; identical to SEQ ID NO: 325
  source 1..333: mol_type = other DNA

SEQ ID NO: 564 - DNA, 333 bp, synthetic construct
  source 1..333: mol_type = other DNA
gaggtgcagctggtggagtctgggggaggcgtggtgcagcctggggggtctctacgtctctcctgcgcagcctcgggaacggacttcagtatcaattttatacgctggtaccgccaggctccagggaagggtctggagttcgtcgcaggatttactgcgactggtaacacaaactatgcagactccatgaaggggcgattcaccatctccagagacaacgcaaagaacaccctgtatctgcaaatgaatagcctgcgtcctgaggacacggccgtgtattactgctatatgttggacaagtggggccaggggacccaggtcaccgtctcctca

SEQ ID NO: 565 - DNA, 333 bp, synthetic construct
  source 1..333: mol_type = other DNA
gaggtgcagctggtggagtctgggggaggcgtggtgcagcctggggggtctctacgtctctcctgcgcagcctcgggaacggacttcagtatcaattttatacgctgggttcgccaggctccagggaagggtctggagttcgtcgcaggatttactgcgactggtaacacaaactatgcagactccgttaaggggcgattcaccatctccagagacaacgcaaagaacaccctgtatctgcaaatagacagcctgcgtcctgaggacacggccgtgtattactgctatatgttggacaagtggggccaggggacccaggtcaccgtctcctca

SEQ ID NO: 566 - DNA, 333 bp, synthetic construct
  source 1..333: mol_type = other DNA
gaggtgcagctggtggagtctgggggaggcgtggtgcagcctggggggtctctacgtctctcctgcgcagcctcgggaacggacttcagtatcaattttatacgctggtaccgccaggctccagggaagggtctggagtgggtcgcaggatttactgcgactggtaacacaaactatgcagactccgttaaggggcgattcaccatctccagagacaacgcaaagaacaccctgtatctgcaaatagacagcctgcgtcctgaggacacggccgtgtattactgctatatgttggacaagtggggccaggggacccaggtcaccgtctcctca

SEQ ID NO: 567 - DNA, 333 bp, synthetic construct
  source 1..333: mol_type = other DNA
gaggtgcagctggtggagtctgggggaggcgtggtgcagcctggggggtctctaaaactctcctgcgtagcctcgggaacggacttcagtatcaattttatacgctggtaccgccaggctccagggaagcagcgcgagttcgtcgcaggatttactgcgactggtaacacaaactatgcagactccatgaaggggcgattcaccatctccagagacaacaccaagaacgcggtgtatctgcaaatagacagcctgaaacctgaggacacggccgtgtattactgcgcgatggcggacaagtggggccaggggacccaggtcaccgtctcctca

SEQ ID NO: 568 - DNA, 333 bp, synthetic construct
  source 1..333: mol_type = other DNA
gaggtgcagctggtggagtctgggggaggcgtggtgcagcctggggggtctctgagactctcctgtgcagcctctggagagatcttcagtatcaattttatgcgctggtaccgccaggctccagggaagggtctggagtgggtcgcaggttttactagggatggaagcacaaactatccagactccgttaagggccgattcaccatctctagagacaacgccaagaacacggtgtatctgcaaatgaatagcctgcgtcctgaggacacggccgtctattattgttatatgttggacacctggggccaggggacccaggtcactgtctcctca

SEQ ID NO: 569 - DNA, 333 bp, synthetic construct
  source 1..333: mol_type = other DNA
gaggtgcagctggtggagtctgggggaggcgtggtgcagcctggggggtctctacgtctctcctgcgcagcctcgggaacggacttcagtatcaattttatacgctggtaccgccaggctccagggaagggtctggagttcgtcgcaggattttcagcgactggtaacacaaactatgcagactccgttaaggggcgattcaccatctccagagacaacgcaaagaacgcggtgtatctgcaaatgaatagcctgcgtcctgaggacacggccgtgtattactgctatatgttggacaagtggggccaggggacccaggtcaccgtctcctca

SEQ ID NO: 570 - DNA, 333 bp, synthetic construct
  source 1..333: mol_type = other DNA
gaggtgcagctggtggagtctgggggaggcgtggtgcagcctggggggtctctacgtctctcctgcgcagcctcgggaacggacttcagtatcaattttatacgctggtaccgccaggctccagggaagggtctggagttcgtcgcaggatttactgcgactggtaacacaaactatgcagactccgttaaggggcgattcaccatctccagagacaacgcaaagaacgcggtgtatctgcaaatgaatagcctgcgtcctgaggacacggccgtgtattactgctatattttggacaagtggggccaggggacccaggtcaccgtctcctca

SEQ ID NO: 571 - DNA, 333 bp, synthetic construct
  source 1..333: mol_type = other DNA
gaggtgcagctggtggagtctgggggaggcgtggtgcagcctggggggtctctgagactctcctgtgcagccgatggagagatcttcagtatcaattttatgcgctggtaccgccaggctccagggaagcagcgcgagtgggtcgcaggttttactagggatggaagcacaaactatccagactccgcgaagggccgattcaccatctctagagacaacgccaagaacacggtgtatctgcaaatagacagcctgaaacctgaggacacggccgtctattattgttatatgttggacacctggggccaggggacccaggtcactgtctcctca

SEQ ID NO: 572 - DNA, 333 bp, synthetic construct
  source 1..333: mol_type = other DNA
gaggtgcagctggtggagtctgggggaggcgtggtgcagcctggggggtctctgagactctcctgtgcagcctctggagagatcttcagtatcaattttatgcgctggtacggccaggctccagggaagcagcgcgagtgggtcgcaggttttactagggatggaagcacaaactatccagactccgcgaagggccgattcaccatctctagagacaacgccaagaacacggtgtatctgcaaatagacagcctgaaacctgaggacacggccgtctattattgttatatgttggacacctggggccaggggacccaggtcactgtctcctca

SEQ ID NO: 573 - DNA, 333 bp, synthetic construct
  source 1..333: mol_type = other DNA
gaggtgcagctggtggagtctgggggaggcgtggtgcagcctggggggtctctgagactctcctgtgcagcctctggagagatcttcagtatcaattttatgcgctggtaccgcgaagctccagggaagcagcgcgagtgggtcgcaggttttactagggatggaagcacaaactatccagactccgcgaagggccgattcaccatctctagagacaacgccaagaacacggtgtatctgcaaatagacagcctgaaacctgaggacacggccgtctattattgttatatgttggacacctggggccaggggacccaggtcactgtctcctca

SEQ ID NO: 574 - DNA, 333 bp, synthetic construct
  source 1..333: mol_type = other DNA
gaggtgcagctggtggagtctgggggaggcgtggtgcagcctggggggtctctgagactctcctgtgcagcctctggagagatcttcagtatcaattttatgcgctggtaccgccaggctccaattaagcagcgcgagtgggtcgcaggttttactagggatggaagcacaaactatccagactccgcgaagggccgattcaccatctctagagacaacgccaagaacacggtgtatctgcaaatagacagcctgaaacctgaggacacggccgtctattattgttatatgttggacacctggggccaggggacccaggtcactgtctcctca

SEQ ID NO: 575 - DNA, 333 bp, synthetic construct
  source 1..333: mol_type = other DNA
gaggtgcagctggtggagtctgggggaggcgtggtgcagcctggggggtctctgagactctcctgtgcagcctctggagagatcttcagtatcaattttatgcgctggtaccgccaggctccagggaagattcgcgagtgggtcgcaggttttactagggatggaagcacaaactatccagactccgcgaagggccgattcaccatctctagagacaacgccaagaacacggtgtatctgcaaatagacagcctgaaacctgaggacacggccgtctattattgttatatgttggacacctggggccaggggacccaggtcactgtctcctca

SEQ ID NO: 576 - DNA, 333 bp, synthetic construct
  source 1..333: mol_type = other DNA
gaggtgcagctggtggagtctgggggaggcgtggtgcagcctggggggtctctgagactctcctgtgcagcctctggagagatcttcagtatcaattttatgcgctggtaccgccaggctccagggaagcagcgcgagtgggtcgcaggttttactagggatggatttacaaactatccagactccgcgaagggccgattcaccatctctagagacaacgccaagaacacggtgtatctgcaaatagacagcctgaaacctgaggacacggccgtctattattgttatatgttggacacctggggccaggggacccaggtcactgtctcctca

SEQ ID NO: 577 - DNA, 333 bp, synthetic construct
  source 1..333: mol_type = other DNA
gaggtgcagctggtggagtctgggggaggcgtggtgcagcctggggggtctctgagactctcctgtgcagcctctggagagatcttcagtatcaattttatgcgctggtaccgccaggctccagggaagcagcgcgagtgggtcgcaggttttactagggatggatatacaaactatccagactccgcgaagggccgattcaccatctctagagacaacgccaagaacacggtgtatctgcaaatagacagcctgaaacctgaggacacggccgtctattattgttatatgttggacacctggggccaggggacccaggtcactgtctcctca

SEQ ID NO: 578 - DNA, 333 bp, synthetic construct
  source 1..333: mol_type = other DNA
gaggtgcagctggtggagtctgggggaggcgtggtgcagcctggggggtctctgagactctcctgtgcagcctctggagagatcttcagtatcaattttatgcgctggtaccgccaggctccagggaagcagcgcgagtgggtcgcaggttttactagggatggaagcctgaactatccagactccgcgaagggccgattcaccatctctagagacaacgccaagaacacggtgtatctgcaaatagacagcctgaaacctgaggacacggccgtctattattgttatatgttggacacctggggccaggggacccaggtcactgtctcctca

SEQ ID NO: 579 - DNA, 333 bp, synthetic construct
  source 1..333: mol_type = other DNA
gaggtgcagctggtggagtctgggggaggcgtggtgcagcctggggggtctctgagactctcctgtgcagcctctggagagatcttcagtatcaattttatgcgctggtaccgccaggctccagggaagcagcgcgagtgggtcgcaggttttactagggatggaagcaaaaactatccagactccgcgaagggccgattcaccatctctagagacaacgccaagaacacggtgtatctgcaaatagacagcctgaaacctgaggacacggccgtctattattgttatatgttggacacctggggccaggggacccaggtcactgtctcctca

SEQ ID NO: 580 - DNA, 333 bp, synthetic construct
  source 1..333: mol_type = other DNA
gaggtgcagctggtggagtctgggggaggcgtggtgcagcctggggggtctctgagactctcctgtgcagcctctgatgagatcttcagtatcaattttatgcgctggtaccgccaggctccagggaagcagcgcgagtgggtcgcaggttttactagggatggaagcacaaactatccagactccgcgaagggccgattcaccatctctagagacaacgccaagaacacggtgtatctgcaaatagacagcctgaaacctgaggacacggccgtctattattgttatatgttggacacctggggccaggggacccaggtcactgtctcctca

SEQ ID NO: 581 - DNA, 333 bp, synthetic construct
  source 1..333: mol_type = other DNA
gaggtgcagctggtggagtctgggggaggcgtggtgcagcctggggggtctctgagactctcctgtgcagcctctggagagatcttctatatcaattttatgcgctggtaccgccaggctccagggaagcagcgcgagtgggtcgcaggttttactagggatggaagcacaaactatccagactccgcgaagggccgattcaccatctctagagacaacgccaagaacacggtgtatctgcaaatagacagcctgaaacctgaggacacggccgtctattattgttatatgttggacacctggggccaggggacccaggtcactgtctcctca

SEQ ID NO: 582 - DNA, 333 bp, synthetic construct
  source 1..333: mol_type = other DNA
gaggtgcagctggtggagtctgggggaggcgtggtgcagcctggggggtctctgagactctcctgtgcagcctctggagagatcttcagtatcaattttatgcgctggtaccgccaggctccagggaagcagcgcgagtgggtcgcaggttttactaggctgggaagcacaaactatccagactccgcgaagggccgattcaccatctctagagacaacgccaagaacacggtgtatctgcaaatagacagcctgaaacctgaggacacggccgtctattattgttatatgttggacacctggggccaggggacccaggtcactgtctcctca

SEQ ID NO: 583 - DNA, 333 bp, synthetic construct
  source 1..333: mol_type = other DNA
gaggtgcagctggtggagtctgggggaggcgtggtgcagcctggggggtctctgagactctcctgtgcagcctctggagagatcttcagtatcaattttatgcgctggtaccgccaggctccagggaagcagcgcgagtgggtcgcaggttttactagggatgatagcacaaactatccagactccgcgaagggccgattcaccatctctagagacaacgccaagaacacggtgtatctgcaaatagacagcctgaaacctgaggacacggccgtctattattgttatatgttggacacctggggccaggggacccaggtcactgtctcctca

SEQ ID NO: 584 - DNA, 333 bp, synthetic construct
  source 1..333: mol_type = other DNA
gaggtgcagctggtggagtctgggggaggcgtggtgcagcctggggggtctctgagactctcctgtgcagcctctggagagatcttcagtatcaattttatgcgctggtaccgccaggctccagggaagcagcgcgagcaggtcgcaggttttactagggatggaagcacaaactatccagactccgcgaagggccgattcaccatctctagagacaacgccaagaacacggtgtatctgcaaatagacagcctgaaacctgaggacacggccgtctattattgttatatgttggacacctggggccaggggacccaggtcactgtctcctca

SEQ ID NO: 585 - DNA, 333 bp, synthetic construct
  source 1..333: mol_type = other DNA
gaggtgcagctggtggagtctgggggaggcgtggtgcagcctggggggtctctgagactctcctgtgcagcctctggagagatcttcagtatcaattttatgcgctggtaccgccaggctccagggaagcagcgcgagtttgtcgcaggttttactagggatggaagcacaaactatccagactccgcgaagggccgattcaccatctctagagacaacgccaagaacacggtgtatctgcaaatagacagcctgaaacctgaggacacggccgtctattattgttatatgttggacacctggggccaggggacccaggtcactgtctcctca

SEQ ID NO: 586 - DNA, 333 bp, synthetic construct
  source 1..333: mol_type = other DNA
gaggtgcagctggtggagtctgggggaggcgtggtgcagcctggggggtctctgagactctcctgtgcagcctctggagagatccatagtatcaattttatgcgctggtaccgccaggctccagggaagcagcgcgagtgggtcgcaggttttactagggatggaagcacaaactatccagactccgcgaagggccgattcaccatctctagagacaacgccaagaacacggtgtatctgcaaatagacagcctgaaacctgaggacacggccgtctattattgttatatgttggacacctggggccaggggacccaggtcactgtctcctca

SEQ ID NO: 587 - DNA, 333 bp, synthetic construct
  source 1..333: mol_type = other DNA
gaggtgcagctggtggagtctgggggaggcgtggtgcagcctggggggtctctgagactctcctgtgcagcctctggagagatcttcagtatcaattttatgcgctggtaccgccaggctccagggaagcagcgccattgggtcgcaggttttactagggatggaagcacaaactatccagactccgcgaagggccgattcaccatctctagagacaacgccaagaacacggtgtatctgcaaatagacagcctgaaacctgaggacacggccgtctattattgttatatgttggacacctggggccaggggacccaggtcactgtctcctca

SEQ ID NO: 588 - DNA, 333 bp, synthetic construct
  source 1..333: mol_type = other DNA
gaggtgcagctggtggagtctgggggaggcgtggtgcagcctggggggtctctgagactctcctgtgcagcctctggagagatcttcagtatcaattttatgcgctggtaccgccaggctccagggaagcagcgcgagtgggtcgcaggttttactagggatggaagccataactatccagactccgcgaagggccgattcaccatctctagagacaacgccaagaacacggtgtatctgcaaatagacagcctgaaacctgaggacacggccgtctattattgttatatgttggacacctggggccaggggacccaggtcactgtctcctca

SEQ ID NO: 589 - DNA, 333 bp, synthetic construct
  source 1..333: mol_type = other DNA
gaggtgcagctggtggagtctgggggaggcgtggtgcagcctggggggtctctgagactctcctgtgcagcctctggagagatcttcagtatcaataacatgcgctggtaccgccaggctccagggaagcagcgcgagtgggtcgcaggttttactagggatggaagcacaaactatccagactccgcgaagggccgattcaccatctctagagacaacgccaagaacacggtgtatctgcaaatagacagcctgaaacctgaggacacggccgtctattattgttatatgttggacacctggggccaggggacccaggtcactgtctcctca

SEQ ID NO: 590 - DNA, 333 bp, synthetic construct
  source 1..333: mol_type = other DNA
gaggtgcagctggtggagtctgggggaggcgtggtgcagcctggggggtctctgagactctcctgtgcagcctctggagagatcttcagtatcaatcagatgcgctggtaccgccaggctccagggaagcagcgcgagtgggtcgcaggttttactagggatggaagcacaaactatccagactccgcgaagggccgattcaccatctctagagacaacgccaagaacacggtgtatctgcaaatagacagcctgaaacctgaggacacggccgtctattattgttatatgttggacacctggggccaggggacccaggtcactgtctcctca

SEQ ID NO: 591 - DNA, 333 bp, synthetic construct
  source 1..333: mol_type = other DNA
gaggtgcagctggtggagtctgggggaggcgtggtgcagcctggggggtctctgagactctcctgtgcagcctctggagagatcttcagtatcaattttatgatttggtaccgccaggctccagggaagcagcgcgagtgggtcgcaggttttactagggatggaagcacaaactatccagactccgcgaagggccgattcaccatctctagagacaacgccaagaacacggtgtatctgcaaatagacagcctgaaacctgaggacacggccgtctattattgttatatgttggacacctggggccaggggacccaggtcactgtctcctca

SEQ ID NO: 592 - DNA, 333 bp, synthetic construct
  source 1..333: mol_type = other DNA
gaggtgcagctggtggagtctgggggaggcgtggtgcagcctggggggtctctgagactctcctgtgcagcctctggagagatcttcagtatcaattttatggaatggtaccgccaggctccagggaagcagcgcgagtgggtcgcaggttttactagggatggaagcacaaactatccagactccgcgaagggccgattcaccatctctagagacaacgccaagaacacggtgtatctgcaaatagacagcctgaaacctgaggacacggccgtctattattgttatatgttggacacctggggccaggggacccaggtcactgtctcctca

SEQ ID NO: 593 - DNA, 333 bp, synthetic construct
  source 1..333: mol_type = other DNA
gaggtgcagctggtggagtctgggggaggcgtggtgcagcctggggggtctctgagactctcctgtgcagcctctggagagatcttcagtatcaattttatgcgctggtaccgccaggctccagggaagcagcgcgagtgggtcgcagcgtttactagggatggaagcacaaactatccagactccgcgaagggccgattcaccatctctagagacaacgccaagaacacggtgtatctgcaaatagacagcctgaaacctgaggacacggccgtctattattgttatatgttggacacctggggccaggggacccaggtcactgtctcctca

SEQ ID NO: 594 - DNA, 333 bp, synthetic construct
  source 1..333: mol_type = other DNA
gaggtgcagctggtggagtctgggggaggcgtggtgcagcctggggggtctctgagactctcctgtgcagcctctggagagatcttcagtatcaattttatgcgctggtaccgccaggctccagggaagcagcgcgagtgggtcgcaaaatttactagggatggaagcacaaactatccagactccgcgaagggccgattcaccatctctagagacaacgccaagaacacggtgtatctgcaaatagacagcctgaaacctgaggacacggccgtctattattgttatatgttggacacctggggccaggggacccaggtcactgtctcctca

SEQ ID NO: 595 - DNA, 333 bp, synthetic construct
  source 1..333: mol_type = other DNA
gaggtgcagctggtggagtctgggggaggcgtggtgcagcctggggggtctctgagactctcctgtgcagcctctggagagatcttcagtatcaattttatgcgctggtaccgccaggctccagggaagcagcgcgagtgggtcgcaggttttactagggatggaagcacagtgtatccagactccgcgaagggccgattcaccatctctagagacaacgccaagaacacggtgtatctgcaaatagacagcctgaaacctgaggacacggccgtctattattgttatatgttggacacctggggccaggggacccaggtcactgtctcctca

SEQ ID NO: 596 - DNA, 333 bp, synthetic construct
  source 1..333: mol_type = other DNA
gaggtgcagctggtggagtctgggggaggcgtggtgcagcctggggggtctctgagactctcctgtgcagcctctggagagatcttcagtatcaattttatgcgctggtaccgccaggctccagggaagcagcgcgagtgggtcgcaggttttactagggatggaagcacattttatccagactccgcgaagggccgattcaccatctctagagacaacgccaagaacacggtgtatctgcaaatagacagcctgaaacctgaggacacggccgtctattattgttatatgttggacacctggggccaggggacccaggtcactgtctcctca

SEQ ID NO: 597 - DNA, 333 bp, synthetic construct
  source 1..333: mol_type = other DNA
gaggtgcagctggtggagtctgggggaggcgtggtgcagcctggggggtctctgagactctcctgtgcagcctctggagagatcttcagtatcaattttatgcgctggtaccgccaggctccagggaagcagcgcgagtgggtcgcaggttttactagggatggaagcacaaactatccagactccgcgaagggccgattcaccatctctagagacaacgccaagaacacggtgtatctgcaaatagacagcctgaaacctgaggacacggccgtctattattgttatatggcggacacctggggccaggggacccaggtcactgtctcctca

SEQ ID NO: 598 - DNA, 333 bp, synthetic construct
  source 1..333: mol_type = other DNA
gaggtgcagctggtggagtctgggggaggcgtggtgcagcctggggggtctctgagactctcctgtgcagcctctggagagatcttcagtatcaattttatgcgctggtaccgccaggctccagggaagcagcgcgagtgggtcgcaggttttactagggatggaagcacaaactatccagactccgcgaagggccgattcaccatctctagagacaacgccaagaacacggtgtatctgcaaatagacagcctgaaacctgaggacacggccgtctattattgttatatgcaggacacctggggccaggggacccaggtcactgtctcctca

SEQ ID NO: 599 - DNA, 351 bp, synthetic construct
  source 1..351: mol_type = other DNA
gaggtgcagctggtggagtctgggggaggcttggtgcagcctgggggttctctgagactctcctgtacagcctctggaggccccatcgagcagtatcccatgggctggttccgccgggccccaggaaaggagcgtaacttggtagcaagtattagccgaagtggagatggcacatactatgcaatctcttccgtgaagggccgattcaccatctctagagacaacgccgagaacacggtatttctgcaaatgaacagcctgaaacctgacgacacggccgtttattactgtggggctggtataaacccaaccaagatctggggccaggggacccaggtcaccgtctcctca

SEQ ID NO: 600 - DNA, 351 bp, synthetic construct
  source 1..351: mol_type = other DNA
gaggtgcagctggtggagtctgggggaggcttggtgcagcctgggggttctctgagactctcctgtacagcctctggaggccccatcgagcagtatcccatgggctggttccgccgggccccaggaaaggagcgtgaattggtagcaagttttagccgaagtggagatggcacatactatgcaatctcttccgtgaagggccgattcaccatctctagagacaacgccgagaacacggtatttctgcaaatgaacagcctgaaacctgacgacacggccgtttattactgtggggctggtataaacccaaccaagatctggggccaggggacccaggtcaccgtctcctca

SEQ ID NO: 601 - DNA, 351 bp, synthetic construct
  source 1..351: mol_type = other DNA
gaggtgcagctggtggagtctgggggaggcttggtgcagcctgggggttctctgagactctcctgtacagcctctggaggccccatcgagcagtatcccatgggctggttccgccgggccccaggaaaggagcgtgaattggtagcaagttccagccgaagtggagatggcacatactatgcaatctcttccgtgaagggccgattcaccatctctagagacaacgccgagaacacggtatttctgcaaatgaacagcctgaaacctgacgacacggccgtttattactgtggggctggtataaacccaaccaagatctggggccaggggacccaggtcaccgtctcctca

SEQ ID NO: 602 - DNA, 351 bp, synthetic construct
  source 1..351: mol_type = other DNA
gaggtgcagctggtggagtctgggggaggcttggtgcagcctgggggttctctgagactctcctgtacagcctctggaggccccatcgagcagtatcccatgggctggttccgccgggccccaggaaaggagcgtgaaagcgtagcaagtattagccgaagtggagatggcacatactatgcaatctcttccgtgaagggccgattcaccatctctagagacaacgccgagaacacggtatttctgcaaatgaacagcctgaaacctgacgacacggccgtttattactgtggggctggtataaacccaaccaagatctggggccaggggacccaggtcaccgtctcctca

SEQ ID NO: 603 - DNA, 348 bp, synthetic construct
  source 1..348: mol_type = other DNA
caggtgcagctggtgcagtctgggggaggattggtgcaggctgggggctctctgacactctcctgtacagcctctggacgccccctcagtgactatcccatgggctggttccgccgggccccagaaaaggagcgtgaattggtagcgagtattagccgaactggagatggcacatactatgcagacggcatgaggggccgattcaccatctccagagacaacagcgagaacacggtgtctctgcaaatgaacaacctgaaacctgaggacacggccgtttattactgtggggctggtataaacccaaccaagtactggggccaggggacccaggtcaccgtctcctca

SEQ ID NO: 604 - DNA, 348 bp, synthetic construct
  source 1..348: mol_type = other DNA
gaggtgcagctggtggagtctgggggaggattggtgcaggctgggggctctctgagactctcctgtacagcctctggacgccccatcagtgactatcccatgggctggttccgccgggccccaggaaaggatcgtgaattggtagcaagtattagccgaactggagatggcacatactatgcaaactccatgaaggaacgattcaccatctccagagacaacgcccagaatacggtgtctctgcaaatttccagtctgaaacctgaggacacagccgtttattactgtggggctggaataaatccaaccaggtactggggccaggggacccaggtcactgtctcctca

SEQ ID NO: 605 - DNA, 348 bp, synthetic construct
  source 1..348: mol_type = other DNA
caggtgcagctggtgcagtctgggggaggtttggtgcagcctggggggtctctgagactctcctgtgcagcctctggattcaccttcagtgcctatgccatgagctgggtccgccaggctccaggaaaggggcgtgaactggtagcaagtattagccgaactggagacggcacatactatgcagacggcatgaagggccgattcaccatctccagagacaacgccgagaacacggtgtctctacaaattaacagcctgaaacctgaggacacggccatttattactgtggggctggtataaacccaaccaagtactggggccaggggacccaggtcaccgtctcctca

SEQ ID NO: 606 - DNA, 351 bp, synthetic construct
  source 1..351: mol_type = other DNA
gaggtgcagctggtggagtctgggggaggattggtgcaggctggggactctctgagactctcctgtacagcctctggactcccccttagcaactatcccatgggctggttccgccgggccccaggaaaggagcgtgaattgatagcaagtattagtcgtacgggagacggcacatattatgcagactcctccgtgaagggccgattcaccatctccagagacaacgccgagaacacggtgtctctgcaaatgaacagcctgaaacctgaggacacggccgtttattactgtggggctggtataaacccaaccaagtactggggccaggggacccaggtcaccgtctcctca

SEQ ID NO: 607 - protein, 8 aa, synthetic construct
GFASHLYA

SEQ ID NO: 608 - protein, 8 aa, synthetic construct
ISSNDGST

SEQ ID NO: 609 - protein, 15 aa, synthetic construct
ATDLTVHCFMAEYDW

SEQ ID NO: 610 - protein, 8 aa, synthetic construct
GLAFSTHT

SEQ ID NO: 611 - protein, 8 aa, synthetic construct
IRWSDEDT

SEQ ID NO: 612 - protein, 14 aa, synthetic construct
AAARGVGTSGHMKY

SEQ ID NO: 613 - protein, 122 aa, synthetic construct
EVQLVESGGGLVQAGDSLRLSCAASGFASHLYAIGWFRQAPGKEREKVSCISSNDGSTYYADSVKGRFTISRDTVKDMVYLQMNSLKPEDTAVYYCATDLTVHCFMAEYDWWGQGTQVTVSS

SEQ ID NO: 614 - protein, 122 aa, synthetic construct
EVQLVESGGGLVQPGGSLRLSCAASGFASHLYAIGWFRQAPGKEREKVSCISSNDGSTYYADSVKGRFTISRDTVKDMVYLQMNSLKPEDTAVYYCATDLTVHCFMAEYDWWGQGTQVTVSS

SEQ ID NO: 615 - protein, 121 aa, synthetic construct
EVQLVESGGRLVQAGGSLRLSCTASGLAFSTHTMHWFRQAPGKEREFVGAIRWSDEDTEYADSVKGRFTISRDNAKSTVYLQMNNLKPEDTAVYYCAAARGVGTSGHMKYWGQGTQVTVSS

SEQ ID NO: 616 - protein, 147 aa, synthetic construct
EVQLVESGGGLVQAGDSLRLSCAASGFASHLYAIGWFRQAPGKEREKVSCISSNDGSTYYADSVKGRFTISRDTVKDMVYLQMNSLKPEDTAVYYCATDLTVHCFMAEYDWWGQGTQVTVSSAAAEQKLISEEDLNGAAHHHHHHGS

SEQ ID NO: 617 - protein, 147 aa, synthetic construct
EVQLVESGGGLVQPGGSLRLSCAASGFASHLYAIGWFRQAPGKEREKVSCISSNDGSTYYADSVKGRFTISRDTVKDMVYLQMNSLKPEDTAVYYCATDLTVHCFMAEYDWWGQGTQVTVSSAAAEQKLISEEDLNGAAHHHHHHGS

SEQ ID NO: 618 - protein, 146 aa, synthetic construct
EVQLVESGGRLVQAGGSLRLSCTASGLAFSTHTMHWFRQAPGKEREFVGAIRWSDEDTEYADSVKGRFTISRDNAKSTVYLQMNNLKPEDTAVYYCAAARGVGTSGHMKYWGQGTQVTVSSAAAEQKLISEEDLNGAAHHHHHHGS

SEQ ID NO: 619 - protein, 25 aa, synthetic construct
EVQLVESGGGLVQAGDSLRLSCAAS

SEQ ID NO: 620 - protein, 25 aa, synthetic construct
EVQLVESGGRLVQAGGSLRLSCTAS

SEQ ID NO: 621 - protein, 17 aa, synthetic construct
IGWFRQAPGKEREKVSC

SEQ ID NO: 622 - protein, 17 aa, synthetic construct
MHWFRQAPGKEREFVGA

SEQ ID NO: 623 - protein, 38 aa, synthetic construct
YYADSVKGRFTISRDTVKDMVYLQMNSLKPEDTAVYYC

SEQ ID NO: 624 - protein, 38 aa, synthetic construct
EYADSVKGRFTISRDNAKSTVYLQMNNLKPEDTAVYYC

SEQ ID NO: 625 - protein, 38 aa, synthetic construct
VYPDSAKGRFTISRDNAKNTVYLQIDSLKPEDTAVYYC

SEQ ID NO: 626 - protein, 38 aa, synthetic construct
FYPDSAKGRFTISRDNAKNTVYLQIDSLKPEDTAVYYC

SEQ ID NO: 627 - protein, 4 aa, synthetic construct
GSGS

SEQ ID NO: 628 - protein, 8 aa, synthetic construct
SGSGGGGG

SEQ ID NO: 629 - protein, 5 aa, synthetic construct
GGGGS

SEQ ID NO: 630 - protein, 10 aa, synthetic construct
GGGGSGGGGS

SEQ ID NO: 631 - protein, 15 aa, synthetic construct
GGGGSGGGGSGGGGS

SEQ ID NO: 632 - protein, 20 aa, synthetic construct
GGGGSGGGGSGGGGSGGGGS

SEQ ID NO: 633 - protein, 25 aa, synthetic construct
GGGGSGGGGSGGGGSGGGGSGGGGS

SEQ ID NO: 634 - protein, 30 aa, synthetic construct
GGGGSGGGGSGGGGSGGGGSGGGGSGGGGS

SEQ ID NO: 635 - protein, 17 aa, synthetic construct
GGGGGGSGGGGSGGGGS

SEQ ID NO: 636 - protein, 5 aa, synthetic construct
EAAAK

SEQ ID NO: 637 - protein, 12 aa, synthetic construct
AEAAAKEAAAKA

SEQ ID NO: 638 - protein, 17 aa, synthetic construct
AEAAAKEAAAKEAAAKA

SEQ ID NO: 639 - protein, 14 aa, synthetic construct
GGEAAAKEAAAKEA

SEQ ID NO: 640 - protein, 24 aa, synthetic construct
GGEAAAKEAAAKEAAAKEAAAKEA

SEQ ID NO: 641 - protein, 48 aa, synthetic construct
GGAEAAAKEAAAKEAAAKEAAAKALEAEAAAKEAAAKEAAAKEAAAKA

SEQ ID NO: 642 - protein, 36 aa, synthetic construct
GGAPAPAPAPAPAPAPAPAPAPAPAPAPAPAPAPAP

SEQ ID NO: 643 - protein, 13 aa, synthetic construct
ASTKGPSVFPLAP

SEQ ID NO: 644 - protein, 12 aa, synthetic construct
GSAGSAAGSGEF

SEQ ID NO: 645 - protein, 18 aa, synthetic construct
KESGSVSSEQLAQFRSLD

SEQ ID NO: 646 - DNA, 333 bp, synthetic construct
  source 1..333: mol_type = other DNA
caggtgcagctggtgcagtctgggggaggcttggtgcaggctggggggtctctgagactctcctgtgcagcctctggaagtatcttcagtgacattaccctggcctggcaccgccagattccagggaaagagcgcgagtgggtcgcaggtatcagtcgcagtggaagccccagctatcgggactccgtgaagggccgattcaccatctctcgagacaacgccaagaacacggtattcctacaaatgaacagtctggaacccgaggacacaggcgtctattactgttacagtaggggctactggggccaggggacccaggtcaccgtctcctca

SEQ ID NO: 647 - DNA, 336 bp, synthetic construct
  source 1..336: mol_type = other DNA
gaggtgcagctggtgcagtctgggggaggattggtgcaggctgggggctctctgagactctcctgtgcagcctctggaagggacttcagtgacacttccatggcctggcaccgccaggctccagggaaggagcggctgtgggtcgcaggtattcgaagtggtagtaccagtacgagctatgcagactccgtgaagggccgattcaccatctccagagacgacgccaagaacacagtgtatctgcaaatggacaacctgacccctgaggacacagccgtctatttctgttattcaaaggggtactggggccaggggacccaggtcactgtctcctca

SEQ ID NO: 648 - DNA, 342 bp, synthetic construct
  source 1..342: mol_type = other DNA
gaggtgcagctggtggagtctgggggaggcttggtgcaacctggggagtctctgagactctcctgtacagcctctgaaagcatcagtatatacggcgtgggctggtaccgtcaggctccgggcgagcagcgcgtgttggtcgcacatcttaaaaggaatggtttaacagagtataaagactccgtgaagggccgattcaccatctccagagacaacgccaggaacacgatctatctggaaatgaagaacctgaaacctgaggacacggccatctattactgtaatactgcgttgggctcggttttgccctggggccgggggacccaggtcactgtctcctca

SEQ ID NO: 649 - DNA, 384 bp, synthetic construct
  source 1..384: mol_type = other DNA
gaggtgcagctggtggagtctgggggaggcttggtgcagcctggggggtctctgagactctcctgtgtgtcctctgccaccttcggtggctacagcatgggctggttccgccaggctccggggaaggagcgtgaatttgtagcggcgattacctggaatggtggtatcatcaaagattatgcagacggcgtgatgggccgattcaccatctccagaaacagcgccttgaacacggtgtatctgcaaatggacagcctgaaaagtacagacacgggcgtttatgtatgtgcaggagatcggacctactatgctgggggttatgttccgacgagtgagcgtgagtatgccttctggggccaggggacccaggtcaccgtctcctca

SEQ ID NO: 650 - DNA, 345 bp, synthetic construct
  source 1..345: mol_type = other DNA
caggtgcagctggtgcagtctgggggaggcttggtgcaggctggggggtctctgagactctcctgtgcagcctctggaagcatcttccttatcaatgatatgggctggtaccgccaggctccagggaagcagcgcgaattggtcgcagttaggggtggtagcacaaagtatggagactccgtgaagggccgattcaccatctccagagacgacgccaagaacacggtatatctgcaaatgaacagcctgaaacctgaggacacagccgtctattactgtcatagagaatctggacttgggtcgagtgaatactggggccaggggacccaggtcactgtctcctca

SEQ ID NO: 651 - DNA, 354 bp, synthetic construct
  source 1..354: mol_type = other DNA
gaggtgcagctggtggagtctgggggaggattggtgcaggctgggggctctctgagactctcctgtacggcctctggacgcactgtcagtaactatcgcatgggctggttccgccagactccagggaaggagcgtgagtttgtagcagcgattgcctgggctggtggtagcttaacctatgcagactccgtgaagggccgattcaccatctccagagacaacgccaagaacacggtgtatctgcaaatgaatagcctggaacctacggacacagccgtctattactgtaagggtagtcgtatcttcccgaccagggactattggggcaaagggacccaggtcaccgtctcctca

SEQ ID NO: 652 - DNA, 366 bp, synthetic construct
  source 1..366: mol_type = other DNA
gaggtgcagctggtggagtctgggggaggattggtgcaggctggggactctctgagactctcctgtgcagcctctggattcgcttcgcatctttatgccatcggctggttccgccaggccccagggaaggagcgcgagaaggtctcatgtattagtagcaatgatggtagcacatactatgcagactccgtgaagggccgattcaccatctccagagacaccgtcaaagacatggtgtatctgcaaatgaacagcctgaaacctgaggacacggccgtttattactgtgcgacagatctgactgtacactgtttcatggcggagtatgactggtggggccaggggacccaggtcactgtctcctca

SEQ ID NO: 653 - DNA, 366 bp, synthetic construct
  source 1..366: mol_type = other DNA
gaggtgcagctggtggagtctgggggaggcttggtgcagcctggggggtctctgaggctctcctgtgcagcctctggattcgcttcgcatctttatgccatcggctggttccgccaggccccagggaaggagcgcgagaaggtctcatgtattagtagcaatgatggtagcacatactatgcagactccgtgaagggccgattcaccatctccagagacaccgtcaaagacatggtgtatctgcaaatgaacagcctgaaacctgaggacacggccgtttattactgtgcgacagatctgactgtacactgtttcatggcggagtatgactggtggggccaggggacccaggtcaccgtctcctca

SEQ ID NO: 654 - DNA, 363 bp, synthetic construct
  source 1..363: mol_type = other DNA
gaggtgcagctggtggagtctgggggacgattggtgcaggccgggggctctctgagactctcctgtacagcctctggactggccttcagtacccatactatgcactggttccgccaggctccagggaaggagcgtgagtttgtaggagcgattaggtggagtgatgaagacactgagtatgcagactctgtgaagggccgattcaccatctccagagacaacgccaagagcacggtgtatctgcaaatgaacaacctgaaacctgaggacacggccgtttattactgtgcagcagcccggggagtaggtacttctggccatatgaaatactggggccaggggacccaggtcactgtctcctca

SEQ ID NO: 655 - DNA, 411 bp, synthetic construct
  source 1..411: mol_type = other DNA
caggtgcagctggtgcagtctgggggaggcttggtgcaggctggggggtctctgagactctcctgtgcagcctctggaagtatcttcagtgacattaccctggcctggcaccgccagattccagggaaagagcgcgagtgggtcgcaggtatcagtcgcagtggaagccccagctatcgggactccgtgaagggccgattcaccatctctcgagacaacgccaagaacacggtattcctacaaatgaacagtctggaacccgaggacacaggcgtctattactgttacagtaggggctactggggccaggggacccaggtcaccgtctcctcagcggccgcagaacaaaaactcatctcagaagaggatctgaatggggccgcacatcaccaccatcaccatgggagctag

SEQ ID NO: 656 - DNA, 414 bp, synthetic construct
  source 1..414: mol_type = other DNA
gaggtgcagctggtgcagtctgggggaggattggtgcaggctgggggctctctgagactctcctgtgcagcctctggaagggacttcagtgacacttccatggcctggcaccgccaggctccagggaaggagcggctgtgggtcgcaggtattcgaagtggtagtaccagtacgagctatgcagactccgtgaagggccgattcaccatctccagagacgacgccaagaacacagtgtatctgcaaatggacaacctgacccctgaggacacagccgtctatttctgttattcaaaggggtactggggccaggggacccaggtcactgtctcctcagcggccgcagaacaaaaactcatctcagaagaggatctgaatggggccgcacatcaccaccatcaccatgggagctag

SEQ ID NO: 657 - DNA, 420 bp, synthetic construct
  source 1..420: mol_type = other DNA
gaggtgcagctggtggagtctgggggaggcttggtgcaacctggggagtctctgagactctcctgtacagcctctgaaagcatcagtatatacggcgtgggctggtaccgtcaggctccgggcgagcagcgcgtgttggtcgcacatcttaaaaggaatggtttaacagagtataaagactccgtgaagggccgattcaccatctccagagacaacgccaggaacacgatctatctggaaatgaagaacctgaaacctgaggacacggccatctattactgtaatactgcgttgggctcggttttgccctggggccgggggacccaggtcactgtctcctcagcggccgcagaacaaaaactcatctcagaagaggatctgaatggggccgcacatcaccaccatcaccatgggagctag

SEQ ID NO: 658 - DNA, 462 bp, synthetic construct
  source 1..462: mol_type = other DNA
gaggtgcagctggtggagtctgggggaggcttggtgcagcctggggggtctctgagactctcctgtgtgtcctctgccaccttcggtggctacagcatgggctggttccgccaggctccggggaaggagcgtgaatttgtagcggcgattacctggaatggtggtatcatcaaagattatgcagacggcgtgatgggccgattcaccatctccagaaacagcgccttgaacacggtgtatctgcaaatggacagcctgaaaagtacagacacgggcgtttatgtatgtgcaggagatcggacctactatgctgggggttatgttccgacgagtgagcgtgagtatgccttctggggccaggggacccaggtcaccgtctcctcagcggccgcagaacaaaaactcatctcagaagaggatctgaatggggccgcacatcaccaccatcaccatgggagctag

SEQ ID NO: 659 - DNA, 423 bp, synthetic construct
  source 1..423: mol_type = other DNA
caggtgcagctggtgcagtctgggggaggcttggtgcaggctggggggtctctgagactctcctgtgcagcctctggaagcatcttccttatcaatgatatgggctggtaccgccaggctccagggaagcagcgcgaattggtcgcagttaggggtggtagcacaaagtatggagactccgtgaagggccgattcaccatctccagagacgacgccaagaacacggtatatctgcaaatgaacagcctgaaacctgaggacacagccgtctattactgtcatagagaatctggacttgggtcgagtgaatactggggccaggggacccaggtcactgtctcctcagcggccgcagaacaaaaactcatctcagaagaggatctgaatggggccgcacatcaccaccatcaccatgggagctag

SEQ ID NO: 660 - DNA, 432 bp, synthetic construct
  source 1..432: mol_type = other DNA
gaggtgcagctggtggagtctgggggaggattggtgcaggctgggggctctctgagactctcctgtacggcctctggacgcactgtcagtaactatcgcatgggctggttccgccagactccagggaaggagcgtgagtttgtagcagcgattgcctgggctggtggtagcttaacctatgcagactccgtgaagggccgattcaccatctccagagacaacgccaagaacacggtgtatctgcaaatgaatagcctggaacctacggacacagccgtctattactgtaagggtagtcgtatcttcccgaccagggactattggggcaaagggacccaggtcaccgtctcctcagcggccgcagaacaaaaactcatctcagaagaggatctgaatggggccgcacatcaccaccatcaccatgggagctag

SEQ ID NO: 661 - DNA, 444 bp, synthetic construct
  source 1..444: mol_type = other DNA
gaggtgcagctggtggagtctgggggaggattggtgcaggctggggactctctgagactctcctgtgcagcctctggattcgcttcgcatctttatgccatcggctggttccgccaggccccagggaaggagcgcgagaaggtctcatgtattagtagcaatgatggtagcacatactatgcagactccgtgaagggccgattcaccatctccagagacaccgtcaaagacatggtgtatctgcaaatgaacagcctgaaacctgaggacacggccgtttattactgtgcgacagatctgactgtacactgtttcatggcggagtatgactggtggggccaggggacccaggtcactgtctcctcagcggccgcagaacaaaaactcatctcagaagaggatctgaatggggccgcacatcaccaccatcaccatgggagctag

SEQ ID NO: 662 - DNA, 444 bp, synthetic construct
  source 1..444: mol_type = other DNA
gaggtgcagctggtggagtctgggggaggcttggtgcagcctggggggtctctgaggctctcctgtgcagcctctggattcgcttcgcatctttatgccatcggctggttccgccaggccccagggaaggagcgcgagaaggtctcatgtattagtagcaatgatggtagcacatactatgcagactccgtgaagggccgattcaccatctccagagacaccgtcaaagacatggtgtatctgcaaatgaacagcctgaaacctgaggacacggccgtttattactgtgcgacagatctgactgtacactgtttcatggcggagtatgactggtggggccaggggacccaggtcaccgtctcctcagcggccgcagaacaaaaactcatctcagaagaggatctgaatggggccgcacatcaccaccatcaccatgggagctag

SEQ ID NO: 663 - DNA, 441 bp, synthetic construct
  source 1..441: mol_type = other DNA
gaggtgcagctggtggagtctgggggacgattggtgcaggccgggggctctctgagactctcctgtacagcctctggactggccttcagtacccatactatgcactggttccgccaggctccagggaaggagcgtgagtttgtaggagcgattaggtggagtgatgaagacactgagtatgcagactctgtgaagggccgattcaccatctccagagacaacgccaagagcacggtgtatctgcaaatgaacaacctgaaacctgaggacacggccgtttattactgtgcagcagcccggggagtaggtacttctggccatatgaaatactggggccaggggacccaggtcactgtctcctcagcggccgcagaacaaaaactcatctcagaagaggatctgaatggggccgcacatcaccaccatcaccatgggagctag

SEQ ID NO: 664 - protein, 227 aa, synthetic construct
DKTHTCPPCPAPEAAGGPSVFLFPPKPKDTLMISRTPEVTCVVVDVSHEDPEVKFNWYVDGVEVHNAKTKPREEQYNSTYRVVSVLTVLHQDWLNGKEYKCKVSNKALPAPIEKTISKAKGQPREPQVYTLPPSRDELTKNQVSLWCLVKGFYPSDIAVEWESNGQPENNYKTTPPVLDSDGSFFLYSKLTVDKSRWQQGNVFSCSVMHEALHNHYTQKSLSLSPGK

SEQ ID NO: 665 - protein, 227 aa, synthetic construct
DKTHTCPPCPAPEAAGGPSVFLFPPKPKDTLMISRTPEVTCVVVDVSHEDPEVKFNWYVDGVEVHNAKTKPREEQYNSTYRVVSVLTVLHQDWLNGKEYKCKVSNKALPAPIEKTISKAKGQPREPQVYTLPPSRDELTKNQVSLSCAVKGFYPSDIAVEWESNGQPENNYKTTPPVLDSDGSFFLVSKLTVDKSRWQQGNVFSCSVMHEALHNHYTQKSLSLSPGK

SEQ ID NO: 666 - protein, 368 aa, synthetic construct
MYRMQLLSCIALSLALVTNSEVQLVESGGGVVQPGGSLKLSCVASGTDFSINFIRWYRQAPGKQREFVAGFTATGNTNYADSMKGRFTISRDNTKNAVYLQIDSLKPEDTAVYYCYMLDKWGQGTQVTVSSGGGGSGGGGSDKTHTCPPCPAPEAAGGPSVFLFPPKPKDTLMISRTPEVTCVVVDVSHEDPEVKFNWYVDGVEVHNAKTKPREEQYNSTYRVVSVLTVLHQDWLNGKEYKCKVSNKALPAPIEKTISKAKGQPREPQVYTLPPSRDELTKNQVSLWCLVKGFYPSDIAVEWESNGQPENNYKTTPPVLDSDGSFFLYSKLTVDKSRWQQGNVFSCSVMHEALHNHYTQKSLSLSPGK

SEQ ID NO: 667 - protein, 257 aa, synthetic construct
MYRMQLLSCIALSLALVTNSDKTHTCPPCPAPEAAGGPSVFLFPPKPKDTLMISRTPEVTCVVVDVSHEDPEVKFNWYVDGVEVHNAKTKPREEQYNSTYRVVSVLTVLHQDWLNGKEYKCKVSNKALPAPIEKTISKAKGQPREPQVYTLPPSRDELTKNQVSLSCAVKGFYPSDIAVEWESNGQPENNYKTTPPVLDSDGSFFLVSKLTVDKSRWQQGNVFSCSVMHEALHNHYTQKSLSLSPGKEQKLISEEDL

SEQ ID NO: 668 - DNA, 1098 bp, synthetic construct
  source 1..1098: mol_type = other DNA
atgcaactcctgtcttgcattgcactaagtcttgcacttgtcacgaattcggaggtgcagctggtggagagcggcggcggcgtggtgcagcccggcggcagcctgaagctgagctgcgtggccagcggcaccgacttcagcatcaacttcatcagatggtacagacaggcccccggcaagcagagagagttcgtggccggcttcaccgccaccggcaacaccaactacgccgacagcatgaagggcagattcaccatcagcagagacaacaccaagaacgccgtgtacctgcagatcgacagcctgaagcccgaggacaccgccgtgtactactgctacatgctggacaagtggggccagggcacccaggtgaccgtgagcagcggcggcggaggcagcggcggcggaggcagcgacaaaactcacacatgcccaccgtgcccagcacctgaagccgccgggggaccgtcagtcttcctcttccccccaaaacccaaggacaccctcatgatctcccggacccctgaggtcacatgcgtggtggtggacgtgagccacgaagaccctgaggtcaagttcaactggtacgtggacggcgtggaggtgcataatgccaagacaaagccgcgggaggagcagtacaacagcacgtaccgtgtggtcagcgtcctcaccgtcctgcaccaggactggctgaatggcaaggagtacaagtgcaaggtctccaacaaagccctcccagcccccatcgagaaaaccatctccaaagccaaagggcagccccgagaaccacaggtgtataccctgcccccatcccgggatgagctgaccaagaaccaggtcagcctgtggtgcctggtcaaaggcttctatcccagcgacatcgccgtggagtgggagagcaatgggcagccggagaacaactacaagaccacgcctcccgtgctggactccgacggctccttcttcctctacagcaagctcaccgtggacaagagcaggtggcagcaggggaacgtcttctcatgctccgtgatgcatgaggctctgcacaaccactacacgcagaagagcctctccctgtctccgggtaaatga

SEQ ID NO: 669 - DNA, 774 bp, synthetic construct
  source 1..774: mol_type = other DNA
atgtacaggatgcaactcctgtcttgcattgcactaagtcttgcacttgtcacgaattcggacaaaactcacacatgcccaccgtgcccagcacctgaagccgccgggggaccgtcagtcttcctcttccccccaaaacccaaggacaccctcatgatctcccggacccctgaggtcacatgcgtggtggtggacgtgagccacgaagaccctgaggtcaagttcaactggtacgtggacggcgtggaggtgcataatgccaagacaaagccgcgggaggagcagtacaacagcacgtaccgtgtggtcagcgtcctcaccgtcctgcaccaggactggctgaatggcaaggagtacaagtgcaaggtctccaacaaagccctcccagcccccatcgagaaaaccatctccaaagccaaagggcagccccgagaaccacaggtgtataccctgcccccatcccgggatgagctgaccaagaaccaggtcagcctgagctgcgccgtcaaaggcttctatcccagcgacatcgccgtggagtgggagagcaatgggcagccggagaacaactacaagaccacgcctcccgtgctggactccgacggctccttcttcctcgtgagcaagctcaccgtggacaagagcaggtggcagcaggggaacgtcttctcatgctccgtgatgcatgaggctctgcacaaccactacacgcagaagagcctctccctgtctccgggtaaagagcagaagctgatcagcgaggaggacctgtga

SEQ ID NO: 670 - protein, 11 aa, synthetic construct
WGRGTQVTVSS

SEQ ID NO: 671 - protein, 8 aa, synthetic construct
GTDKSINF

SEQ ID NO: 672 - protein, 8 aa, synthetic construct
GTDRSINF

SEQ ID NO: 673 - protein, 8 aa, synthetic construct
GEIKSINF

SEQ ID NO: 674 - protein, 8 aa, synthetic construct
GEIRSINF

SEQ ID NO: 675 - protein, 111 aa, synthetic construct
EVQLVESGGGVVQPGGSLKLSCVASGTDKSINFIRWYRQAPGKQREFVAGFTATGNTNYADSMKGRFTISRDNTKNAVYLQIDSLKPEDTAVYYCYMLDKWGQGTQVTVSS

SEQ ID NO: 676 - protein, 111 aa, synthetic construct
EVQLVESGGGVVQPGGSLKLSCVASGTDRSINFIRWYRQAPGKQREFVAGFTATGNTNYADSMKGRFTISRDNTKNAVYLQIDSLKPEDTAVYYCYMLDKWGQGTQVTVSS

SEQ ID NO: 677 - protein, 111 aa, synthetic construct
EVQLVESGGGVVQPGGSLRLSCAASGEIKSINFMRWYRQAPGKQREWVAGFTRDGSTNYPDSAKGRFTISRDNAKNTVYLQIDSLKPEDTAVYYCYMLDTWGQGTQVTVSS

SEQ ID NO: 678 - protein, 111 aa, synthetic construct
EVQLVESGGGVVQPGGSLRLSCAASGEIRSINFMRWYRQAPGKQREWVAGFTRDGSTNYPDSAKGRFTISRDNAKNTVYLQIDSLKPEDTAVYYCYMLDTWGQGTQVTVSS

SEQ ID NO: 679 - protein, 136 aa, synthetic construct
EVQLVESGGGVVQPGGSLKLSCVASGTDKSINFIRWYRQAPGKQREFVAGFTATGNTNYADSMKGRFTISRDNTKNAVYLQIDSLKPEDTAVYYCYMLDKWGQGTQVTVSSAAAEQKLISEEDLNGAAHHHHHHGS

SEQ ID NO: 680 - protein, 136 aa, synthetic construct
EVQLVESGGGVVQPGGSLKLSCVASGTDRSINFIRWYRQAPGKQREFVAGFTATGNTNYADSMKGRFTISRDNTKNAVYLQIDSLKPEDTAVYYCYMLDKWGQGTQVTVSSAAAEQKLISEEDLNGAAHHHHHHGS

SEQ ID NO: 681 - protein, 136 aa, synthetic construct
EVQLVESGGGVVQPGGSLRLSCAASGEIKSINFMRWYRQAPGKQREWVAGFTRDGSTNYPDSAKGRFTISRDNAKNTVYLQIDSLKPEDTAVYYCYMLDTWGQGTQVTVSSAAAEQKLISEEDLNGAAHHHHHHGS

SEQ ID NO: 682 - protein, 136 aa, synthetic construct
EVQLVESGGGVVQPGGSLRLSCAASGEIRSINFMRWYRQAPGKQREWVAGFTRDGSTNYPDSAKGRFTISRDNAKNTVYLQIDSLKPEDTAVYYCYMLDTWGQGTQVTVSSAAAEQKLISEEDLNGAAHHHHHHGS

SEQ ID NO: 683 - DNA, 333 bp, synthetic construct
  source 1..333: mol_type = other DNA
gaggtgcagctggtggagtctgggggaggcgtggtgcagcctggggggtctctaaaactctcctgcgtagcctcgggaacggacaaaagtatcaattttatacgctggtaccgccaggctccagggaagcagcgcgagttcgtcgcaggatttactgcgactggtaacacaaactatgcagactccatgaaggggcgattcaccatctccagagacaacaccaagaacgcggtgtatctgcaaatagacagcctgaaacctgaggacacggccgtgtattactgctatatgttggacaagtggggccaggggacccaggtcaccgtctcctca

SEQ ID NO: 684 - DNA, 333 bp, synthetic construct
  source 1..333: mol_type = other DNA
gaggtgcagctggtggagtctgggggaggcgtggtgcagcctggggggtctctaaaactctcctgcgtagcctcgggaacggacagaagtatcaattttatacgctggtaccgccaggctccagggaagcagcgcgagttcgtcgcaggatttactgcgactggtaacacaaactatgcagactccatgaaggggcgattcaccatctccagagacaacaccaagaacgcggtgtatctgcaaatagacagcctgaaacctgaggacacggccgtgtattactgctatatgttggacaagtggggccaggggacccaggtcaccgtctcctca

SEQ ID NO: 685 - DNA, 333 bp, synthetic construct
  source 1..333: mol_type = other DNA
gaggtgcagctggtggagtctgggggaggcgtggtgcagcctggggggtctctgagactctcctgtgcagcctctggagagatcaaaagtatcaattttatgcgctggtaccgccaggctccagggaagcagcgcgagtgggtcgcaggttttactagggatggaagcacaaactatccagactccgcgaagggccgattcaccatctctagagacaacgccaagaacacggtgtatctgcaaatagacagcctgaaacctgaggacacggccgtctattattgttatatgttggacacctggggccaggggacccaggtcactgtctcctca

SEQ ID NO: 686 - DNA, 333 bp, synthetic construct
  source 1..333: mol_type = other DNA
gaggtgcagctggtggagtctgggggaggcgtggtgcagcctggggggtctctgagactctcctgtgcagcctctggagagatcagaagtatcaattttatgcgctggtaccgccaggctccagggaagcagcgcgagtgggtcgcaggttttactagggatggaagcacaaactatccagactccgcgaagggccgattcaccatctctagagacaacgccaagaacacggtgtatctgcaaatagacagcctgaaacctgaggacacggccgtctattattgttatatgttggacacctggggccaggggacccaggtcactgtctcctca

SEQ ID NO: 687 - DNA, 411 bp, synthetic construct
  source 1..411: mol_type = other DNA
gaggtgcagctggtggagtctgggggaggcgtggtgcagcctggggggtctctaaaactctcctgcgtagcctcgggaacggacaaaagtatcaattttatacgctggtaccgccaggctccagggaagcagcgcgagttcgtcgcaggatttactgcgactggtaacacaaactatgcagactccatgaaggggcgattcaccatctccagagacaacaccaagaacgcggtgtatctgcaaatagacagcctgaaacctgaggacacggccgtgtattactgctatatgttggacaagtggggccaggggacccaggtcaccgtctcctcagcggccgcagaacaaaaactcatctcagaagaggatctgaatggggccgcacatcaccaccatcaccatgggagctag

SEQ ID NO: 688 - DNA, 411 bp, synthetic construct
  source 1..411: mol_type = other DNA
gaggtgcagctggtggagtctgggggaggcgtggtgcagcctggggggtctctaaaactctcctgcgtagcctcgggaacggacagaagtatcaattttatacgctggtaccgccaggctccagggaagcagcgcgagttcgtcgcaggatttactgcgactggtaacacaaactatgcagactccatgaaggggcgattcaccatctccagagacaacaccaagaacgcggtgtatctgcaaatagacagcctgaaacctgaggacacggccgtgtattactgctatatgttggacaagtggggccaggggacccaggtcaccgtctcctcagcggccgcagaacaaaaactcatctcagaagaggatctgaatggggccgcacatcaccaccatcaccatgggagctag

SEQ ID NO: 689 - DNA, 411 bp, synthetic construct
  source 1..411: mol_type = other DNA
gaggtgcagctggtggagtctgggggaggcgtggtgcagcctggggggtctctgagactctcctgtgcagcctctggagagatcaaaagtatcaattttatgcgctggtaccgccaggctccagggaagcagcgcgagtgggtcgcaggttttactagggatggaagcacaaactatccagactccgcgaagggccgattcaccatctctagagacaacgccaagaacacggtgtatctgcaaatagacagcctgaaacctgaggacacggccgtctattattgttatatgttggacacctggggccaggggacccaggtcactgtctcctcagcggccgcagaacaaaaactcatctcagaagaggatctgaatggggccgcacatcaccaccatcaccatgggagctag

SEQ ID NO: 690 - DNA, 411 bp, synthetic construct
  source 1..411: mol_type = other DNA
gaggtgcagctggtggagtctgggggaggcgtggtgcagcctggggggtctctgagactctcctgtgcagcctctggagagatcagaagtatcaattttatgcgctggtaccgccaggctccagggaagcagcgcgagtgggtcgcaggttttactagggatggaagcacaaactatccagactccgcgaagggccgattcaccatctctagagacaacgccaagaacacggtgtatctgcaaatagacagcctgaaacctgaggacacggccgtctattattgttatatgttggacacctggggccaggggacccaggtcactgtctcctcagcggccgcagaacaaaaactcatctcagaagaggatctgaatggggccgcacatcaccaccatcaccatgggagctag

SEQ ID NO: 691 - protein, 136 aa, synthetic construct
EVQLVESGGGVVQPGGSLKLSCVASGTDFSINFIRWYSQAPGKQREFVAGFTATGNTNYADSMKGRLTISRDNTKNAVYLQIDSLKPEDTAVYYCYMLGKWGQGTQVTVSSAAAEQKLISEEDLNGAAHHHHHHGS

SEQ ID NO: 692 - protein, 136 aa, synthetic construct; identical to SEQ ID NO: 691

SEQ ID NO: 693 - protein, 136 aa, synthetic construct
EVQLVESGGGVVQPGGSLRLSCAASGEIFSINFMRWYRQAPGKQREWVAGFTRDGSTNYPDSAKGRFTISRDNAKNTVYLQIDSLKPEDTAVYYCYMLKTWGQGTQVTVSSAAAEQKLISEEDLNGAAHHHHHHGS

SEQ ID NO: 694 - protein, 136 aa, synthetic construct
EVQLVESGGGVVQPGGSLRLSCAASGEIRSINFMRWYRQAPGKQREWVAGFTRDGSTNYPDIAKGRFTISRDNAKNTVYLQIDSLKPEDTAVYYCYMLDTWGQGTQVTVSSAAAEQKLISEEDLNGAAHHHHHHGS

SEQ ID NO: 695 - protein, 136 aa, synthetic construct
EVQLVESGGGVVQPGGSLRLSCAASGEIRSINFMRWYRQAPGKQREWVAGFTRDGSLNYPDSAKGRFTISRDNAKNTVYLQIDSLKPEDTAVYYCYMLDTWGKGTQVTVSSAAAEQKLISEEDLNGAAHHHHHHGS

SEQ ID NO: 696 - protein, 136 aa, synthetic construct
EVQLVESGGGVVQPGGSLRLSCAASGEIFSINVMRWYRQAPGKQREWVAGFTRDGSTNYPDSAKGRFTISRDNAKNTVYLQIDSLKPEDTAVYYCYMLDTWGQGTQVTVSSAAAEQKLISEEDLNGAAHHHHHHGS

SEQ ID NO: 697 - protein, 136 aa, synthetic construct
EVQLVESGGGVVQPGGSLRLSCAASGEIFSINFMRWYRQAPGKQREWVAGFTRDGSTNYPDSAKGRFTISEDNAKNTVYLQIDSLKPEDTAVYYCYMLRTWGQGTQVTVSSAAAEQKLISEEDLNGAAHHHHHHGS

SEQ ID NO: 698 - protein, 136 aa, synthetic construct
EVQLVESGGGVVQPGGSLRLSCAASGEIRSINFMRWYRQAPGKQREWVAGFTRTGSTNYPDSAKGRFTISRDNAKNTVYLQIDSLKPEDTAVYYCYMLDTWGQGTQVTVSSAAAEQKLISEEDLNGAAHHHHHHGS

SEQ ID NO: 699 - protein, 136 aa, synthetic construct
EVQLVESGGGVVQPGGSLRLSCAASGEIFKINFMRWYRQAPGKQREWVAGFTRDGSTNYPDSAKGRFTISRDNAKNTVYLQIDSLKPEDTAVYYCYMLDTWGQGTQVTVSSAAAEQKLISEEDLNGAAHHHHHHGS

SEQ ID NO: 700 - protein, 136 aa, synthetic construct
EVQLVESGGGVVQPGGSLRLSCAASGEIKSINFMRWYRQAPGKQREWVSGFTRDGSTNYPDSAKGRFTISRDNAKNTVYLQIDSLKPEDTAVYYCYMLDTWGQGTQVTVSSAAAEQKLISEEDLNGAAHHHHHHGS

SEQ ID NO: 701 - protein, 111 aa, synthetic construct
EVQLVESGGGVVQPGGSLKLSCVASGTDFSINFIRWYSQAPGKQREFVAGFTATGNTNYADSMKGRLTISRDNTKNAVYLQIDSLKPEDTAVYYCYMLGKWGQGTQVTVSS

SEQ ID NO: 702 - protein, 111 aa, synthetic construct
EVQLVESGGGVVQPGGSLRLSCAASGEIFSINFMRWYRQAPGKQREWVAGFTRDGSTNYPDSAKGRFTISRDNAKNTVYLQIDSLKPEDTAVYYCYMLKTWGQGTQVTVSS

SEQ ID NO: 703 - protein, 111 aa, synthetic construct
EVQLVESGGGVVQPGGSLRLSCAASGEIRSINFMRWYRQAPGKQREWVAGFTRDGSTNYPDIAKGRFTISRDNAKNTVYLQIDSLKPEDTAVYYCYMLDTWGQGTQVTVSS

SEQ ID NO: 704 - protein, 111 aa, synthetic construct
EVQLVESGGGVVQPGGSLRLSCAASGEIRSINFMRWYRQAPGKQREWVAGFTRDGSLNYPDSAKGRFTISRDNAKNTVYLQIDSLKPEDTAVYYCYMLDTWGKGTQVTVSS

SEQ ID NO: 705 - protein, 111 aa, synthetic construct
EVQLVESGGGVVQPGGSLRLSCAASGEIFSINVMRWYRQAPGKQREWVAGFTRDGSTNYPDSAKGRFTISRDNAKNTVYLQIDSLKPEDTAVYYCYMLDTWGQGTQVTVSS

SEQ ID NO: 706 - protein, 111 aa, synthetic construct
EVQLVESGGGVVQPGGSLRLSCAASGEIFSINFMRWYRQAPGKQREWVAGFTRDGSTNYPDSAKGRFTISEDNAKNTVYLQIDSLKPEDTAVYYCYMLRTWGQGTQVTVSS

SEQ ID NO: 707 - protein, 111 aa, synthetic construct
EVQLVESGGGVVQPGGSLRLSCAASGEIRSINFMRWYRQAPGKQREWVAGFTRTGSTNYPDSAKGRFTISRDNAKNTVYLQIDSLKPEDTAVYYCYMLDTWGQGTQVTVSS

SEQ ID NO: 708 - protein, 111 aa, synthetic construct
EVQLVESGGGVVQPGGSLRLSCAASGEIFKINFMRWYRQAPGKQREWVAGFTRDGSTNYPDSAKGRFTISRDNAKNTVYLQIDSLKPEDTAVYYCYMLDTWGQGTQVTVSS

SEQ ID NO: 709 - protein, 111 aa, synthetic construct
EVQLVESGGGVVQPGGSLRLSCAASGEIKSINFMRWYRQAPGKQREWVSGFTRDGSTNYPDSAKGRFTISRDNAKNTVYLQIDSLKPEDTAVYYCYMLDTWGQGTQVTVSS

SEQ ID NO: 710 - protein, 8 aa, synthetic construct
GEIFSINV

SEQ ID NO: 711 - protein, 8 aa, synthetic construct
GEIFKINF

SEQ ID NO: 712 - protein, 7 aa, synthetic construct
FTRTGST

SEQ ID NO: 713 - protein, 5 aa, synthetic construct
YMLGK

SEQ ID NO: 714 - protein, 5 aa, synthetic construct
YMLKT

SEQ ID NO: 715 - protein, 5 aa, synthetic construct
YMLRT

SEQ ID NO: 716 - protein, 17 aa, synthetic construct
IRWYSQAPGKQREFVAG

SEQ ID NO: 717 - protein, 38 aa, synthetic construct
NYADSMKGRLTISRDNTKNAVYLQIDSLKPEDTAVYYC

SEQ ID NO: 718 - protein, 38 aa, synthetic construct
NYPDIAKGRFTISRDNAKNTVYLQIDSLKPEDTAVYYC

SEQ ID NO: 719 - protein, 38 aa, synthetic construct
NYPDSAKGRFTISEDNAKNTVYLQIDSLKPEDTAVYYC

SEQ ID NO: 720 - protein, 17 aa, synthetic construct
MRWYRQAPGKQREWVSG

SEQ ID NO: 721 - DNA, 333 bp, synthetic construct
  source 1..333: mol_type = other DNA
gaggtgcagctggtggagtctgggggaggcgtggtgcagcctggggggtctctaaaactctcctgcgtagcctcgggaacggacttcagtatcaattttatacgctggtacagccaggctccagggaagcagcgcgagttcgtcgcaggatttactgcgactggtaacacaaactatgcagactccatgaaggggcgactgaccatctccagagacaacaccaagaacgcggtgtatctgcaaatagacagcctgaaacctgaggacacggccgtgtattactgctatatgttgggtaagtggggccaggggacccaggtcaccgtctcctca

SEQ ID NO: 722 - DNA, 333 bp, synthetic construct
  source 1..333: mol_type = other DNA
gaggtgcagctggtggagtctgggggaggcgtggtgcagcctggggggtctctgagactctcctgtgcagcctctggagagatcttcagtatcaattttatgcgctggtaccgccaggctccagggaagcagcgcgagtgggtcgcaggttttactagggatggaagcacaaactatccagactccgcgaagggccgattcaccatctctagagacaacgccaagaacacggtgtatctgcaaatagacagcctgaaacctgaggacacggccgtctattattgttatatgttgaaaacctggggccaggggacccaggtcactgtctcctca

SEQ ID NO: 723 - DNA, 333 bp, synthetic construct
  source 1..333: mol_type = other DNA
gaggtgcagctggtggagtctgggggaggcgtggtgcagcctggggggtctctgagactctcctgtgcagcctctggagagatcagaagtatcaattttatgcgctggtaccgccaggctccagggaagcagcgcgagtgggtcgcaggttttactagggatggaagcacaaactatccagacattgcgaagggccgattcaccatctctagagacaacgccaagaacacggtgtatctgcaaatagacagcctgaaacctgaggacacggccgtctattattgttatatgttggacacctggggccaggggacccaggtcactgtctcctca

SEQ ID NO: 724 - DNA, 333 bp, synthetic construct
  source 1..333: mol_type = other DNA
gaggtgcagctggtggagtctgggggaggcgtggtgcagcctggggggtctctgagactctcctgtgcagcctctggagagatcagaagtatcaattttatgcgctggtaccgccaggctccagggaagcagcgcgagtgggtcgcaggttttactagggatggaagcctgaactatccagactccgcgaagggccgattcaccatctctagagacaacgccaagaacacggtgtatctgcaaatagacagcctgaaacctgaggacacggccgtctattattgttatatgttggacacctggggcaaagggacccaggtcactgtctcctca

SEQ ID NO: 725 - DNA, 333 bp, synthetic construct
  source 1..333: mol_type = other DNA
gaggtgcagctggtggagtctgggggaggcgtggtgcagcctggggggtctctgagactctcctgtgcagcctctggagagatcttcagtatcaatgttatgcgctggtaccgccaggctccagggaagcagcgcgagtgggtcgcaggttttactagggatggaagcacaaactatccagactccgcgaagggccgattcaccatctctagagacaacgccaagaacacggtgtatctgcaaatagacagcctgaaacctgaggacacggccgtctattattgttatatgttggacacctggggccaggggacccaggtcactgtctcctca

SEQ ID NO: 726 - DNA, 333 bp, synthetic construct
  source 1..333: mol_type = other DNA
gaggtgcagctggtggagtctgggggaggcgtggtgcagcctggggggtctctgagactctcctgtgcagcctctggagagatcttcagtatcaattttatgcgctggtaccgccaggctccagggaagcagcgcgagtgggtcgcaggttttactagggatggaagcacaaactatccagactccgcgaagggccgattcaccatctctgaagacaacgccaagaacacggtgtatctgcaaatagacagcctgaaacctgaggacacggccgtctattattgttatatgttgcgtacctggggccaggggacccaggtcactgtctcctca

SEQ ID NO: 727 - DNA, 333 bp, synthetic construct
  source 1..333: mol_type = other DNA
gaggtgcagctggtggagtctgggggaggcgtggtgcagcctggggggtctctgagactctcctgtgcagcctctggagagatcagaagtatcaattttatgcgctggtaccgccaggctccagggaagcagcgcgagtgggtcgcaggttttactaggaccggaagcacaaactatccagactccgcgaagggccgattcaccatctctagagacaacgccaagaacacggtgtatctgcaaatagacagcctgaaacctgaggacacggccgtctattattgttatatgttggacacctggggccaggggacccaggtcactgtctcctca

SEQ ID NO: 728 - DNA, 333 bp, synthetic construct
  source 1..333: mol_type = other DNA
gaggtgcagctggtggagtctgggggaggcgtggtgcagcctggggggtctctgagactctcctgtgcagcctctggagagatcttcaaaatcaattttatgcgctggtaccgccaggctccagggaagcagcgcgagtgggtcgcaggttttactagggatggaagcacaaactatccagactccgcgaagggccgattcaccatctctagagacaacgccaagaacacggtgtatctgcaaatagacagcctgaaacctgaggacacggccgtctattattgttatatgttggacacctggggccaggggacccaggtcactgtctcctca

SEQ ID NO: 729 - DNA, 333 bp, synthetic construct
  source 1..333: mol_type = other DNA
gaggtgcagctggtggagtctgggggaggcgtggtgcagcctggggggtctctgagactctcctgtgcagcctctggagagatcaaaagtatcaattttatgcgctggtaccgccaggctccagggaagcagcgcgagtgggtcagcggttttactagggatggaagcacaaactatccagactccgcgaagggccgattcaccatctctagagacaacgccaagaacacggtgtatctgcaaatagacagcctgaaacctgaggacacggccgtctattattgttatatgttggacacctggggccaggggacccaggtcactgtctcctca

SEQ ID NO: 730 - DNA, 411 bp, synthetic construct
  source 1..411: mol_type = other DNA
gaggtgcagctggtggagtctgggggaggcgtggtgcagcctggggggtctctaaaactctcctgcgtagcctcgggaacggacttcagtatcaattttatacgctggtacagccaggctccagggaagcagcgcgagttcgtcgcaggatttactgcgactggtaacacaaactatgcagactccatgaaggggcgactgaccatctccagagacaacaccaagaacgcggtgtatctgcaaatagacagcctgaaacctgaggacacggccgtgtattactgctatatgttgggtaagtggggccaggggacccaggtcaccgtctcctcagcggccgcagaacaaaaactcatctcagaagaggatctgaatggggccgcacatcaccaccatcaccatgggagctag

SEQ ID NO: 731 - DNA, 411 bp, synthetic construct
  source 1..411: mol_type = other DNA
gaggtgcagctggtggagtctgggggaggcgtggtgcagcctggggggtctctgagactctcctgtgcagcctctggagagatcttcagtatcaattttatgcgctggtaccgccaggctccagggaagcagcgcgagtgggtcgcaggttttactagggatggaagcacaaactatccagactccgcgaagggccgattcaccatctctagagacaacgccaagaacacggtgtatctgcaaatagacagcctgaaacctgaggacacggccgtctattattgttatatgttgaaaacctggggccaggggacccaggtcactgtctcctcagcggccgcagaacaaaaactcatctcagaagaggatctgaatggggccgcacatcaccaccatcaccatgggagctag

SEQ ID NO: 732 - DNA, 411 bp, synthetic construct
  source 1..411: mol_type = other DNA
gaggtgcagctggtggagtctgggggaggcgtggtgcagcctggggggtctctgagactctcctgtgcagcctctggagagatcagaagtatcaattttatgcgctggtaccgccaggctccagggaagcagcgcgagtgggtcgcaggttttactagggatggaagcacaaactatccagacattgcgaagggccgattcaccatctctagagacaacgccaagaacacggtgtatctgcaaatagacagcctgaaacctgaggacacggccgtctattattgttatatgttggacacctggggccaggggacccaggtcactgtctcctcagcggccgcagaacaaaaactcatctcagaagaggatctgaatggggccgcacatcaccaccatcaccatgggagctag

SEQ ID NO: 733 - DNA, 411 bp, synthetic construct
  source 1..411: mol_type = other DNA
gaggtgcagctggtggagtctgggggaggcgtggtgcagcctggggggtctctgagactctcctgtgcagcctctggagagatcagaagtatcaattttatgcgctggtaccgccaggctccagggaagcagcgcgagtgggtcgcaggttttactagggatggaagcctgaactatccagactccgcgaagggccgattcaccatctctagagacaacgccaagaacacggtgtatctgcaaatagacagcctgaaacctgaggacacggccgtctattattgttatatgttggacacctggggcaaagggacccaggtcactgtctcctcagcggccgcagaacaaaaactcatctcagaagaggatctgaatggggccgcacatcaccaccatcaccatgggagctag

SEQ ID NO: 734 - DNA, 411 bp, synthetic construct
  source 1..411: mol_type = other DNA
gaggtgcagctggtggagtctgggggaggcgtggtgcagcctggggggtctctgagactctcctgtgcagcctctggagagatcttcagtatcaatgttatgcgctggtaccgccaggctccagggaagcagcgcgagtgggtcgcaggttttactagggatggaagcacaaactatccagactccgcgaagggccgattcaccatctctagagacaacgccaagaacacggtgtatctgcaaatagacagcctgaaacctgaggacacggccgtctattattgttatatgttggacacctggggccaggggacccaggtcactgtctcctcagcggccgcagaacaaaaactcatctcagaagaggatctgaatggggccgcacatcaccaccatcaccatgggagctag

SEQ ID NO: 735 - DNA, 411 bp, synthetic construct
  source 1..411: mol_type = other DNA
gaggtgcagctggtggagtctgggggaggcgtggtgcagcctggggggtctctgagactctcctgtgcagcctctggagagatcttcagtatcaattttatgcgctggtaccgccaggctccagggaagcagcgcgagtgggtcgcaggttttactagggatggaagcacaaactatccagactccgcgaagggccgattcaccatctctgaagacaacgccaagaacacggtgtatctgcaaatagacagcctgaaacctgaggacacggccgtctattattgttatatgttgcgtacctggggccaggggacccaggtcactgtctcctcagcggccgcagaacaaaaactcatctcagaagaggatctgaatggggccgcacatcaccaccatcaccatgggagctag

SEQ ID NO: 736 - DNA, 411 bp, synthetic construct
  source 1..411: mol_type = other DNA
gaggtgcagctggtggagtctgggggaggcgtggtgcagcctggggggtctctgagactctcctgtgcagcctctggagagatcagaagtatcaattttatgcgctggtaccgccaggctccagggaagcagcgcgagtgggtcgcaggttttactaggaccggaagcacaaactatccagactccgcgaagggccgattcaccatctctagagacaacgccaagaacacggtgtatctgcaaatagacagcctgaaacctgaggacacggccgtctattattgttatatgttggacacctggggccaggggacccaggtcactgtctcctcagcggccgcagaacaaaaactcatctcagaagaggatctgaatggggccgcacatcaccaccatcaccatgggagctag

SEQ ID NO: 737 - DNA, 411 bp, synthetic construct
  source 1..411: mol_type = other DNA
gaggtgcagctggtggagtctgggggaggcgtggtgcagcctggggggtctctgagactctcctgtgcagcctctggagagatcttcaaaatcaattttatgcgctggtaccgccaggctccagggaagcagcgcgagtgggtcgcaggttttactagggatggaagcacaaactatccagactccgcgaagggccgattcaccatctctagagacaacgccaagaacacggtgtatctgcaaatagacagcctgaaacctgaggacacggccgtctattattgttatatgttggacacctggggccaggggacccaggtcactgtctcctcagcggccgcagaacaaaaactcatctcagaagaggatctgaatggggccgcacatcaccaccatcaccatgggagctag

SEQ ID NO: 738 - DNA, 411 bp, synthetic construct
  source 1..411: mol_type = other DNA
gaggtgcagctggtggagtctgggggaggcgtggtgcagcctggggggtctctgagactctcctgtgcagcctctggagagatcaaaagtatcaattttatgcgctggtaccgccaggctccagggaagcagcgcgagtgggtcagcggttttactagggatggaagcacaaactatccagactccgcgaagggccgattcaccatctctagagacaacgccaagaacacggtgtatctgcaaatagacagcctgaaacctgaggacacggccgtctattattgttatatgttggacacctggggccaggggacccaggtcactgtctcctcagcggccgcagaacaaaaactcatctcagaagaggatctgaatggggccgcacatcaccaccatcaccatgggagctag